European Patent Application EP 4 814 114 A1, published September 30, 2026. Title: RNA聚合酶变体及其应用. Applicant: 南京诺唯赞生物科技股份有限公司. The sequence listing filed with the application follows.

SEQUENCE LISTING (117 sequences)

SEQ ID NO: 1 - protein, 883 aa, synthetic construct
MNTINIAKNDFSDIELAAIPFNTLADHYGERLAREQLALEHESYEMGEARFRKMFERQLKAGEVADNAAAKPLITTLLPKMIARINDWFEEVKAKRGKRPTAFQFLQEIKPEAVAYITIKTTLACLTSADNTTVQAVASAIGRAIEDEARFGRIRDLEAKHFKKNVEEQLNKRVGHVYKKAFMQVVEADMLSKGLLGGEAWSSWHKEDSIHVGVRCIEMLIESTGMVSLHRQNAGVVGQDSETIELAPEYAEAIATRAGALAGISPMFQPCVVPPKPWTGITGGGYWANGRRPLALVRTHSKKALMRYEDVYMPEVYKAINIAQNTAWKINKKVLAVANVITKWKHCPVEDIPAIEREELPMKPEDIDMNPEALTAWKRAAAAVYRKDKARKSRRISLEFMLEQANKFANHKAIWFPYNMDWRGRVYAVSMFNPQGNDMTKGLLTLAKGKPIGKEGYYWLKIHGANCAGVDKVPFPERIKFIEENHENIMACAKSPLENTWWAEQDSPFCFLAFCFEYAGVQHHGLSYNCSLPLAFDGSCSGIQHFSAMLRDEVGGRAVNLLPSETVQDIYGIVAKKVNEILQADAINGTDNEVVTVTDENTGEISEKVKLGTKALAGQWLAYGVTRSVTKRSVMTLAYGSKEFGFRQQVLEDTIQPAIDSGKGLMFTQPNQAAGYMAKLIWESVSVTVVAAVEAMNWLKSAAKLLAAEVKDKKTGEILRKRCAVHWVTPDGFPVWQEYKKPIQTRLNLMFLGQFRLQPTINTNKDSEIDAHKQESGIAPNFVHSQDGSHLRKTVVWAHEKYGIESFALIHDSFGTIPADAANLFKAVRETMVDTYESCDVLADFYDQFADQLHESQLDKMPALPAKGNLNLRDILESDFAFA

SEQ ID NO: 2 - protein, 883 aa, synthetic construct
MNTINIAKNDFSDIELAAIPFNTLADHYGERLAAEQLALEHESYEMGEARFRKMFERQLKAGEVADNAAAKPLITTLLPKMIARINDWFEEVKAKRGKRPTAFQFLQEIKPEAVAYITIKTTLACLTSADNTTVQAVASAIGRAIEDEARFGRIRDLEAKHFKKNVEEQLNKRVGHVYKKAFMQVVEADMLSKGLLGGEAWSSWHKEDSIHVGVRCIEMLIESTGMVSLHRQNAGVVGQDSETIELAPEYAEAIATRAGALAGISPMFQPCVVPPKPWTGITGGGYWANGRRPLALVRTHSKKALMRYEDVYMPEVYKAINIAQNTAWKINKKVLAVANVITKWKHCPVEDIPAIEREELPMKPEDIDMNPEALTAWKRAAAAVYRKDKARKSRRISLEFMLEQANKFANHKAIWFPYNMDWRGRVYAVSMFNPQGNDMTKGLLTLAKGKPIGKEGYYWLKIHGANCAGVDKVPFPERIKFIEENHENIMACAKSPLENTWWAEQDSPFCFLAFCFEYAGVQHHGLSYNCSLPLAFDGSCSGIQHFSAMLRDEVGGRAVNLLPSETVQDIYGIVAKKVNEILQADAINGTDNEVVTVTDENTGEISEKVKLGTKALAGQWLAYGVTRSVTKRSVMTLAYGSKEFGFRQQVLEDTIQPAIDSGKGLMFTQPNQAAGYMAKLIWESVSVTVVAAVEAMNWLKSAAKLLAAEVKDKKTGEILRKRCAVHWVTPDGFPVWQEYKKPIQTRLNLMFLGQFRLQPTINTNKDSEIDAHKQESGIAPNFVHSQDGSHLRKTVVWAHEKYGIESFALIHDSFGTIPADAANLFKAVRETMVDTYESCDVLADFYDQFADQLHESQLDKMPALPAKGNLNLRDILESDFAFA

SEQ ID NO: 3 - protein, 883 aa, synthetic construct
MNTINIAKNDFSDIELAAIPFNTLADHYGERLAREQLALEHESYEMGEARFRKMEERQLKAGEVADNAAAKPLITTLLPKMIARINDWFEEVKAKRGKRPTAFQFLQEIKPEAVAYITIKTTLACLTSADNTTVQAVASAIGRAIEDEARFGRIRDLEAKHFKKNVEEQLNKRVGHVYKKAFMQVVEADMLSKGLLGGEAWSSWHKEDSIHVGVRCIEMLIESTGMVSLHRQNAGVVGQDSETIELAPEYAEAIATRAGALAGISPMFQPCVVPPKPWTGITGGGYWANGRRPLALVRTHSKKALMRYEDVYMPEVYKAINIAQNTAWKINKKVLAVANVITKWKHCPVEDIPAIEREELPMKPEDIDMNPEALTAWKRAAAAVYRKDKARKSRRISLEFMLEQANKFANHKAIWFPYNMDWRGRVYAVSMFNPQGNDMTKGLLTLAKGKPIGKEGYYWLKIHGANCAGVDKVPFPERIKFIEENHENIMACAKSPLENTWWAEQDSPFCFLAFCFEYAGVQHHGLSYNCSLPLAFDGSCSGIQHFSAMLRDEVGGRAVNLLPSETVQDIYGIVAKKVNEILQADAINGTDNEVVTVTDENTGEISEKVKLGTKALAGQWLAYGVTRSVTKRSVMTLAYGSKEFGFRQQVLEDTIQPAIDSGKGLMFTQPNQAAGYMAKLIWESVSVTVVAAVEAMNWLKSAAKLLAAEVKDKKTGEILRKRCAVHWVTPDGFPVWQEYKKPIQTRLNLMFLGQFRLQPTINTNKDSEIDAHKQESGIAPNFVHSQDGSHLRKTVVWAHEKYGIESFALIHDSFGTIPADAANLFKAVRETMVDTYESCDVLADFYDQFADQLHESQLDKMPALPAKGNLNLRDILESDFAFA

SEQ ID NO: 4 - protein, 883 aa, synthetic construct
MNTINIAKNDFSDIELAAIPFNTLADHYGERLAREQLALEHESYEMGEARFRKMGERQLKAGEVADNAAAKPLITTLLPKMIARINDWFEEVKAKRGKRPTAFQFLQEIKPEAVAYITIKTTLACLTSADNTTVQAVASAIGRAIEDEARFGRIRDLEAKHFKKNVEEQLNKRVGHVYKKAFMQVVEADMLSKGLLGGEAWSSWHKEDSIHVGVRCIEMLIESTGMVSLHRQNAGVVGQDSETIELAPEYAEAIATRAGALAGISPMFQPCVVPPKPWTGITGGGYWANGRRPLALVRTHSKKALMRYEDVYMPEVYKAINIAQNTAWKINKKVLAVANVITKWKHCPVEDIPAIEREELPMKPEDIDMNPEALTAWKRAAAAVYRKDKARKSRRISLEFMLEQANKFANHKAIWFPYNMDWRGRVYAVSMFNPQGNDMTKGLLTLAKGKPIGKEGYYWLKIHGANCAGVDKVPFPERIKFIEENHENIMACAKSPLENTWWAEQDSPFCFLAFCFEYAGVQHHGLSYNCSLPLAFDGSCSGIQHFSAMLRDEVGGRAVNLLPSETVQDIYGIVAKKVNEILQADAINGTDNEVVTVTDENTGEISEKVKLGTKALAGQWLAYGVTRSVTKRSVMTLAYGSKEFGFRQQVLEDTIQPAIDSGKGLMFTQPNQAAGYMAKLIWESVSVTVVAAVEAMNWLKSAAKLLAAEVKDKKTGEILRKRCAVHWVTPDGFPVWQEYKKPIQTRLNLMFLGQFRLQPTINTNKDSEIDAHKQESGIAPNFVHSQDGSHLRKTVVWAHEKYGIESFALIHDSFGTIPADAANLFKAVRETMVDTYESCDVLADFYDQFADQLHESQLDKMPALPAKGNLNLRDILESDFAFA

SEQ ID NO: 5 - protein, 883 aa, synthetic construct
MNTINIAKNDFSDIELAAIPFNTLADHYGERLAREQLALEHESYEMGEARFRKMKERQLKAGEVADNAAAKPLITTLLPKMIARINDWFEEVKAKRGKRPTAFQFLQEIKPEAVAYITIKTTLACLTSADNTTVQAVASAIGRAIEDEARFGRIRDLEAKHFKKNVEEQLNKRVGHVYKKAFMQVVEADMLSKGLLGGEAWSSWHKEDSIHVGVRCIEMLIESTGMVSLHRQNAGVVGQDSETIELAPEYAEAIATRAGALAGISPMFQPCVVPPKPWTGITGGGYWANGRRPLALVRTHSKKALMRYEDVYMPEVYKAINIAQNTAWKINKKVLAVANVITKWKHCPVEDIPAIEREELPMKPEDIDMNPEALTAWKRAAAAVYRKDKARKSRRISLEFMLEQANKFANHKAIWFPYNMDWRGRVYAVSMFNPQGNDMTKGLLTLAKGKPIGKEGYYWLKIHGANCAGVDKVPFPERIKFIEENHENIMACAKSPLENTWWAEQDSPFCFLAFCFEYAGVQHHGLSYNCSLPLAFDGSCSGIQHFSAMLRDEVGGRAVNLLPSETVQDIYGIVAKKVNEILQADAINGTDNEVVTVTDENTGEISEKVKLGTKALAGQWLAYGVTRSVTKRSVMTLAYGSKEFGFRQQVLEDTIQPAIDSGKGLMFTQPNQAAGYMAKLIWESVSVTVVAAVEAMNWLKSAAKLLAAEVKDKKTGEILRKRCAVHWVTPDGFPVWQEYKKPIQTRLNLMFLGQFRLQPTINTNKDSEIDAHKQESGIAPNFVHSQDGSHLRKTVVWAHEKYGIESFALIHDSFGTIPADAANLFKAVRETMVDTYESCDVLADFYDQFADQLHESQLDKMPALPAKGNLNLRDILESDFAFA

SEQ ID NO: 6 - protein, 883 aa, synthetic construct
MNTINIAKNDFSDIELAAIPFNTLADHYGERLAREQLALEHESYEMGEARFRKMLERQLKAGEVADNAAAKPLITTLLPKMIARINDWFEEVKAKRGKRPTAFQFLQEIKPEAVAYITIKTTLACLTSADNTTVQAVASAIGRAIEDEARFGRIRDLEAKHFKKNVEEQLNKRVGHVYKKAFMQVVEADMLSKGLLGGEAWSSWHKEDSIHVGVRCIEMLIESTGMVSLHRQNAGVVGQDSETIELAPEYAEAIATRAGALAGISPMFQPCVVPPKPWTGITGGGYWANGRRPLALVRTHSKKALMRYEDVYMPEVYKAINIAQNTAWKINKKVLAVANVITKWKHCPVEDIPAIEREELPMKPEDIDMNPEALTAWKRAAAAVYRKDKARKSRRISLEFMLEQANKFANHKAIWFPYNMDWRGRVYAVSMFNPQGNDMTKGLLTLAKGKPIGKEGYYWLKIHGANCAGVDKVPFPERIKFIEENHENIMACAKSPLENTWWAEQDSPFCFLAFCFEYAGVQHHGLSYNCSLPLAFDGSCSGIQHFSAMLRDEVGGRAVNLLPSETVQDIYGIVAKKVNEILQADAINGTDNEVVTVTDENTGEISEKVKLGTKALAGQWLAYGVTRSVTKRSVMTLAYGSKEFGFRQQVLEDTIQPAIDSGKGLMFTQPNQAAGYMAKLIWESVSVTVVAAVEAMNWLKSAAKLLAAEVKDKKTGEILRKRCAVHWVTPDGFPVWQEYKKPIQTRLNLMFLGQFRLQPTINTNKDSEIDAHKQESGIAPNFVHSQDGSHLRKTVVWAHEKYGIESFALIHDSFGTIPADAANLFKAVRETMVDTYESCDVLADFYDQFADQLHESQLDKMPALPAKGNLNLRDILESDFAFA

SEQ ID NO: 7 - protein, 883 aa, synthetic construct
MNTINIAKNDFSDIELAAIPFNTLADHYGERLAREQLALEHESYEMGEARFRKMNERQLKAGEVADNAAAKPLITTLLPKMIARINDWFEEVKAKRGKRPTAFQFLQEIKPEAVAYITIKTTLACLTSADNTTVQAVASAIGRAIEDEARFGRIRDLEAKHFKKNVEEQLNKRVGHVYKKAFMQVVEADMLSKGLLGGEAWSSWHKEDSIHVGVRCIEMLIESTGMVSLHRQNAGVVGQDSETIELAPEYAEAIATRAGALAGISPMFQPCVVPPKPWTGITGGGYWANGRRPLALVRTHSKKALMRYEDVYMPEVYKAINIAQNTAWKINKKVLAVANVITKWKHCPVEDIPAIEREELPMKPEDIDMNPEALTAWKRAAAAVYRKDKARKSRRISLEFMLEQANKFANHKAIWFPYNMDWRGRVYAVSMFNPQGNDMTKGLLTLAKGKPIGKEGYYWLKIHGANCAGVDKVPFPERIKFIEENHENIMACAKSPLENTWWAEQDSPFCFLAFCFEYAGVQHHGLSYNCSLPLAFDGSCSGIQHFSAMLRDEVGGRAVNLLPSETVQDIYGIVAKKVNEILQADAINGTDNEVVTVTDENTGEISEKVKLGTKALAGQWLAYGVTRSVTKRSVMTLAYGSKEFGFRQQVLEDTIQPAIDSGKGLMFTQPNQAAGYMAKLIWESVSVTVVAAVEAMNWLKSAAKLLAAEVKDKKTGEILRKRCAVHWVTPDGFPVWQEYKKPIQTRLNLMFLGQFRLQPTINTNKDSEIDAHKQESGIAPNFVHSQDGSHLRKTVVWAHEKYGIESFALIHDSFGTIPADAANLFKAVRETMVDTYESCDVLADFYDQFADQLHESQLDKMPALPAKGNLNLRDILESDFAFA

SEQ ID NO: 8 - protein, 883 aa, synthetic construct
MNTINIAKNDFSDIELAAIPFNTLADHYGERLAREQLALEHESYEMGEARFRKMFERQLKAGEVADNAAAKPLITTLLPKMIARINDWFEEVKAKRGKRPTAFQFLQEIKPEAVAYITIKTTLACLTSADNTTVQAVASAIGRAIEDEARFGRIRDLEAKHFKKNVEEQLNKRVGHVYKKAFMQVVEADMLSKGLLGGEAWSSWHKEDSIHVGVRCIEMLIESTGMVSLHRQNAGVVGQDSETIELAPEYAEAIATRAGALAGISPMFQPCVVPPKPWTGITGGGYWANGRRPLALVRTHSKKALMRYEDVYMPEVYKAINIAQNTAWKINKKVLAVANVITKWKHCPVEDIPAIEREELPMKPEDIDMNPEALTAWKRAAAAVYRKDKARKSRRISLEFMLEQANKFANHKAIWFPYNMDWRGRVYAVSMFNPQGNDMTKGLLTLAKGKPIGKEGYYWLKIHGANCAGVDKVPFPERIKFIEENHENIMACAKSPLENTWWAEQDSPFCFLAFCFEYAGVQHHGLSYNCSLPLAFDGSCSGIQHFSAMLRDEVGGRAVNLLPSETVQDIYGIVAKKVNEILQADAINGTDNEVVTVTDENTGEISEKVKLGTKALAGQWLAYGVTRSVTKRSVMTLAYGSKEFGFRQQVLEDTIQPAIDSGKGLMFTQPNQAAGYMAKLIWESVSVTVVAAVEAMNWLKSAAKLLAAEVKDKKTGEILRKRCAVHWVTPDGFPVWQEYKKPIQTRLNLMFLDQFRLQPTINTNKDSEIDAHKQESGIAPNFVHSQDGSHLRKTVVWAHEKYGIESFALIHDSFGTIPADAANLFKAVRETMVDTYESCDVLADFYDQFADQLHESQLDKMPALPAKGNLNLRDILESDFAFA

SEQ ID NO: 9 - protein, 883 aa, synthetic construct
MNTINIAKNDFSDIELAAIPFNTLADHYGERLAREQLALEHESYEMGEARFRKMFERQLKAGEVADNAAAKPLITTLLPKMIARINDWFEEVKAKRGKRPTAFQFLQEIKPEAVAYITIKTTLACLTSADNTTVQAVASAIGRAIEDEARFGRDRDLEAKHFKKNVEEQLNKRVGHVYKKAFMQVVEADMLSKGLLGGEAWSSWHKEDSIHVGVRCIEMLIESTGMVSLHRQNAGVVGQDSETIELAPEYAEAIATRAGALAGISPMFQPCVVPPKPWTGITGGGYWANGRRPLALVRTHSKKALMRYEDVYMPEVYKAINIAQNTAWKINKKVLAVANVITKWKHCPVEDIPAIEREELPMKPEDIDMNPEALTAWKRAAAAVYRKDKARKSRRISLEFMLEQANKFANHKAIWFPYNMDWRGRVYAVSMFNPQGNDMTKGLLTLAKGKPIGKEGYYWLKIHGANCAGVDKVPFPERIKFIEENHENIMACAKSPLENTWWAEQDSPFCFLAFCFEYAGVQHHGLSYNCSLPLAFDGSCSGIQHFSAMLRDEVGGRAVNLLPSETVQDIYGIVAKKVNEILQADAINGTDNEVVTVTDENTGEISEKVKLGTKALAGQWLAYGVTRSVTKRSVMTLAYGSKEFGFRQQVLEDTIQPAIDSGKGLMFTQPNQAAGYMAKLIWESVSVTVVAAVEAMNWLKSAAKLLAAEVKDKKTGEILRKRCAVHWVTPDGFPVWQEYKKPIQTRLNLMFLGQFRLQPTINTNKDSEIDAHKQESGIAPNFVHSQDGSHLRKTVVWAHEKYGIESFALIHDSFGTIPADAANLFKAVRETMVDTYESCDVLADFYDQFADQLHESQLDKMPALPAKGNLNLRDILESDFAFA

SEQ ID NO: 10 - protein, 883 aa, synthetic construct
MNTINIAKNDFSDIELAAIPFNTLADHYGERLAREQLALEHESYEMGEARFRKMFERQLKAGEVADNAAAKPLITTLLPKMIARINDWFEEVKAKRGKRPTAFQFLQEIKPEAVAYITIKTTLACLTSADNTTVQAVASAIGRAIEDEARFGRIRDLEAKHFKKNVEEQANKRVGHVYKKAFMQVVEADMLSKGLLGGEAWSSWHKEDSIHVGVRCIEMLIESTGMVSLHRQNAGVVGQDSETIELAPEYAEAIATRAGALAGISPMFQPCVVPPKPWTGITGGGYWANGRRPLALVRTHSKKALMRYEDVYMPEVYKAINIAQNTAWKINKKVLAVANVITKWKHCPVEDIPAIEREELPMKPEDIDMNPEALTAWKRAAAAVYRKDKARKSRRISLEFMLEQANKFANHKAIWFPYNMDWRGRVYAVSMFNPQGNDMTKGLLTLAKGKPIGKEGYYWLKIHGANCAGVDKVPFPERIKFIEENHENIMACAKSPLENTWWAEQDSPFCFLAFCFEYAGVQHHGLSYNCSLPLAFDGSCSGIQHFSAMLRDEVGGRAVNLLPSETVQDIYGIVAKKVNEILQADAINGTDNEVVTVTDENTGEISEKVKLGTKALAGQWLAYGVTRSVTKRSVMTLAYGSKEFGFRQQVLEDTIQPAIDSGKGLMFTQPNQAAGYMAKLIWESVSVTVVAAVEAMNWLKSAAKLLAAEVKDKKTGEILRKRCAVHWVTPDGFPVWQEYKKPIQTRLNLMFLGQFRLQPTINTNKDSEIDAHKQESGIAPNFVHSQDGSHLRKTVVWAHEKYGIESFALIHDSFGTIPADAANLFKAVRETMVDTYESCDVLADFYDQFADQLHESQLDKMPALPAKGNLNLRDILESDFAFA

SEQ ID NO: 11 - protein, 882 aa, synthetic construct
MNTINIAKNDFSDIELAAIPFNTLADHYGERLAREQLALEHESYEMGEARFRKMFERQLKAGEVADNAAAKPLITTLLPKMIARINDWFEEVKAKRGKRPTAFQFLQEIKPEAVAYITIKTTLACLTSADNTTVQAVASAIGRAIEDEARFGRIRDLEAKHFKKNVEEQLNRVGHVYKKAFMQVVEADMLSKGLLGGEAWSSWHKEDSIHVGVRCIEMLIESTGMVSLHRQNAGVVGQDSETIELAPEYAEAIATRAGALAGISPMFQPCVVPPKPWTGITGGGYWANGRRPLALVRTHSKKALMRYEDVYMPEVYKAINIAQNTAWKINKKVLAVANVITKWKHCPVEDIPAIEREELPMKPEDIDMNPEALTAWKRAAAAVYRKDKARKSRRISLEFMLEQANKFANHKAIWFPYNMDWRGRVYAVSMFNPQGNDMTKGLLTLAKGKPIGKEGYYWLKIHGANCAGVDKVPFPERIKFIEENHENIMACAKSPLENTWWAEQDSPFCFLAFCFEYAGVQHHGLSYNCSLPLAFDGSCSGIQHFSAMLRDEVGGRAVNLLPSETVQDIYGIVAKKVNEILQADAINGTDNEVVTVTDENTGEISEKVKLGTKALAGQWLAYGVTRSVTKRSVMTLAYGSKEFGFRQQVLEDTIQPAIDSGKGLMFTQPNQAAGYMAKLIWESVSVTVVAAVEAMNWLKSAAKLLAAEVKDKKTGEILRKRCAVHWVTPDGFPVWQEYKKPIQTRLNLMFLGQFRLQPTINTNKDSEIDAHKQESGIAPNFVHSQDGSHLRKTVVWAHEKYGIESFALIHDSFGTIPADAANLFKAVRETMVDTYESCDVLADFYDQFADQLHESQLDKMPALPAKGNLNLRDILESDFAFA

SEQ ID NO: 12 - protein, 883 aa, synthetic construct
MNTINIAKNDFSDIELAAIPFNTLADHYGERLAREQLALEHESYEMGEARFRKMFERQLKAGEVADNAAAKPLITTLLPKMIARINDWFEEVKAKRGKRPTAFQFLQEIKPEAVAYITIKTTLACLTSADNTTVQAVASAIGRAIEDEARFGRIRDLEAKHFKKNVEEQLNARVGHVYKKAFMQVVEADMLSKGLLGGEAWSSWHKEDSIHVGVRCIEMLIESTGMVSLHRQNAGVVGQDSETIELAPEYAEAIATRAGALAGISPMFQPCVVPPKPWTGITGGGYWANGRRPLALVRTHSKKALMRYEDVYMPEVYKAINIAQNTAWKINKKVLAVANVITKWKHCPVEDIPAIEREELPMKPEDIDMNPEALTAWKRAAAAVYRKDKARKSRRISLEFMLEQANKFANHKAIWFPYNMDWRGRVYAVSMFNPQGNDMTKGLLTLAKGKPIGKEGYYWLKIHGANCAGVDKVPFPERIKFIEENHENIMACAKSPLENTWWAEQDSPFCFLAFCFEYAGVQHHGLSYNCSLPLAFDGSCSGIQHFSAMLRDEVGGRAVNLLPSETVQDIYGIVAKKVNEILQADAINGTDNEVVTVTDENTGEISEKVKLGTKALAGQWLAYGVTRSVTKRSVMTLAYGSKEFGFRQQVLEDTIQPAIDSGKGLMFTQPNQAAGYMAKLIWESVSVTVVAAVEAMNWLKSAAKLLAAEVKDKKTGEILRKRCAVHWVTPDGFPVWQEYKKPIQTRLNLMFLGQFRLQPTINTNKDSEIDAHKQESGIAPNFVHSQDGSHLRKTVVWAHEKYGIESFALIHDSFGTIPADAANLFKAVRETMVDTYESCDVLADFYDQFADQLHESQLDKMPALPAKGNLNLRDILESDFAFA

SEQ ID NO: 13 - protein, 883 aa, synthetic construct
MNTINIAKNDFSDIELAAIPFNTLADHYGERLAREQLALEHESYEMGEARFRKMFERQLKAGEVADNAAAKPLITTLLPKMIARINDWFEEVKAKRGKRPTAFQFLQEIKPEAVAYITIKTTLACLTSADNTTVQAVASAIGRAIEDEARFGRIRDLEAKHFKKNVEEQLNGRVGHVYKKAFMQVVEADMLSKGLLGGEAWSSWHKEDSIHVGVRCIEMLIESTGMVSLHRQNAGVVGQDSETIELAPEYAEAIATRAGALAGISPMFQPCVVPPKPWTGITGGGYWANGRRPLALVRTHSKKALMRYEDVYMPEVYKAINIAQNTAWKINKKVLAVANVITKWKHCPVEDIPAIEREELPMKPEDIDMNPEALTAWKRAAAAVYRKDKARKSRRISLEFMLEQANKFANHKAIWFPYNMDWRGRVYAVSMFNPQGNDMTKGLLTLAKGKPIGKEGYYWLKIHGANCAGVDKVPFPERIKFIEENHENIMACAKSPLENTWWAEQDSPFCFLAFCFEYAGVQHHGLSYNCSLPLAFDGSCSGIQHFSAMLRDEVGGRAVNLLPSETVQDIYGIVAKKVNEILQADAINGTDNEVVTVTDENTGEISEKVKLGTKALAGQWLAYGVTRSVTKRSVMTLAYGSKEFGFRQQVLEDTIQPAIDSGKGLMFTQPNQAAGYMAKLIWESVSVTVVAAVEAMNWLKSAAKLLAAEVKDKKTGEILRKRCAVHWVTPDGFPVWQEYKKPIQTRLNLMFLGQFRLQPTINTNKDSEIDAHKQESGIAPNFVHSQDGSHLRKTVVWAHEKYGIESFALIHDSFGTIPADAANLFKAVRETMVDTYESCDVLADFYDQFADQLHESQLDKMPALPAKGNLNLRDILESDFAFA

SEQ ID NO: 14 - protein, 883 aa, synthetic construct
MNTINIAKNDFSDIELAAIPFNTLADHYGERLAREQLALEHESYEMGEARFRKMFERQLKAGEVADNAAAKPLITTLLPKMIARINDWFEEVKAKRGKRPTAFQFLQEIKPEAVAYITIKTTLACLTSADNTTVQAVASAIGRAIEDEARFGRIRDLEAKHFKKNVEEQLNPRVGHVYKKAFMQVVEADMLSKGLLGGEAWSSWHKEDSIHVGVRCIEMLIESTGMVSLHRQNAGVVGQDSETIELAPEYAEAIATRAGALAGISPMFQPCVVPPKPWTGITGGGYWANGRRPLALVRTHSKKALMRYEDVYMPEVYKAINIAQNTAWKINKKVLAVANVITKWKHCPVEDIPAIEREELPMKPEDIDMNPEALTAWKRAAAAVYRKDKARKSRRISLEFMLEQANKFANHKAIWFPYNMDWRGRVYAVSMFNPQGNDMTKGLLTLAKGKPIGKEGYYWLKIHGANCAGVDKVPFPERIKFIEENHENIMACAKSPLENTWWAEQDSPFCFLAFCFEYAGVQHHGLSYNCSLPLAFDGSCSGIQHFSAMLRDEVGGRAVNLLPSETVQDIYGIVAKKVNEILQADAINGTDNEVVTVTDENTGEISEKVKLGTKALAGQWLAYGVTRSVTKRSVMTLAYGSKEFGFRQQVLEDTIQPAIDSGKGLMFTQPNQAAGYMAKLIWESVSVTVVAAVEAMNWLKSAAKLLAAEVKDKKTGEILRKRCAVHWVTPDGFPVWQEYKKPIQTRLNLMFLGQFRLQPTINTNKDSEIDAHKQESGIAPNFVHSQDGSHLRKTVVWAHEKYGIESFALIHDSFGTIPADAANLFKAVRETMVDTYESCDVLADFYDQFADQLHESQLDKMPALPAKGNLNLRDILESDFAFA

SEQ ID NO: 15 - protein, 883 aa, synthetic construct
MNTINIAKNDFSDIELAAIPFNTLADHYGERLAREQLALEHESYEMGEARFRKMFERQLKAGEVADNAAAKPLITTLLPKMIARINDWFEEVKAKRGKRPTAFQFLQEIKPEAVAYITIKTTLACLTSADNTTVQAVASAIGRAIEDEARFGRIRDLEAKHFKKNVEEQDNKRVGHVYKKAFMQVVEADMLSKGLLGGEAWSSWHKEDSIHVGVRCIEMLIESTGMVSLHRQNAGVVGQDSETIELAPEYAEAIATRAGALAGISPMFQPCVVPPKPWTGITGGGYWANGRRPLALVRTHSKKALMRYEDVYMPEVYKAINIAQNTAWKINKKVLAVANVITKWKHCPVEDIPAIEREELPMKPEDIDMNPEALTAWKRAAAAVYRKDKARKSRRISLEFMLEQANKFANHKAIWFPYNMDWRGRVYAVSMFNPQGNDMTKGLLTLAKGKPIGKEGYYWLKIHGANCAGVDKVPFPERIKFIEENHENIMACAKSPLENTWWAEQDSPFCFLAFCFEYAGVQHHGLSYNCSLPLAFDGSCSGIQHFSAMLRDEVGGRAVNLLPSETVQDIYGIVAKKVNEILQADAINGTDNEVVTVTDENTGEISEKVKLGTKALAGQWLAYGVTRSVTKRSVMTLAYGSKEFGFRQQVLEDTIQPAIDSGKGLMFTQPNQAAGYMAKLIWESVSVTVVAAVEAMNWLKSAAKLLAAEVKDKKTGEILRKRCAVHWVTPDGFPVWQEYKKPIQTRLNLMFLGQFRLQPTINTNKDSEIDAHKQESGIAPNFVHSQDGSHLRKTVVWAHEKYGIESFALIHDSFGTIPADAANLFKAVRETMVDTYESCDVLADFYDQFADQLHESQLDKMPALPAKGNLNLRDILESDFAFA

SEQ ID NO: 16 - protein, 883 aa, synthetic construct
MNTINIAKNDFSDIELAAIPFNTLADHYGERLAREQLALEHESYEMGEARFRKMFERQAKAGEVADNAAAKPLITTLLPKMIARINDWFEEVKAKRGKRPTAFQFLQEIKPEAVAYITIKTTLACLTSADNTTVQAVASAIGRAIEDEARFGRIRDLEAKHFKKNVEEQLNKRVGHVYKKAFMQVVEADMLSKGLLGGEAWSSWHKEDSIHVGVRCIEMLIESTGMVSLHRQNAGVVGQDSETIELAPEYAEAIATRAGALAGISPMFQPCVVPPKPWTGITGGGYWANGRRPLALVRTHSKKALMRYEDVYMPEVYKAINIAQNTAWKINKKVLAVANVITKWKHCPVEDIPAIEREELPMKPEDIDMNPEALTAWKRAAAAVYRKDKARKSRRISLEFMLEQANKFANHKAIWFPYNMDWRGRVYAVSMFNPQGNDMTKGLLTLAKGKPIGKEGYYWLKIHGANCAGVDKVPFPERIKFIEENHENIMACAKSPLENTWWAEQDSPFCFLAFCFEYAGVQHHGLSYNCSLPLAFDGSCSGIQHFSAMLRDEVGGRAVNLLPSETVQDIYGIVAKKVNEILQADAINGTDNEVVTVTDENTGEISEKVKLGTKALAGQWLAYGVTRSVTKRSVMTLAYGSKEFGFRQQVLEDTIQPAIDSGKGLMFTQPNQAAGYMAKLIWESVSVTVVAAVEAMNWLKSAAKLLAAEVKDKKTGEILRKRCAVHWVTPDGFPVWQEYKKPIQTRLNLMFLGQFRLQPTINTNKDSEIDAHKQESGIAPNFVHSQDGSHLRKTVVWAHEKYGIESFALIHDSFGTIPADAANLFKAVRETMVDTYESCDVLADFYDQFADQLHESQLDKMPALPAKGNLNLRDILESDFAFA

SEQ ID NO: 17 - protein, 883 aa, synthetic construct
MNTINIAKNDFSDIELAAIPFNTLADHYGERLAREQLALEHESYEMGEARFRKMFERQLKAGEVADNAAAKPLITTLLPKMIARINDWFEEVKAKRGKRPTAFQFLQEIKPEAVAYITIKTTLACLTSADNTTVQAVASAIGRAIEDEARFGRIRDLEAKHFKKNVEEQLNKRVGHVPKKAFMQVVEADMLSKGLLGGEAWSSWHKEDSIHVGVRCIEMLIESTGMVSLHRQNAGVVGQDSETIELAPEYAEAIATRAGALAGISPMFQPCVVPPKPWTGITGGGYWANGRRPLALVRTHSKKALMRYEDVYMPEVYKAINIAQNTAWKINKKVLAVANVITKWKHCPVEDIPAIEREELPMKPEDIDMNPEALTAWKRAAAAVYRKDKARKSRRISLEFMLEQANKFANHKAIWFPYNMDWRGRVYAVSMFNPQGNDMTKGLLTLAKGKPIGKEGYYWLKIHGANCAGVDKVPFPERIKFIEENHENIMACAKSPLENTWWAEQDSPFCFLAFCFEYAGVQHHGLSYNCSLPLAFDGSCSGIQHFSAMLRDEVGGRAVNLLPSETVQDIYGIVAKKVNEILQADAINGTDNEVVTVTDENTGEISEKVKLGTKALAGQWLAYGVTRSVTKRSVMTLAYGSKEFGFRQQVLEDTIQPAIDSGKGLMFTQPNQAAGYMAKLIWESVSVTVVAAVEAMNWLKSAAKLLAAEVKDKKTGEILRKRCAVHWVTPDGFPVWQEYKKPIQTRLNLMFLGQFRLQPTINTNKDSEIDAHKQESGIAPNFVHSQDGSHLRKTVVWAHEKYGIESFALIHDSFGTIPADAANLFKAVRETMVDTYESCDVLADFYDQFADQLHESQLDKMPALPAKGNLNLRDILESDFAFA

SEQ ID NO: 18 - protein, 883 aa, synthetic construct
MNTINIAKNDFSDIELAAIPFNTLADHYGERLAREQLALEHESYEMGEARFRKMFERQLKAGEVADNAAAKPLITTLLPKMIARINDWFEEVKAKRGKRPTAFQFLQEIKPEAVAYITIKTTLACLTSADNTTVQAVASAIGRAIEDEARFGRIRDLEAKHFKKNVEEQLNKRVGHVGKKAFMQVVEADMLSKGLLGGEAWSSWHKEDSIHVGVRCIEMLIESTGMVSLHRQNAGVVGQDSETIELAPEYAEAIATRAGALAGISPMFQPCVVPPKPWTGITGGGYWANGRRPLALVRTHSKKALMRYEDVYMPEVYKAINIAQNTAWKINKKVLAVANVITKWKHCPVEDIPAIEREELPMKPEDIDMNPEALTAWKRAAAAVYRKDKARKSRRISLEFMLEQANKFANHKAIWFPYNMDWRGRVYAVSMFNPQGNDMTKGLLTLAKGKPIGKEGYYWLKIHGANCAGVDKVPFPERIKFIEENHENIMACAKSPLENTWWAEQDSPFCFLAFCFEYAGVQHHGLSYNCSLPLAFDGSCSGIQHFSAMLRDEVGGRAVNLLPSETVQDIYGIVAKKVNEILQADAINGTDNEVVTVTDENTGEISEKVKLGTKALAGQWLAYGVTRSVTKRSVMTLAYGSKEFGFRQQVLEDTIQPAIDSGKGLMFTQPNQAAGYMAKLIWESVSVTVVAAVEAMNWLKSAAKLLAAEVKDKKTGEILRKRCAVHWVTPDGFPVWQEYKKPIQTRLNLMFLGQFRLQPTINTNKDSEIDAHKQESGIAPNFVHSQDGSHLRKTVVWAHEKYGIESFALIHDSFGTIPADAANLFKAVRETMVDTYESCDVLADFYDQFADQLHESQLDKMPALPAKGNLNLRDILESDFAFA

SEQ ID NO: 19 - protein, 883 aa, synthetic construct
MNTINIAKNDFSDIELAAIPFNTLADHYGERLAREQLALEHESYEMGEARFRKMFERQLKAGEVADNAAAKPLITTLLPKMIARINDWFEEVKAKRGKRPTAFQFLQEIKPEAVAYITIKTTLACLTSADNTTVQAVASAIGRAIEDEARFGRIRDLEAKHFKKNVEEQLNKRVGHVYKKAFEQVVEADMLSKGLLGGEAWSSWHKEDSIHVGVRCIEMLIESTGMVSLHRQNAGVVGQDSETIELAPEYAEAIATRAGALAGISPMFQPCVVPPKPWTGITGGGYWANGRRPLALVRTHSKKALMRYEDVYMPEVYKAINIAQNTAWKINKKVLAVANVITKWKHCPVEDIPAIEREELPMKPEDIDMNPEALTAWKRAAAAVYRKDKARKSRRISLEFMLEQANKFANHKAIWFPYNMDWRGRVYAVSMFNPQGNDMTKGLLTLAKGKPIGKEGYYWLKIHGANCAGVDKVPFPERIKFIEENHENIMACAKSPLENTWWAEQDSPFCFLAFCFEYAGVQHHGLSYNCSLPLAFDGSCSGIQHFSAMLRDEVGGRAVNLLPSETVQDIYGIVAKKVNEILQADAINGTDNEVVTVTDENTGEISEKVKLGTKALAGQWLAYGVTRSVTKRSVMTLAYGSKEFGFRQQVLEDTIQPAIDSGKGLMFTQPNQAAGYMAKLIWESVSVTVVAAVEAMNWLKSAAKLLAAEVKDKKTGEILRKRCAVHWVTPDGFPVWQEYKKPIQTRLNLMFLGQFRLQPTINTNKDSEIDAHKQESGIAPNFVHSQDGSHLRKTVVWAHEKYGIESFALIHDSFGTIPADAANLFKAVRETMVDTYESCDVLADFYDQFADQLHESQLDKMPALPAKGNLNLRDILESDFAFA

SEQ ID NO: 20 - protein, 883 aa, synthetic construct
MNTINIAKNDFSDIELAAIPFNTLADHYGERLAREQLALEHESYEMGEARFAKMFERQLKAGEVADNAAAKPLITTLLPKMIARINDWFEEVKAKRGKRPTAFQFLQEIKPEAVAYITIKTTLACLTSADNTTVQAVASAIGRAIEDEARFGRIRDLEAKHFKKNVEEQLNKRVGHVYKKAFMQVVEADMLSKGLLGGEAWSSWHKEDSIHVGVRCIEMLIESTGMVSLHRQNAGVVGQDSETIELAPEYAEAIATRAGALAGISPMFQPCVVPPKPWTGITGGGYWANGRRPLALVRTHSKKALMRYEDVYMPEVYKAINIAQNTAWKINKKVLAVANVITKWKHCPVEDIPAIEREELPMKPEDIDMNPEALTAWKRAAAAVYRKDKARKSRRISLEFMLEQANKFANHKAIWFPYNMDWRGRVYAVSMFNPQGNDMTKGLLTLAKGKPIGKEGYYWLKIHGANCAGVDKVPFPERIKFIEENHENIMACAKSPLENTWWAEQDSPFCFLAFCFEYAGVQHHGLSYNCSLPLAFDGSCSGIQHFSAMLRDEVGGRAVNLLPSETVQDIYGIVAKKVNEILQADAINGTDNEVVTVTDENTGEISEKVKLGTKALAGQWLAYGVTRSVTKRSVMTLAYGSKEFGFRQQVLEDTIQPAIDSGKGLMFTQPNQAAGYMAKLIWESVSVTVVAAVEAMNWLKSAAKLLAAEVKDKKTGEILRKRCAVHWVTPDGFPVWQEYKKPIQTRLNLMFLGQFRLQPTINTNKDSEIDAHKQESGIAPNFVHSQDGSHLRKTVVWAHEKYGIESFALIHDSFGTIPADAANLFKAVRETMVDTYESCDVLADFYDQFADQLHESQLDKMPALPAKGNLNLRDILESDFAFA

SEQ ID NO: 21 - protein, 883 aa, synthetic construct
MNTINIAKNDFSDIELAAIPFNTLADHYGERLAREQLALEHESYEMGEARFRKMFERQLKAGEVADNAAAKPLITTLLPKMIARINDWFEEVKAKRGKRPTAFQFLQEIKPEAVAYITIKTTLACLTSADNTTVQAVASAIGRAIEDEARFGRIRDLEAKHFKKNVEEQLNKRVGHVHKKAFMQVVEADMLSKGLLGGEAWSSWHKEDSIHVGVRCIEMLIESTGMVSLHRQNAGVVGQDSETIELAPEYAEAIATRAGALAGISPMFQPCVVPPKPWTGITGGGYWANGRRPLALVRTHSKKALMRYEDVYMPEVYKAINIAQNTAWKINKKVLAVANVITKWKHCPVEDIPAIEREELPMKPEDIDMNPEALTAWKRAAAAVYRKDKARKSRRISLEFMLEQANKFANHKAIWFPYNMDWRGRVYAVSMFNPQGNDMTKGLLTLAKGKPIGKEGYYWLKIHGANCAGVDKVPFPERIKFIEENHENIMACAKSPLENTWWAEQDSPFCFLAFCFEYAGVQHHGLSYNCSLPLAFDGSCSGIQHFSAMLRDEVGGRAVNLLPSETVQDIYGIVAKKVNEILQADAINGTDNEVVTVTDENTGEISEKVKLGTKALAGQWLAYGVTRSVTKRSVMTLAYGSKEFGFRQQVLEDTIQPAIDSGKGLMFTQPNQAAGYMAKLIWESVSVTVVAAVEAMNWLKSAAKLLAAEVKDKKTGEILRKRCAVHWVTPDGFPVWQEYKKPIQTRLNLMFLGQFRLQPTINTNKDSEIDAHKQESGIAPNFVHSQDGSHLRKTVVWAHEKYGIESFALIHDSFGTIPADAANLFKAVRETMVDTYESCDVLADFYDQFADQLHESQLDKMPALPAKGNLNLRDILESDFAFA

SEQ ID NO: 22 - protein, 883 aa, synthetic construct
MNTINIAKNDFSDIELAAIPFNTLADHYGERLAREQLALEHESYEMGEARFRKMFERQLKAGEVADNAAAKPLITTLLPKMIARINDWFEEVKAKRGKRPTAFQFLQEIKPEAVAYITIKTTLACLTSADNTTVQAVASAIGRAIEDEARFGRIRDLEAKHFKKNVEEQLNKRVGHVYKKAFMQVVDADMLSKGLLGGEAWSSWHKEDSIHVGVRCIEMLIESTGMVSLHRQNAGVVGQDSETIELAPEYAEAIATRAGALAGISPMFQPCVVPPKPWTGITGGGYWANGRRPLALVRTHSKKALMRYEDVYMPEVYKAINIAQNTAWKINKKVLAVANVITKWKHCPVEDIPAIEREELPMKPEDIDMNPEALTAWKRAAAAVYRKDKARKSRRISLEFMLEQANKFANHKAIWFPYNMDWRGRVYAVSMFNPQGNDMTKGLLTLAKGKPIGKEGYYWLKIHGANCAGVDKVPFPERIKFIEENHENIMACAKSPLENTWWAEQDSPFCFLAFCFEYAGVQHHGLSYNCSLPLAFDGSCSGIQHFSAMLRDEVGGRAVNLLPSETVQDIYGIVAKKVNEILQADAINGTDNEVVTVTDENTGEISEKVKLGTKALAGQWLAYGVTRSVTKRSVMTLAYGSKEFGFRQQVLEDTIQPAIDSGKGLMFTQPNQAAGYMAKLIWESVSVTVVAAVEAMNWLKSAAKLLAAEVKDKKTGEILRKRCAVHWVTPDGFPVWQEYKKPIQTRLNLMFLGQFRLQPTINTNKDSEIDAHKQESGIAPNFVHSQDGSHLRKTVVWAHEKYGIESFALIHDSFGTIPADAANLFKAVRETMVDTYESCDVLADFYDQFADQLHESQLDKMPALPAKGNLNLRDILESDFAFA

SEQ ID NO: 23 - protein, 883 aa, synthetic construct
MNTINIAKNDFSDIELAAIPFNTLADHYGERLAREQLALEHESYEMGEARFRKMFERQLKAGEVADNAAAKPLITTLLPKMIARINDWFEEVKAKRGKRPTAFQFLQEIKPEAVAYITIKTTLACLTSADNTTVQAVASAIGRAIEDEARFGRIRDLEAKHFKKNVEEQLNKRVGHVYKKAFMQVVEADMLSKGLLGGEAWSSWHKEDSIHVGVRCIEMLIESTGMVSLHRQNAGVVGQDSETIELAPEYAEAIATRAGALAGISPMFQPCVVPPKPWTGITGGGYWANGRRPLALVRTHSKKALMRYEDVYMPEVYKAINIAQNTAWKINKKVLAVANVITKWKHCPVEDIPAIEREELPMKPEDIDMNPEALTAWKRAAAAVYRKDKARKSRRISLEFMLEQANKFANHKAIWFPYNMDWRGRVYAVSMFNPQGNDMTKGLLTFAKGKPIGKEGYYWLKIHGANCAGVDKVPFPERIKFIEENHENIMACAKSPLENTWWAEQDSPFCFLAFCFEYAGVQHHGLSYNCSLPLAFDGSCSGIQHFSAMLRDEVGGRAVNLLPSETVQDIYGIVAKKVNEILQADAINGTDNEVVTVTDENTGEISEKVKLGTKALAGQWLAYGVTRSVTKRSVMTLAYGSKEFGFRQQVLEDTIQPAIDSGKGLMFTQPNQAAGYMAKLIWESVSVTVVAAVEAMNWLKSAAKLLAAEVKDKKTGEILRKRCAVHWVTPDGFPVWQEYKKPIQTRLNLMFLGQFRLQPTINTNKDSEIDAHKQESGIAPNFVHSQDGSHLRKTVVWAHEKYGIESFALIHDSFGTIPADAANLFKAVRETMVDTYESCDVLADFYDQFADQLHESQLDKMPALPAKGNLNLRDILESDFAFA

SEQ ID NO: 24 - protein, 883 aa, synthetic construct
MNTINIAKNDFSDIELAAIPFNTLADHYGERLAREQLALEHESYEMGEARFRKMFERQLKAGEVADNAAAKPLITTLLPKMIARINDWFEEVKAKRGKRPTAFQFLQEIKPEAVAYITIKTTLACLTSADNTTVQAVASAIGRAIEDEARFGRIRDLEAKHFKKNVEEQLNKRVGHVYKKAFMQVVEADMLSKGLLGGEAWSSWHKEDSIHVGVRCIEMLIESTGMVSLHRQNAGVVGQDSETIELAPEYAEAIATRAGALAGISPMFQPCVVPPKPWTGITGGGYWANGRRPLALVRTHSKKALMRYEDVYMPEVYKAINIAQNTAWKINKKVLAVANVITKWKHCPVEDIPAIEREELPMKPEDIDMNPEALTAWKRAAAAVYRSDKARKSRRISLEFMLEQANKFANHKAIWFPYNMDWRGRVYAVSMFNPQGNDMTKGLLTLAKGKPIGKEGYYWLKIHGANCAGVDKVPFPERIKFIEENHENIMACAKSPLENTWWAEQDSPFCFLAFCFEYAGVQHHGLSYNCSLPLAFDGSCSGIQHFSAMLRDEVGGRAVNLLPSETVQDIYGIVAKKVNEILQADAINGTDNEVVTVTDENTGEISEKVKLGTKALAGQWLAYGVTRSVTKRSVMTLAYGSKEFGFRQQVLEDTIQPAIDSGKGLMFTQPNQAAGYMAKLIWESVSVTVVAAVEAMNWLKSAAKLLAAEVKDKKTGEILRKRCAVHWVTPDGFPVWQEYKKPIQTRLNLMFLGQFRLQPTINTNKDSEIDAHKQESGIAPNFVHSQDGSHLRKTVVWAHEKYGIESFALIHDSFGTIPADAANLFKAVRETMVDTYESCDVLADFYDQFADQLHESQLDKMPALPAKGNLNLRDILESDFAFA

SEQ ID NO: 25 - protein, 883 aa, synthetic construct
MNTINIAKNDFSDIELAAIPFNTLADHYGERLAREQLALEHESYEMGEARFRKMFERQLKAGEVADNAAAKPLITTLLPKMIARINDWFEEVKAKRGKRPTAFQFLQEIKPEAVAYITIKTTLACLTSADNTTVQAVASAIGRAIEDEARFGRIRDLEAKHFKKNVEEQLNKRVGHVYKKAFMQVVEADMLSKGLLGGEAWSSWHKEDSIHVGVRCIEMLIESTGMVSLHRQNAGVVGQDSETIELAPEYAEAIATRAGALAGISPMFQPCVVPPKPWTGITGGGYWANGRRPLALVRTHSKKALMRYEDVYMPEVYKAINIAQNTAWKINKKVLAVANVITKWKHCPVEDIPAIEREELPMKPEDIDMNPEALTAWKRAAAAVYRKDAARKSRRISLEFMLEQANKFANHKAIWFPYNMDWRGRVYAVSMFNPQGNDMTKGLLTLAKGKPIGKEGYYWLKIHGANCAGVDKVPFPERIKFIEENHENIMACAKSPLENTWWAEQDSPFCFLAFCFEYAGVQHHGLSYNCSLPLAFDGSCSGIQHFSAMLRDEVGGRAVNLLPSETVQDIYGIVAKKVNEILQADAINGTDNEVVTVTDENTGEISEKVKLGTKALAGQWLAYGVTRSVTKRSVMTLAYGSKEFGFRQQVLEDTIQPAIDSGKGLMFTQPNQAAGYMAKLIWESVSVTVVAAVEAMNWLKSAAKLLAAEVKDKKTGEILRKRCAVHWVTPDGFPVWQEYKKPIQTRLNLMFLGQFRLQPTINTNKDSEIDAHKQESGIAPNFVHSQDGSHLRKTVVWAHEKYGIESFALIHDSFGTIPADAANLFKAVRETMVDTYESCDVLADFYDQFADQLHESQLDKMPALPAKGNLNLRDILESDFAFA

SEQ ID NO: 26 - protein, 883 aa, synthetic construct
MNTINIAKNDFSDIELAAIPFNTLADHYGERLAREQLALEHESYEMGEARFRKMFERQLKAGEVADNAAAKPLITTLLPKMIARINDWFEEVKAKRGKRPTAFQFLQEIKPEAVAYITIKTTLACLTSADNTTVQAVASAIGRAIEDEARFGRIRDLEAKHFKKNVEEQLNKRVGHVYKKAFMQVVEADMLSKGLLGGEAWSSWHKEDSIHVGVRCIEMLIESTGMVSLHRQNAGVVGQDSETIELAPEYAEAIATRAGALAGISPMFQPCVVPPKPWTGITGGGYWANGRRPLALVRTHSKKALMRYEDVYMPEVYKAINIAQNTAWKINKKVLAVANVITKWKHCPVEDIPAIEREELPMKPEDIDMNPEALTAWKRAAAAVYRKDKARKSRRISLEFMLEQANKFANHKAIWFPYNMDWRGRVYAVSMFNPQGNDMTKGLLTLAKGKPIGKEGYYWLKIHGANCAGVDKVPFPERIKFIEENHENIMACAKSPLENTWWAEQDSPFCFLAFCFEYAGVQHHGLSYNSSLPLAFDGSCSGIQHFSAMLRDEVGGRAVNLLPSETVQDIYGIVAKKVNEILQADAINGTDNEVVTVTDENTGEISEKVKLGTKALAGQWLAYGVTRSVTKRSVMTLAYGSKEFGFRQQVLEDTIQPAIDSGKGLMFTQPNQAAGYMAKLIWESVSVTVVAAVEAMNWLKSAAKLLAAEVKDKKTGEILRKRCAVHWVTPDGFPVWQEYKKPIQTRLNLMFLGQFRLQPTINTNKDSEIDAHKQESGIAPNFVHSQDGSHLRKTVVWAHEKYGIESFALIHDSFGTIPADAANLFKAVRETMVDTYESCDVLADFYDQFADQLHESQLDKMPALPAKGNLNLRDILESDFAFA

SEQ ID NO: 27 - protein, 883 aa, synthetic construct
MNTINIAKNDFSDIELAAIPFNTLADHYGERLAREQLALEHESYEMGEARFRKMFERQLKAGEVADNAAAKPLITTLLPKMIARINDWFEEVKAKRGKRPTAFQFLQEIKPEAVAYITIKTTLACLTSADNTTVQAVASAIGRAIEDEARFGRIRDLEAKHFKKNVEEQLNKRVGHVYKKAFMQVVEADMLSKGLLGGEAWSSWHKEDSIHVGVRCIEMLIESTGMVSLHRQNAGVVGQDSETIELAPEYAEAIATRAGALAGISPMFQPCVVPPKPWTGITGGGYWANGRRPLALVRTHSKKALMRYEDVYMPEVYKAINIAQNTAWKINKKVLAVANVITKWKHCPVEDIPAIEREELPMKPEDIDMNPEALTAWKRAAAAVYRKDKARKSRRISLEFMLEQANKFANHKAIWFPYNMDWRGRVYAVSMFNPQGNDMTKGLLTLAKGKPIGKEGYYWLKIHGANCAGVDKVPFPERIKFIEENHENIMACAKSPLENTWWAEQDSPFCFLAFCFEYAGVQHHGLSYNCSLPLAFDGSCSGIQHFSAMLRDEVGGRAVNLLPSETVQDIYGIVAKKVNEILQADAINGTDNEVVTVTDENTGEISEKVKLGTKALAGQWLAYGVTRSVTKRSVMTLAYGSKEFGFRQQVLEDTIQPAIDSGKGLMFTQPNQAAGYMAKLIWESVSVTVVAAVEAMNWLKSAAKLLAAEVKDKKTGEILRKRCAVHWVTPDGFPVWQEYKKPIQTRLNLMFLGQFRLQPTINTNKDSEIDAHKQESGIAPNFVHSQDGSHLRKTVVWAHEKYGIESFALIHDSFGTIPADAANLFKAVRETMVDTYESCDVLADFYDQFADQLHESQLDKMPALPAKGNLDLRDILESDFAFA

SEQ ID NO: 28 - protein, 881 aa, synthetic construct
MNTINIAKNDFSDIELAAIPFNTLADHYGERLAREQLALEHESYEMGEARFRKMFERQLKAGEVADNAAAKPLITTLLPKMIARINDWFEEVKAKRGKRPTAFQFLQEIKPEAVAYITIKTTLACLTSADNTTVQAVASAIGRAIEDEARFGRIRDLEAKHFKKNVEEQLNVGHVYKKAFMQVVEADMLSKGLLGGEAWSSWHKEDSIHVGVRCIEMLIESTGMVSLHRQNAGVVGQDSETIELAPEYAEAIATRAGALAGISPMFQPCVVPPKPWTGITGGGYWANGRRPLALVRTHSKKALMRYEDVYMPEVYKAINIAQNTAWKINKKVLAVANVITKWKHCPVEDIPAIEREELPMKPEDIDMNPEALTAWKRAAAAVYRKDKARKSRRISLEFMLEQANKFANHKAIWFPYNMDWRGRVYAVSMFNPQGNDMTKGLLTLAKGKPIGKEGYYWLKIHGANCAGVDKVPFPERIKFIEENHENIMACAKSPLENTWWAEQDSPFCFLAFCFEYAGVQHHGLSYNCSLPLAFDGSCSGIQHFSAMLRDEVGGRAVNLLPSETVQDIYGIVAKKVNEILQADAINGTDNEVVTVTDENTGEISEKVKLGTKALAGQWLAYGVTRSVTKRSVMTLAYGSKEFGFRQQVLEDTIQPAIDSGKGLMFTQPNQAAGYMAKLIWESVSVTVVAAVEAMNWLKSAAKLLAAEVKDKKTGEILRKRCAVHWVTPDGFPVWQEYKKPIQTRLNLMFLGQFRLQPTINTNKDSEIDAHKQESGIAPNFVHSQDGSHLRKTVVWAHEKYGIESFALIHDSFGTIPADAANLFKAVRETMVDTYESCDVLADFYDQFADQLHESQLDKMPALPAKGNLNLRDILESDFAFA

SEQ ID NO: 29 - protein, 883 aa, synthetic construct
MNTINIAKNDFSDIELAAIPFNTLADHYGERLAREQLALEHESYEMGEARFRKMFERQLKAGEVADNAAAKPLITTLLPKMIARINDWFEEVKAKRGKRPTAFQFLQEIKPEAVAYITIKTTLACLTSADNTTVQAVASAIGRAIEDEARFGRIRDLEAKHFKKNVEEQLNAGVGHVYKKAFMQVVEADMLSKGLLGGEAWSSWHKEDSIHVGVRCIEMLIESTGMVSLHRQNAGVVGQDSETIELAPEYAEAIATRAGALAGISPMFQPCVVPPKPWTGITGGGYWANGRRPLALVRTHSKKALMRYEDVYMPEVYKAINIAQNTAWKINKKVLAVANVITKWKHCPVEDIPAIEREELPMKPEDIDMNPEALTAWKRAAAAVYRKDKARKSRRISLEFMLEQANKFANHKAIWFPYNMDWRGRVYAVSMFNPQGNDMTKGLLTLAKGKPIGKEGYYWLKIHGANCAGVDKVPFPERIKFIEENHENIMACAKSPLENTWWAEQDSPFCFLAFCFEYAGVQHHGLSYNCSLPLAFDGSCSGIQHFSAMLRDEVGGRAVNLLPSETVQDIYGIVAKKVNEILQADAINGTDNEVVTVTDENTGEISEKVKLGTKALAGQWLAYGVTRSVTKRSVMTLAYGSKEFGFRQQVLEDTIQPAIDSGKGLMFTQPNQAAGYMAKLIWESVSVTVVAAVEAMNWLKSAAKLLAAEVKDKKTGEILRKRCAVHWVTPDGFPVWQEYKKPIQTRLNLMFLGQFRLQPTINTNKDSEIDAHKQESGIAPNFVHSQDGSHLRKTVVWAHEKYGIESFALIHDSFGTIPADAANLFKAVRETMVDTYESCDVLADFYDQFADQLHESQLDKMPALPAKGNLNLRDILESDFAFA

SEQ ID NO: 30 - protein, 883 aa, synthetic construct
MNTINIAKNDFSDIELAAIPFNTLADHYGERLAREQLALEHESYEMGEARFRKMFERQLKAGEVADNAAAKPLITTLLPKMIARINDWFEEVKAKRGKRPTAFQFLQEIKPEAVAYITIKTTLACLTSADNTTVQAVASAIGRAIEDEARFGRIRDLEAKHFKKNVEEQLNAGVGHVYKKAFMQVVEADMLSKGLLGGEAWSSWHKEDSIHVGVRCIEMLIESTGMVSLHRQNAGVVGQDSETIELAPEYAEAIATRAGALAGISPMFQPCVVPPKPWTGITGGGYWANGRRPLALVRTHSKKALMRYEDVYMPEVYKAINIAQNTAWKINKKVLAVANVITKWKHCPVEDIPAIEREELPMKPEDIDMNPEALTAWKRAAAAVYRYDKARKSRRISLEFMLEQANKFANHKAIWFPYNMDWRGRVYAVSMFNPQGNDMTKGLLTLAKGKPIGKEGYYWLKIHGANCAGVDKVPFPERIKFIEENHENIMACAKSPLENTWWAEQDSPFCFLAFCFEYAGVQHHGLSYNCSLPLAFDGSCSGIQHFSAMLRDEVGGRAVNLLPSETVQDIYGIVAKKVNEILQADAINGTDNEVVTVTDENTGEISEKVKLGTKALAGQWLAYGVTRSVTKRSVMTLAYGSKEFGFRQQVLEDTIQPAIDSGKGLMFTQPNQAAGYMAKLIWESVSVTVVAAVEAMNWLKSAAKLLAAEVKDKKTGEILRKRCAVHWVTPDGFPVWQEYKKPIQTRLNLMFLGQFRLQPTINTNKDSEIDAHKQESGIAPNFVHSQDGSHLRKTVVWAHEKYGIESFALIHDSFGTIPADAANLFKAVRETMVDTYESCDVLADFYDQFADQLHESQLDKMPALPAKGNLNLRDILESDFAFA

SEQ ID NO: 31 - protein, 883 aa, synthetic construct
MNTINIAKNDFSDIELAAIPFNTLADHYGERLAREQLALEHESYEMGEARFRKMFERQLKAGEVADNAAAKPLITTLLPKMIARINDWFEEVKAKRGKRPTAFQFLQEIKPEAVAYITIKTTLACLTSADNTTVQAVASAIGRAIEDEARFGRIRDLEAKHFKKNVEEQLNAGVGHVYKKAFMQVVEADMLSKGLLGGEAWSSWHKEDSIHVGVRCIEMLIESTGMVSLHRQNAGVVGQDSETIELAPEYAEAIATRAGALAGISPMFQPCVVPPKPWTGITGGGYWANGRRPLALVRTHSKKALMRYEDVYMPEVYKAINIAQNTAWKINKKVLAVANVITKWKHCPVEDIPAIEREELPMKPEDIDMNPEALTAWKRAAAAVYRSDKARKSRRISLEFMLEQANKFANHKAIWFPYNMDWRGRVYAVSMFNPQGNDMTKGLLTLAKGKPIGKEGYYWLKIHGANCAGVDKVPFPERIKFIEENHENIMACAKSPLENTWWAEQDSPFCFLAFCFEYAGVQHHGLSYNCSLPLAFDGSCSGIQHFSAMLRDEVGGRAVNLLPSETVQDIYGIVAKKVNEILQADAINGTDNEVVTVTDENTGEISEKVKLGTKALAGQWLAYGVTRSVTKRSVMTLAYGSKEFGFRQQVLEDTIQPAIDSGKGLMFTQPNQAAGYMAKLIWESVSVTVVAAVEAMNWLKSAAKLLAAEVKDKKTGEILRKRCAVHWVTPDGFPVWQEYKKPIQTRLNLMFLGQFRLQPTINTNKDSEIDAHKQESGIAPNFVHSQDGSHLRKTVVWAHEKYGIESFALIHDSFGTIPADAANLFKAVRETMVDTYESCDVLADFYDQFADQLHESQLDKMPALPAKGNLNLRDILESDFAFA

SEQ ID NO: 32 - protein, 882 aa, synthetic construct
MNTINIAKNDFSDIELAAIPFNTLADHYGERLAREQLALEHESYEMGEARFRKMFERQLKAGEVADNAAAKPLITTLLPKMIARINDWFEEVKAKRGKRPTAFQFLQEIKPEAVAYITIKTTLACLTSADNTTVQAVASAIGRAIEDEARFGRIRDLEAKHFKKNVDEQLNRVGHVYKKAFMQVVEADMLSKGLLGGEAWSSWHKEDSIHVGVRCIEMLIESTGMVSLHRQNAGVVGQDSETIELAPEYAEAIATRAGALAGISPMFQPCVVPPKPWTGITGGGYWANGRRPLALVRTHSKKALMRYEDVYMPEVYKAINIAQNTAWKINKKVLAVANVITKWKHCPVEDIPAIEREELPMKPEDIDMNPEALTAWKRAAAAVYRKDKARKSRRISLEFMLEQANKFANHKAIWFPYNMDWRGRVYAVSMFNPQGNDMTKGLLTLAKGKPIGKEGYYWLKIHGANCAGVDKVPFPERIKFIEENHENIMACAKSPLENTWWAEQDSPFCFLAFCFEYAGVQHHGLSYNCSLPLAFDGSCSGIQHFSAMLRDEVGGRAVNLLPSETVQDIYGIVAKKVNEILQADAINGTDNEVVTVTDENTGEISEKVKLGTKALAGQWLAYGVTRSVTKRSVMTLAYGSKEFGFRQQVLEDTIQPAIDSGKGLMFTQPNQAAGYMAKLIWESVSVTVVAAVEAMNWLKSAAKLLAAEVKDKKTGEILRKRCAVHWVTPDGFPVWQEYKKPIQTRLNLMFLGQFRLQPTINTNKDSEIDAHKQESGIAPNFVHSQDGSHLRKTVVWAHEKYGIESFALIHDSFGTIPADAANLFKAVRETMVDTYESCDVLADFYDQFADQLHESQLDKMPALPAKGNLNLRDILESDFAFA

SEQ ID NO: 33 - protein, 881 aa, synthetic construct
MNTINIAKNDFSDIELAAIPFNTLADHYGERLAREQLALEHESYEMGEARFRKMFERQLKAGEVADNAAAKPLITTLLPKMIARINDWFEEVKAKRGKRPTAFQFLQEIKPEAVAYITIKTTLACLTSADNTTVQAVASAIGRAIEDEARFGRIRDLEAKHFKKNVEDQLNVGHVYKKAFMQVVEADMLSKGLLGGEAWSSWHKEDSIHVGVRCIEMLIESTGMVSLHRQNAGVVGQDSETIELAPEYAEAIATRAGALAGISPMFQPCVVPPKPWTGITGGGYWANGRRPLALVRTHSKKALMRYEDVYMPEVYKAINIAQNTAWKINKKVLAVANVITKWKHCPVEDIPAIEREELPMKPEDIDMNPEALTAWKRAAAAVYRKDKARKSRRISLEFMLEQANKFANHKAIWFPYNMDWRGRVYAVSMFNPQGNDMTKGLLTLAKGKPIGKEGYYWLKIHGANCAGVDKVPFPERIKFIEENHENIMACAKSPLENTWWAEQDSPFCFLAFCFEYAGVQHHGLSYNCSLPLAFDGSCSGIQHFSAMLRDEVGGRAVNLLPSETVQDIYGIVAKKVNEILQADAINGTDNEVVTVTDENTGEISEKVKLGTKALAGQWLAYGVTRSVTKRSVMTLAYGSKEFGFRQQVLEDTIQPAIDSGKGLMFTQPNQAAGYMAKLIWESVSVTVVAAVEAMNWLKSAAKLLAAEVKDKKTGEILRKRCAVHWVTPDGFPVWQEYKKPIQTRLNLMFLGQFRLQPTINTNKDSEIDAHKQESGIAPNFVHSQDGSHLRKTVVWAHEKYGIESFALIHDSFGTIPADAANLFKAVRETMVDTYESCDVLADFYDQFADQLHESQLDKMPALPAKGNLNLRDILESDFAFA

SEQ ID NO: 34 - protein, 881 aa, synthetic construct
MNTINIAKNDFSDIELAAIPFNTLADHYGERLAREQLALEHESYEMGEARFRKMFERQLKAGEVADNAAAKPLITTLLPKMIARINDWFEEVKAKRGKRPTAFQFLQEIKPEAVAYITIKTTLACLTSADNTTVQAVASAIGRAIEDEARFGRIRDLEAKHFKKNVEEQLNVGHVYKKAFMQVVEADMLSKGLLGGEAWSSWHKEDSIHVGVRCIEMLIESTGMVSLHRQNAGVVGQDSETIELAPEYAEAIATRAGALAGISPMFQPCVVPPKPWTGITGGGYWANGRRPLALVRTHSKKALMRYEDVYMPEVYKAINIAQNTAWKINKKVLAVANVITKWKHCPVEDIPAIEREELPMKPEDIDMNPEALTAWKRAAAAVYRSDKARKSRRISLEFMLEQANKFANHKAIWFPYNMDWRGRVYAVSMFNPQGNDMTKGLLTLAKGKPIGKEGYYWLKIHGANCAGVDKVPFPERIKFIEENHENIMACAKSPLENTWWAEQDSPFCFLAFCFEYAGVQHHGLSYNCSLPLAFDGSCSGIQHFSAMLRDEVGGRAVNLLPSETVQDIYGIVAKKVNEILQADAINGTDNEVVTVTDENTGEISEKVKLGTKALAGQWLAYGVTRSVTKRSVMTLAYGSKEFGFRQQVLEDTIQPAIDSGKGLMFTQPNQAAGYMAKLIWESVSVTVVAAVEAMNWLKSAAKLLAAEVKDKKTGEILRKRCAVHWVTPDGFPVWQEYKKPIQTRLNLMFLGQFRLQPTINTNKDSEIDAHKQESGIAPNFVHSQDGSHLRKTVVWAHEKYGIESFALIHDSFGTIPADAANLFKAVRETMVDTYESCDVLADFYDQFADQLHESQLDKMPALPAKGNLNLRDILESDFAFA

SEQ ID NO: 35 - protein, 881 aa, synthetic construct
MNTINIAKNDFSDIELAAIPFNTLADHYGERLAREQLALEHESYEMGEARFRKMFERQLKAGEVADNAAAKPLITTLLPKMIARINDWFEEVKAKRGKRPTAFQFLQEIKPEAVAYITIKTTLACLTSADNTTVQAVASAIGRAIEDEARFGRIRDLEAKHFKKNVEEQLNVGHVGKKAFMQVVEADMLSKGLLGGEAWSSWHKEDSIHVGVRCIEMLIESTGMVSLHRQNAGVVGQDSETIELAPEYAEAIATRAGALAGISPMFQPCVVPPKPWTGITGGGYWANGRRPLALVRTHSKKALMRYEDVYMPEVYKAINIAQNTAWKINKKVLAVANVITKWKHCPVEDIPAIEREELPMKPEDIDMNPEALTAWKRAAAAVYRKDKARKSRRISLEFMLEQANKFANHKAIWFPYNMDWRGRVYAVSMFNPQGNDMTKGLLTLAKGKPIGKEGYYWLKIHGANCAGVDKVPFPERIKFIEENHENIMACAKSPLENTWWAEQDSPFCFLAFCFEYAGVQHHGLSYNCSLPLAFDGSCSGIQHFSAMLRDEVGGRAVNLLPSETVQDIYGIVAKKVNEILQADAINGTDNEVVTVTDENTGEISEKVKLGTKALAGQWLAYGVTRSVTKRSVMTLAYGSKEFGFRQQVLEDTIQPAIDSGKGLMFTQPNQAAGYMAKLIWESVSVTVVAAVEAMNWLKSAAKLLAAEVKDKKTGEILRKRCAVHWVTPDGFPVWQEYKKPIQTRLNLMFLGQFRLQPTINTNKDSEIDAHKQESGIAPNFVHSQDGSHLRKTVVWAHEKYGIESFALIHDSFGTIPADAANLFKAVRETMVDTYESCDVLADFYDQFADQLHESQLDKMPALPAKGNLNLRDILESDFAFA

SEQ ID NO: 36 - protein, 881 aa, synthetic construct
MNTINIAKNDFSDIELAAIPFNTLADHYGERLAREQLALEHESYEMGEARFRKMFERQLKAGEVADNAAAKPLITTLLPKMIARINDWFEEVKAKRGKRPTAFQFLQEIKPEAVAYITIKTTLACLTSADNTTVQAVASAIGRAIEDEARFGRIRDLEAKHFKKNVEEQLNVGHVPKKAFMQVVEADMLSKGLLGGEAWSSWHKEDSIHVGVRCIEMLIESTGMVSLHRQNAGVVGQDSETIELAPEYAEAIATRAGALAGISPMFQPCVVPPKPWTGITGGGYWANGRRPLALVRTHSKKALMRYEDVYMPEVYKAINIAQNTAWKINKKVLAVANVITKWKHCPVEDIPAIEREELPMKPEDIDMNPEALTAWKRAAAAVYRKDKARKSRRISLEFMLEQANKFANHKAIWFPYNMDWRGRVYAVSMFNPQGNDMTKGLLTLAKGKPIGKEGYYWLKIHGANCAGVDKVPFPERIKFIEENHENIMACAKSPLENTWWAEQDSPFCFLAFCFEYAGVQHHGLSYNCSLPLAFDGSCSGIQHFSAMLRDEVGGRAVNLLPSETVQDIYGIVAKKVNEILQADAINGTDNEVVTVTDENTGEISEKVKLGTKALAGQWLAYGVTRSVTKRSVMTLAYGSKEFGFRQQVLEDTIQPAIDSGKGLMFTQPNQAAGYMAKLIWESVSVTVVAAVEAMNWLKSAAKLLAAEVKDKKTGEILRKRCAVHWVTPDGFPVWQEYKKPIQTRLNLMFLGQFRLQPTINTNKDSEIDAHKQESGIAPNFVHSQDGSHLRKTVVWAHEKYGIESFALIHDSFGTIPADAANLFKAVRETMVDTYESCDVLADFYDQFADQLHESQLDKMPALPAKGNLNLRDILESDFAFA

SEQ ID NO: 37 - protein, 883 aa, synthetic construct
MNTINIAKNDFSDIELAAIPFNTLADHYGERLAREQLALEHESYEMGEARFRKMGERQLKAGEVADNAAAKPLITTLLPKMIARINDWFEEVKAKRGKRPTAFQFLQEIKPEAVAYITIKTTLACLTSADNTTVQAVASAIGRAIEDEARFGRIRDLEAKHFKKNVEEQLNKRVGHVHKKAFMQVVEADMLSKGLLGGEAWSSWHKEDSIHVGVRCIEMLIESTGMVSLHRQNAGVVGQDSETIELAPEYAEAIATRAGALAGISPMFQPCVVPPKPWTGITGGGYWANGRRPLALVRTHSKKALMRYEDVYMPEVYKAINIAQNTAWKINKKVLAVANVITKWKHCPVEDIPAIEREELPMKPEDIDMNPEALTAWKRAAAAVYRKDKARKSRRISLEFMLEQANKFANHKAIWFPYNMDWRGRVYAVSMFNPQGNDMTKGLLTLAKGKPIGKEGYYWLKIHGANCAGVDKVPFPERIKFIEENHENIMACAKSPLENTWWAEQDSPFCFLAFCFEYAGVQHHGLSYNCSLPLAFDGSCSGIQHFSAMLRDEVGGRAVNLLPSETVQDIYGIVAKKVNEILQADAINGTDNEVVTVTDENTGEISEKVKLGTKALAGQWLAYGVTRSVTKRSVMTLAYGSKEFGFRQQVLEDTIQPAIDSGKGLMFTQPNQAAGYMAKLIWESVSVTVVAAVEAMNWLKSAAKLLAAEVKDKKTGEILRKRCAVHWVTPDGFPVWQEYKKPIQTRLNLMFLGQFRLQPTINTNKDSEIDAHKQESGIAPNFVHSQDGSHLRKTVVWAHEKYGIESFALIHDSFGTIPADAANLFKAVRETMVDTYESCDVLADFYDQFADQLHESQLDKMPALPAKGNLNLRDILESDFAFA

SEQ ID NO: 38 - protein, 883 aa, synthetic construct
MNTINIAKNDFSDIELAAIPFNTLADHYGERLAREQLALEHESYEMGEARFRKMLERQLKAGEVADNAAAKPLITTLLPKMIARINDWFEEVKAKRGKRPTAFQFLQEIKPEAVAYITIKTTLACLTSADNTTVQAVASAIGRAIEDEARFGRIRDLEAKHFKKNVEEQLNKRVGHVYKKAEMQVVEADMLSKGLLGGEAWSSWHKEDSIHVGVRCIEMLIESTGMVSLHRQNAGVVGQDSETIELAPEYAEAIATRAGALAGISPMFQPCVVPPKPWTGITGGGYWANGRRPLALVRTHSKKALMRYEDVYMPEVYKAINIAQNTAWKINKKVLAVANVITKWKHCPVEDIPAIEREELPMKPEDIDMNPEALTAWKRAAAAVYRKDKARKSRRISLEFMLEQANKFANHKAIWFPYNMDWRGRVYAVSMFNPQGNDMTKGLLTLAKGKPIGKEGYYWLKIHGANCAGVDKVPFPERIKFIEENHENIMACAKSPLENTWWAEQDSPFCFLAFCFEYAGVQHHGLSYNCSLPLAFDGSCSGIQHFSAMLRDEVGGRAVNLLPSETVQDIYGIVAKKVNEILQADAINGTDNEVVTVTDENTGEISEKVKLGTKALAGQWLAYGVTRSVTKRSVMTLAYGSKEFGFRQQVLEDTIQPAIDSGKGLMFTQPNQAAGYMAKLIWESVSVTVVAAVEAMNWLKSAAKLLAAEVKDKKTGEILRKRCAVHWVTPDGFPVWQEYKKPIQTRLNLMFLGQFRLQPTINTNKDSEIDAHKQESGIAPNFVHSQDGSHLRKTVVWAHEKYGIESFALIHDSFGTIPADAANLFKAVRETMVDTYESCDVLADFYDQFADQLHESQLDKMPALPAKGNLNLRDILESDFAFA

SEQ ID NO: 39 - protein, 883 aa, synthetic construct
MNTINIAKNDFSDIELAAIPFNTLADHYGERLAREQLALEHESYEMGEARFRKMLERQLKAGEVADNAAAKPLITTLLPKMIARINDWFEEVKAKRGKRPTAFQFLQEIKPEAVAYITIKTTLACLTSADNTTVQAVASAIGRAIEDEARFGRIRDLEAKHFKKNVEEQENKRVGHVYKKAFMQVVEADMLSKGLLGGEAWSSWHKEDSIHVGVRCIEMLIESTGMVSLHRQNAGVVGQDSETIELAPEYAEAIATRAGALAGISPMFQPCVVPPKPWTGITGGGYWANGRRPLALVRTHSKKALMRYEDVYMPEVYKAINIAQNTAWKINKKVLAVANVITKWKHCPVEDIPAIEREELPMKPEDIDMNPEALTAWKRAAAAVYRKDKARKSRRISLEFMLEQANKFANHKAIWFPYNMDWRGRVYAVSMFNPQGNDMTKGLLTLAKGKPIGKEGYYWLKIHGANCAGVDKVPFPERIKFIEENHENIMACAKSPLENTWWAEQDSPFCFLAFCFEYAGVQHHGLSYNCSLPLAFDGSCSGIQHFSAMLRDEVGGRAVNLLPSETVQDIYGIVAKKVNEILQADAINGTDNEVVTVTDENTGEISEKVKLGTKALAGQWLAYGVTRSVTKRSVMTLAYGSKEFGFRQQVLEDTIQPAIDSGKGLMFTQPNQAAGYMAKLIWESVSVTVVAAVEAMNWLKSAAKLLAAEVKDKKTGEILRKRCAVHWVTPDGFPVWQEYKKPIQTRLNLMFLGQFRLQPTINTNKDSEIDAHKQESGIAPNFVHSQDGSHLRKTVVWAHEKYGIESFALIHDSFGTIPADAANLFKAVRETMVDTYESCDVLADFYDQFADQLHESQLDKMPALPAKGNLNLRDILESDFAFA

SEQ ID NO: 40 - protein, 883 aa, synthetic construct
MNTINIAKNDFSDIELAAIPFNTLADHYGERLAREQLALEHESYEMGEARFRKMLERQLKAGEVADNAAAKPLITTLLPKMIARINDWFEEVKAKRGKRPTAFQFLQEIKPEAVAYITIKTTLACLTSADNTTVQAVASAIGRAIEDEARFGRIRDLEAKHFKKNVEEQLNKRVGHVYKKAFEQVVEADMLSKGLLGGEAWSSWHKEDSIHVGVRCIEMLIESTGMVSLHRQNAGVVGQDSETIELAPEYAEAIATRAGALAGISPMFQPCVVPPKPWTGITGGGYWANGRRPLALVRTHSKKALMRYEDVYMPEVYKAINIAQNTAWKINKKVLAVANVITKWKHCPVEDIPAIEREELPMKPEDIDMNPEALTAWKRAAAAVYRKDKARKSRRISLEFMLEQANKFANHKAIWFPYNMDWRGRVYAVSMFNPQGNDMTKGLLTLAKGKPIGKEGYYWLKIHGANCAGVDKVPFPERIKFIEENHENIMACAKSPLENTWWAEQDSPFCFLAFCFEYAGVQHHGLSYNCSLPLAFDGSCSGIQHFSAMLRDEVGGRAVNLLPSETVQDIYGIVAKKVNEILQADAINGTDNEVVTVTDENTGEISEKVKLGTKALAGQWLAYGVTRSVTKRSVMTLAYGSKEFGFRQQVLEDTIQPAIDSGKGLMFTQPNQAAGYMAKLIWESVSVTVVAAVEAMNWLKSAAKLLAAEVKDKKTGEILRKRCAVHWVTPDGFPVWQEYKKPIQTRLNLMFLGQFRLQPTINTNKDSEIDAHKQESGIAPNFVHSQDGSHLRKTVVWAHEKYGIESFALIHDSFGTIPADAANLFKAVRETMVDTYESCDVLADFYDQFADQLHESQLDKMPALPAKGNLNLRDILESDFAFA

SEQ ID NO: 41 - protein, 883 aa, synthetic construct
MNTINIAKNDFSDIELAAIPFNTLADHYGERLAREQLALEHESYEMGEARFRKMFERQLKAGEVADNAAAKPLITTLLPKMIARINDWFEEVKAKRGKRPTAFQFLQEIKPEAVAYITIKTTLACLTSADNTTVQAVASAIGRAIEDEARFGRDRDLEAKHFKKNVEEQLNKRVGHVYKKAFMQVVEADMLSKGLLGGEAWSSWHKEDSIHVGVRCIEMLIESTGMVSLHRQNAGVVGQDSETIELAPEYAEAIATRAGALAGISPMFQPCVVPPKPWTGITGGGYWANGRRPLALVRTHSKKALMRYEDVYMPEVYKAINIAQNTAWKINKKVLAVANVITKWKHCPVEDIPAIEREELPMKPEDIDMNPEALTAWKRAAAAVYRKDKARKSRRISLEFMLEQANKFANHKAIWFPYNMDWRGRVYAVSMFNPQGNDMTKGLLTLAKGKPIGKEGYYWLKIHGANCAGVDKVPFPERIKFIEENHENIMACAKSPLENTWWAEQDSPFCFLAFCFEYAGVQHHGLSYNSSLPLAFDGSCSGIQHFSAMLRDEVGGRAVNLLPSETVQDIYGIVAKKVNEILQADAINGTDNEVVTVTDENTGEISEKVKLGTKALAGQWLAYGVTRSVTKRSVMTLAYGSKEFGFRQQVLEDTIQPAIDSGKGLMFTQPNQAAGYMAKLIWESVSVTVVAAVEAMNWLKSAAKLLAAEVKDKKTGEILRKRCAVHWVTPDGFPVWQEYKKPIQTRLNLMFLGQFRLQPTINTNKDSEIDAHKQESGIAPNFVHSQDGSHLRKTVVWAHEKYGIESFALIHDSFGTIPADAANLFKAVRETMVDTYESCDVLADFYDQFADQLHESQLDKMPALPAKGNLNLRDILESDFAFA

SEQ ID NO: 42 - protein, 883 aa, synthetic construct
MNTINIAKNDFSDIELAAIPFNTLADHYGERLAREQLALEHESYEMGEARFRKMFERQLKAGEVADNAAAKPLITTLLPKMIARINDWFEEVKAKRGKRPTAFQFLQEIKPEAVAYITIKTTLACLTSADNTTVQAVASAIGRAIEDEARFGRDRDLEAKHFKKNVEEQLNKRVGHVYKKAFMQVVEADMLSKGLLGGEAWSSWHKEDSIHVGVRCIEMLIESTGMVSLHRQNAGVVGQDSETIELAPEYAEAIATRAGALAGISPMFQPCVVPPKPWTGITGGGYWANGRRPLALVRTHSKKALMRYEDVYMPEVYKAINIAQNTAWKINKKVLAVANVITKWKHCPVEDIPAIEREELPMKPEDIDMNPEALTAWKRAAAAVYRKDKARKSRRISLEFMLEQANKFANHKAIWFPYNMDWRGRVYAVSMFNPQGNDMTKGLLTFAKGKPIGKEGYYWLKIHGANCAGVDKVPFPERIKFIEENHENIMACAKSPLENTWWAEQDSPFCFLAFCFEYAGVQHHGLSYNCSLPLAFDGSCSGIQHFSAMLRDEVGGRAVNLLPSETVQDIYGIVAKKVNEILQADAINGTDNEVVTVTDENTGEISEKVKLGTKALAGQWLAYGVTRSVTKRSVMTLAYGSKEFGFRQQVLEDTIQPAIDSGKGLMFTQPNQAAGYMAKLIWESVSVTVVAAVEAMNWLKSAAKLLAAEVKDKKTGEILRKRCAVHWVTPDGFPVWQEYKKPIQTRLNLMFLGQFRLQPTINTNKDSEIDAHKQESGIAPNFVHSQDGSHLRKTVVWAHEKYGIESFALIHDSFGTIPADAANLFKAVRETMVDTYESCDVLADFYDQFADQLHESQLDKMPALPAKGNLNLRDILESDFAFA

SEQ ID NO: 43 - protein, 883 aa, synthetic construct
MNTINIAKNDFSDIELAAIPFNTLADHYGERLAREQLALEHESYEMGEARFRKMFERQLKAGEVADNAAAKPLITTLLPKMIARINDWFEEVKAKRGKRPTAFQFLQEIKPEAVAYITIKTTLACLTSADNTTVQAVASAIGRAIEDEARFGRDRDLEAKHFKKNVEEQLNKRVGHVYKKAFMQVVEADMLSKGLLGGEAWSSWHKEDSIHVGVRCIEMLIESTGMVSLHRRNAGVVGQDSETIELAPEYAEAIATRAGALAGISPMFQPCVVPPKPWTGITGGGYWANGRRPLALVRTHSKKALMRYEDVYMPEVYKAINIAQNTAWKINKKVLAVANVITKWKHCPVEDIPAIEREELPMKPEDIDMNPEALTAWKRAAAAVYRKDKARKSRRISLEFMLEQANKFANHKAIWFPYNMDWRGRVYAVSMFNPQGNDMTKGLLTLAKGKPIGKEGYYWLKIHGANCAGVDKVPFPERIKFIEENHENIMACAKSPLENTWWAEQDSPFQFLAFCFEYAGVQHHGLSYNCSLPLAFDGSCSGIQHFSAMLRDEVGGRAVNLLPSETVQDIYGIVAKKVNEILQADAINGTDNEVVTVTDENTGEISEKVKLGTKALAGQWLAYGVTRSVTKRSVMTLAYGSKEFGFRQQVLEDTIQPAIDSGKGLMFTQPNQAAGYMAKLIWESVSVTVVAAVEAMNWLKSAAKLLAAEVKDKKTGEILRKRCAVHWVTPDGFPVWQEYKKPIQTRLNLMFLGQFRLQPTINTNKDSEIDAHKQESGIAPNFVHSQDGSHLRKTVVWAHEKYGIESFALIHDSFGTIPADAANLFKAVRETMVDTYESCDVLADFYDQFADQLHESQLDKMPALPAKGNLNLRDILESDFAFA

SEQ ID NO: 44 - protein, 883 aa, synthetic construct
MNTINIAKNDFSDIELAAIPFNTLADHYGERLAREQLALEHESYEMGEARFRKMFERQLKAGEVADNAAAKPLITTLLPKMIARINDWFEEVKAKRGKRPTAFQFLQEIKPEAVAYITIKTTLACLTSADNTTVQAVASAIGRAIEDEARFGRIRDLEAKHFKKNVEEQLNAGVGHVYKKAFMQVVEADMLSKGLLGGEAWSSWHKEDSIHVGVRCIEMLIESTGMVSLHRQNAGVVGQDSETIELAPEYAEAIATRAGALAGISPMFQPCVVPPKPWTGITGGGYWANGRRPLALVRTHSKKALMRYEDVYMPEVYKAINIAQNTAWKINKKVLAVANVITKWKHCPVEDIPAIEREELPMKPEDIDMNPEALTAWKRAAAAVYRADKARKSRRISLEFMLEQANKFANHKAIWFPYNMDWRGRVYAVSMFNPQGNDMTKGLLTLAKGKPIGKEGYYWLKIHGANCAGVDKVPFPERIKFIEENHENIMACAKSPLENTWWAEQDSPFCFLAFCFEYAGVQHHGLSYNCSLPLAFDGSCSGIQHFSAMLRDEVGGRAVNLLPSETVQDIYGIVAKKVNEILQADAINGTDNEVVTVTDENTGEISEKVKLGTKALAGQWLAYGVTRSVTKRSVMTLAYGSKEFGFRQQVLEDTIQPAIDSGKGLMFTQPNQAAGYMAKLIWESVSVTVVAAVEAMNWLKSAAKLLAAEVKDKKTGEILRKRCAVHWVTPDGFPVWQEYKKPIQTRLNLMFLGQFRLQPTINTNKDSEIDAHKQESGIAPNFVHSQDGSHLRKTVVWAHEKYGIESFALIHDSFGTIPADAANLFKAVRETMVDTYESCDVLADFYDQFADQLHESQLDKMPALPAKGNLNLRDILESDFAFA

SEQ ID NO: 45 - protein, 883 aa, synthetic construct
MNTINIAKNDFSDIELAAIPFNTLADHYGERLAREQLALEHESYEMGEARFRKMFERQLKAGEVADNAAAKPLITTLLPKMIARINDWFEEVKAKRGKRPTAFQFLQEIKPEAVAYITIKTTLACLTSADNTTVQAVASAIGRAIEDEARFGRIRDLEAKHFKKNVEEQLNAGVGHVYKKAFMQVVEADMLSKGLLGGEAWSSWHKEDSIHVGVRCIEMLIESTGMVSLHRQNAGVVGQDSETIELAPEYAEAIATRAGALAGISPMFQPCVVPPKPWTGITGGGYWANGRRPLALVRTHSKKALMRYEDVYMPEVYKAINIAQNTAWKINKKVLAVANVITKWKHCPVEDIPAIEREELPMKPEDIDMNPEALTAWKRAAAAVYRQDKARKSRRISLEFMLEQANKFANHKAIWFPYNMDWRGRVYAVSMFNPQGNDMTKGLLTLAKGKPIGKEGYYWLKIHGANCAGVDKVPFPERIKFIEENHENIMACAKSPLENTWWAEQDSPFCFLAFCFEYAGVQHHGLSYNCSLPLAFDGSCSGIQHFSAMLRDEVGGRAVNLLPSETVQDIYGIVAKKVNEILQADAINGTDNEVVTVTDENTGEISEKVKLGTKALAGQWLAYGVTRSVTKRSVMTLAYGSKEFGFRQQVLEDTIQPAIDSGKGLMFTQPNQAAGYMAKLIWESVSVTVVAAVEAMNWLKSAAKLLAAEVKDKKTGEILRKRCAVHWVTPDGFPVWQEYKKPIQTRLNLMFLGQFRLQPTINTNKDSEIDAHKQESGIAPNFVHSQDGSHLRKTVVWAHEKYGIESFALIHDSFGTIPADAANLFKAVRETMVDTYESCDVLADFYDQFADQLHESQLDKMPALPAKGNLNLRDILESDFAFA

SEQ ID NO: 46 - protein, 883 aa, synthetic construct
MNTINIAKNDFSDIELAAIPFNTLADHYGERLAREQLALEHESYEMGEARFRKMFERQLKAGEVADNAAAKPLITTLLPKMIARINDWFEEVKAKRGKRPTAFQFLQEIKPEAVAYITIKTTLACLTSADNTTVQAVASAIGRAIEDEARFGRIRDLEAKHFKKNVEEQLNAGVGHVYKKAFMQVVEADMLSKGLLGGEAWSSWHKEDSIHVGVRCIEMLIESTGMVSLHRQNAGVVGQDSETIELAPEYAEAIATRAGALAGISPMFQPCVVPPKPWTGITGGGYWANGRRPLALVRTHSKKALMRYEDVYMPEVYKAINIAQNTAWKINKKVLAVANVITKWKHCPVEDIPAIEREELPMKPEDIDMNPEALTAWKRAAAAVYRKDAARKSRRISLEFMLEQANKFANHKAIWFPYNMDWRGRVYAVSMFNPQGNDMTKGLLTLAKGKPIGKEGYYWLKIHGANCAGVDKVPFPERIKFIEENHENIMACAKSPLENTWWAEQDSPFCFLAFCFEYAGVQHHGLSYNCSLPLAFDGSCSGIQHFSAMLRDEVGGRAVNLLPSETVQDIYGIVAKKVNEILQADAINGTDNEVVTVTDENTGEISEKVKLGTKALAGQWLAYGVTRSVTKRSVMTLAYGSKEFGFRQQVLEDTIQPAIDSGKGLMFTQPNQAAGYMAKLIWESVSVTVVAAVEAMNWLKSAAKLLAAEVKDKKTGEILRKRCAVHWVTPDGFPVWQEYKKPIQTRLNLMFLGQFRLQPTINTNKDSEIDAHKQESGIAPNFVHSQDGSHLRKTVVWAHEKYGIESFALIHDSFGTIPADAANLFKAVRETMVDTYESCDVLADFYDQFADQLHESQLDKMPALPAKGNLNLRDILESDFAFA

SEQ ID NO: 47 - protein, 883 aa, synthetic construct
MNTINIAKNDFSDIELAAIPFNTLADHYGERLAREQLALEHESYEMGEARFRKMFERQLKAGEVADNAAAKPLITTLLPKMIARINDWFEEVKAKRGKRPTAFQFLQEIKPEAVAYITIKTTLACLTSADNTTVQAVASAIGRAIEDEARFGRIRDLEAKHFKKNVEEQDNKRVGHVYKKAFMQVVEADMLSKGLLGGEAWSSWHKEDSIHVGVRCIEMLIESTGMVSLHRQNAGVVGQDSETIELAPEYAEAIATRAGALAGISPMFQPCVVPPKPWTGITGGGYWANGRRPLALVRTHSKKALMRYEDVYMPEVYKAINIAQNTAWKINKKVLAVANVITKWKHCPVEDIPAIEREELPMKPEDIDMNPEALTAWKRAAAAVYRKDKARKSRRISLEFMLEQANKFANHKAIWFPYNMDWRGRVYAVSMFNPQGNDMTKGLLTLAKGKPIGKEGYYWLKIHGANCAGVDKVPFPERIKFIEENHENIMACAKSPLENTWWAEQDSPFCFLAFCFEYAGVQHHGLSYNCSLPLAFDGSCSGIQHFSAMLRDEVGGRAVNLLPSETVQDIYGIVAKKVNEILQADAINGTDNEVVTVTDENTGEISEKVKLGTKALAGQWLAYGVTRSVTKRSVMTLAYGSKEFGFRQQVLEDTIQPAIDSGKGLMFTQPNQAAGYMAKLIWESVSVTVVAAVEAMNWLKSAAKLLAAEVKDKKTGEILRKRCAVHWVTPDGFPVWQEYKKPIQTRLNLMFLGQFRLQPTINTNKDSEIDAHKQESGIAPNFVHSQDGSHLRKTVVWAHEKYGIESFALIHDSFGTIPADAANLFKAVRETMVDTYESCDVLADFYDQFADQLHESQLDKMPALPAKGNLDLRDILESDFAFA

SEQ ID NO: 48 - protein, 881 aa, synthetic construct
MNTINIAKNDFSDIELAAIPFNTLADHYGERLAREQLALEHESYEMGEARFRKMFERQAKAGEVADNAAAKPLITTLLPKMIARINDWFEEVKAKRGKRPTAFQFLQEIKPEAVAYITIKTTLACLTSADNTTVQAVASAIGRAIEDEARFGRIRDLEAKHFKKNVEEQLNVGHVYKKAFMQVVEADMLSKGLLGGEAWSSWHKEDSIHVGVRCIEMLIESTGMVSLHRQNAGVVGQDSETIELAPEYAEAIATRAGALAGISPMFQPCVVPPKPWTGITGGGYWANGRRPLALVRTHSKKALMRYEDVYMPEVYKAINIAQNTAWKINKKVLAVANVITKWKHCPVEDIPAIEREELPMKPEDIDMNPEALTAWKRAAAAVYRKDKARKSRRISLEFMLEQANKFANHKAIWFPYNMDWRGRVYAVSMFNPQGNDMTKGLLTLAKGKPIGKEGYYWLKIHGANCAGVDKVPFPERIKFIEENHENIMACAKSPLENTWWAEQDSPFCFLAFCFEYAGVQHHGLSYNCSLPLAFDGSCSGIQHFSAMLRDEVGGRAVNLLPSETVQDIYGIVAKKVNEILQADAINGTDNEVVTVTDENTGEISEKVKLGTKALAGQWLAYGVTRSVTKRSVMTLAYGSKEFGFRQQVLEDTIQPAIDSGKGLMFTQPNQAAGYMAKLIWESVSVTVVAAVEAMNWLKSAAKLLAAEVKDKKTGEILRKRCAVHWVTPDGFPVWQEYKKPIQTRLNLMFLGQFRLQPTINTNKDSEIDAHKQESGIAPNFVHSQDGSHLRKTVVWAHEKYGIESFALIHDSFGTIPADAANLFKAVRETMVDTYESCDVLADFYDQFADQLHESQLDKMPALPAKGNLNLRDILESDFAFA

SEQ ID NO: 49 - protein, 883 aa, synthetic construct
MNTINIAKNDFSDIELAAIPFNTLADHYGERLAREQLALEHESYEMGEARFRKMFERQAKAGEVADNAAAKPLITTLLPKMIARINDWFEEVKAKRGKRPTAFQFLQEIKPEAVAYITIKTTLACLTSADNTTVQAVASAIGRAIEDEARFGRIRDLEAKHFKKNVEEQLNKRVGHVYKKAFEQVVEADMLSKGLLGGEAWSSWHKEDSIHVGVRCIEMLIESTGMVSLHRQNAGVVGQDSETIELAPEYAEAIATRAGALAGISPMFQPCVVPPKPWTGITGGGYWANGRRPLALVRTHSKKALMRYEDVYMPEVYKAINIAQNTAWKINKKVLAVANVITKWKHCPVEDIPAIEREELPMKPEDIDMNPEALTAWKRAAAAVYRKDKARKSRRISLEFMLEQANKFANHKAIWFPYNMDWRGRVYAVSMFNPQGNDMTKGLLTLAKGKPIGKEGYYWLKIHGANCAGVDKVPFPERIKFIEENHENIMACAKSPLENTWWAEQDSPFCFLAFCFEYAGVQHHGLSYNCSLPLAFDGSCSGIQHFSAMLRDEVGGRAVNLLPSETVQDIYGIVAKKVNEILQADAINGTDNEVVTVTDENTGEISEKVKLGTKALAGQWLAYGVTRSVTKRSVMTLAYGSKEFGFRQQVLEDTIQPAIDSGKGLMFTQPNQAAGYMAKLIWESVSVTVVAAVEAMNWLKSAAKLLAAEVKDKKTGEILRKRCAVHWVTPDGFPVWQEYKKPIQTRLNLMFLGQFRLQPTINTNKDSEIDAHKQESGIAPNFVHSQDGSHLRKTVVWAHEKYGIESFALIHDSFGTIPADAANLFKAVRETMVDTYESCDVLADFYDQFADQLHESQLDKMPALPAKGNLNLRDILESDFAFA

SEQ ID NO: 50 - protein, 883 aa, synthetic construct
MNTINIAKNDFSDIELAAIPFNTLADHYGERLAREQLALEHESYEMGEARFRKMFERQLKAGEVADNAAAKPLITTLLPKMIARINDWFEEVKAKRGKRPTAFQFLQEIKPEAVAYITIKTTLACLTSADNTTVQAVASAIGRAIEDEARFGRIRDLEAKHFKKNVEEQLNKRVGHVYKKAFEQVVEADMLSKGLLGGEAWSSWHKEDSVHVGVRCIEMLIESTGMVSLHRQNAGVVGQDSETIELAPEYAEAIATRAGALAGISPMFQPCVVPPKPWTGITGGGYWANGRRPLALVRTHSKKALMRYEDVYMPEVYKAINIAQNTAWKINKKVLAVANVITKWKHCPVEDIPAIEREELPMKPEDIDMNPEALTAWKRAAAAVYRKDKARKSRRISLEFMLEQANKFANHKAIWFPYNMDWRGRVYAVSMFNPQGNDMTKGLLTLAKGKPIGKEGYYWLKIHGANCAGVDKVPFPERIKFIEENHENIMACAKSPLENTWWAEQDSPFCFLAFCFEYAGVQHHGLSYNCSLPLAFDGSCSGIQHFSAMLRDEVGGRAVNLLPSETVQDIYGIVAKKVNEILQADAINGTDNEVVTVTDENTGEISEKVKLGTKALAGQWLAYGVTRSVTKRSVMTLAYGSKEFGFRQQVLEDTIQPAIDSGKGLMFTQPNQAAGYMAKLIWESVSVTVVAAVEAMNWLKSAAKLLAAEVKDKKTGEILRKRCAVHWVTPDGFPVWQEYKKPIQTRLNLMFLGQFRLQPTINTNKDSEIDAHKQESGIAPNFVHSQDGSHLRKTVVWAHEKYGIESFALIHDSFGTIPADAANLFKAVRETMVDTYESCDVLADFYDQFADQLHESQLDKMPALPAKGNLNLRDILESDFAFA

SEQ ID NO: 51 - protein, 883 aa, synthetic construct
MNTINIAKNDFSDIELAAIPFNTLADHYGERLAREQLALEHESYEMGEARFRKMFERQLKAGEVADNAAAKPLITTLLPKMIARINDWFEEVKAKRGKRPTAFQFLQEIKPEAVAYITIKTTLACLTSADNTTVQAVASAIGRAIEDEARFGRIRDLEAKHFKKNVEEQLKKRVGHVYKKAFEQVVEADMLSKGLLGGEAWSSWHKEDSIHVGVRCIEMLIESTGMVSLHRQNAGVVGQDSETIELAPEYAEAIATRAGALAGISPMFQPCVVPPKPWTGITGGGYWANGRRPLALVRTHSKKALMRYEDVYMPEVYKAINIAQNTAWKINKKVLAVANVITKWKHCPVEDIPAIEREELPMKPEDIDMNPEALTAWKRAAAAVYRKNKARKSRRISLEFMLEQANKFANHKAIWFPYNMDWRGRVYAVSMFNPQGNDMTKGLLTLAKGKPIGKEGYYWLKIHGANCAGVDKVPFPERIKFIEENHENIMACAKSPLENTWWAEQDSPFCFLAFCFEYAGVQHHGLSYNCSLPLAFDGSCSGIQHFSAMLRDEVGGRAVNLLPSETVQDIYGIVAKKVNEILQADAINGTDNEVVTVTDENTGEISEKVKLGTKALAGQWLAYGVTRSVTKRSVMTLAYGSKEFGFRQQVLEDTIQPAIDSGKGLMFTQPNQAAGYMAKLIWESVSVTVVAAVEAMNWLKSAAKLLAAEVKDKKTGEILRKRCAVHWVTPDGFPVWQEYKKPIQTRLNLMFLGQFRLQPTINTNKDSEIDAHKQESGIAPNFVHSQDGSHLRKTVVWAHEKYGIESFALIHDSFGTIPADAANLFKAVRETMVDTYESCDVLADFYDQFADQLHESQLDKMPALPAKGNLNLRDILESDFAFA

SEQ ID NO: 52 - protein, 881 aa, synthetic construct
MNTINIAKNDFSDIELAAIPFNTLADHYGERLAAEQLALEHESYEMGEARFRKMFERQLKAGEVADNAAAKPLITTLLPKMIARINDWFEEVKAKRGKRPTAFQFLQEIKPEAVAYITIKTTLACLTSADNTTVQAVASAIGRAIEDEARFGRIRDLEAKHFKKNVEEQLNVGHVYKKAFMQVVEADMLSKGLLGGEAWSSWHKEDSIHVGVRCIEMLIESTGMVSLHRQNAGVVGQDSETIELAPEYAEAIATRAGALAGISPMFQPCVVPPKPWTGITGGGYWANGRRPLALVRTHSKKALMRYEDVYMPEVYKAINIAQNTAWKINKKVLAVANVITKWKHCPVEDIPAIEREELPMKPEDIDMNPEALTAWKRAAAAVYRKDKARKSRRISLEFMLEQANKFANHKAIWFPYNMDWRGRVYAVSMFNPQGNDMTKGLLTLAKGKPIGKEGYYWLKIHGANCAGVDKVPFPERIKFIEENHENIMACAKSPLENTWWAEQDSPFCFLAFCFEYAGVQHHGLSYNCSLPLAFDGSCSGIQHFSAMLRDEVGGRAVNLLPSETVQDIYGIVAKKVNEILQADAINGTDNEVVTVTDENTGEISEKVKLGTKALAGQWLAYGVTRSVTKRSVMTLAYGSKEFGFRQQVLEDTIQPAIDSGKGLMFTQPNQAAGYMAKLIWESVSVTVVAAVEAMNWLKSAAKLLAAEVKDKKTGEILRKRCAVHWVTPDGFPVWQEYKKPIQTRLNLMFLGQFRLQPTINTNKDSEIDAHKQESGIAPNFVHSQDGSHLRKTVVWAHEKYGIESFALIHDSFGTIPADAANLFKAVRETMVDTYESCDVLADFYDQFADQLHESQLDKMPALPAKGNLNLRDILESDFAFA

SEQ ID NO: 53 - protein, 883 aa, synthetic construct
MNTINIAKNDFSDIELAAIPFNTLADHYGERLAAEQLALEHESYEMGEARFRKMFERQLKAGEVADNAAAKPLITTLLPKMIARINDWFEEVKAKRGKRPTAFQFLQEIKPEAVAYITIKTTLACLTSADNTTVQAVASAIGRAIEDEARFGRIRDLEAKHFKKNVEEQLNKRVGHVYKKAEMQVVEADMLSKGLLGGEAWSSWHKEDSIHVGVRCIEMLIESTGMVSLHRQNAGVVGQDSETIELAPEYAEAIATRAGALAGISPMFQPCVVPPKPWTGITGGGYWANGRRPLALVRTHSKKALMRYEDVYMPEVYKAINIAQNTAWKINKKVLAVANVITKWKHCPVEDIPAIEREELPMKPEDIDMNPEALTAWKRAAAAVYRKDKARKSRRISLEFMLEQANKFANHKAIWFPYNMDWRGRVYAVSMFNPQGNDMTKGLLTLAKGKPIGKEGYYWLKIHGANCAGVDKVPFPERIKFIEENHENIMACAKSPLENTWWAEQDSPFCFLAFCFEYAGVQHHGLSYNCSLPLAFDGSCSGIQHFSAMLRDEVGGRAVNLLPSETVQDIYGIVAKKVNEILQADAINGTDNEVVTVTDENTGEISEKVKLGTKALAGQWLAYGVTRSVTKRSVMTLAYGSKEFGFRQQVLEDTIQPAIDSGKGLMFTQPNQAAGYMAKLIWESVSVTVVAAVEAMNWLKSAAKLLAAEVKDKKTGEILRKRCAVHWVTPDGFPVWQEYKKPIQTRLNLMFLGQFRLQPTINTNKDSEIDAHKQESGIAPNFVHSQDGSHLRKTVVWAHEKYGIESFALIHDSFGTIPADAANLFKAVRETMVDTYESCDVLADFYDQFADQLHESQLDKMPALPAKGNLNLRDILESDFAFA

SEQ ID NO: 54 - protein, 883 aa, synthetic construct
MNTINIAKNDFSDIELAAIPFNTLADHYGERLAAEQLALEHESYEMGEARFRKMFERQLKAGEVADNAAAKPLITTLLPKMIARINDWFEEVKAKRGKRPTAFQFLQEIKPEAVAYITIKTTLACLTSADNTTVQAVASAIGRAIEDEARFGRIRDLEAKHFKKNVEEQENKRVGHVYKKAFMQVVEADMLSKGLLGGEAWSSWHKEDSIHVGVRCIEMLIESTGMVSLHRQNAGVVGQDSETIELAPEYAEAIATRAGALAGISPMFQPCVVPPKPWTGITGGGYWANGRRPLALVRTHSKKALMRYEDVYMPEVYKAINIAQNTAWKINKKVLAVANVITKWKHCPVEDIPAIEREELPMKPEDIDMNPEALTAWKRAAAAVYRKDKARKSRRISLEFMLEQANKFANHKAIWFPYNMDWRGRVYAVSMFNPQGNDMTKGLLTLAKGKPIGKEGYYWLKIHGANCAGVDKVPFPERIKFIEENHENIMACAKSPLENTWWAEQDSPFCFLAFCFEYAGVQHHGLSYNCSLPLAFDGSCSGIQHFSAMLRDEVGGRAVNLLPSETVQDIYGIVAKKVNEILQADAINGTDNEVVTVTDENTGEISEKVKLGTKALAGQWLAYGVTRSVTKRSVMTLAYGSKEFGFRQQVLEDTIQPAIDSGKGLMFTQPNQAAGYMAKLIWESVSVTVVAAVEAMNWLKSAAKLLAAEVKDKKTGEILRKRCAVHWVTPDGFPVWQEYKKPIQTRLNLMFLGQFRLQPTINTNKDSEIDAHKQESGIAPNFVHSQDGSHLRKTVVWAHEKYGIESFALIHDSFGTIPADAANLFKAVRETMVDTYESCDVLADFYDQFADQLHESQLDKMPALPAKGNLNLRDILESDFAFA

SEQ ID NO: 55 - protein, 883 aa, synthetic construct
MNTINIAKNDFSDIELAAIPFNTLADHYGERLAREQLALEHESYEMGEARFRKMFERQLKAGEVADNAAAKPLITTLLPKMIARINDWFEEVKAKRGKRPTAFQFLQEIKPEAVAYITIKTTLACLTSADNTTVQAVASAIGRAIEDEARFGRIRDLEAKHFKKNVEEQLNKRVGHVYKKAFEQVVEADMLSKGLLGGEAWSSWHKEDSVHVGVRCIEMLIESTGMVSLHRQNAGVVGQDSETIELAPEYAEAIATRAGALAGISPMFQPCVVPPKPWTGITGGGYWANGRRPLALVRTHSKKALMRYEDVYMPEVYKAINIAQNTAWKINKKVLAVANVITKWKHCPVEDIPAIEREELPMKPEDIDMNPEALTAWKRAAAAVYHKDKARKSRRISLEFMLEQANKFANHKAIWFPYNMDWRGRVYAVSMFNPQGNDMTKGLLTLAKGKPIGKEGYYWLKIHGANCAGVDKVPFPERIKFIEENHENIMACAKSPLENTWWAEQDSPFCFLAFCFEYAGVQHHGLSYNCSLPLAFDGSCSGIQHFSAMLRDEVGGRAVNLLPSETVQDIYGIVAKKVNEILQADAINGTDNEVVTVTDENTGEISEKVKLGTKALAGQWLAYGVTRSVTKRSVMTLAYGSKEFGFRQQVLEDTIQPAIDSGKGLMFTQPNQAAGYMAKLIWESVSVTVVAAVEAMNWLKSAAKLLAAEVKDKKTGEILRKRCAVHWVTPDGFPVWQEYKKPIQTRLNLMFLGQFRLQPTINTNKDSEIDAHKQESGIAPNFVHSQDGSHLRKTVVWAHEKYGIESFALIHDSFGTIPADAANLFKAVRETMVDTYESCDVLADFYDQFADQLHESQLDKMPALPAKGNLNLRDILESDFAFA

SEQ ID NO: 56 - protein, 883 aa, synthetic construct
MNTINIAKNDFSDIELAAIPFNTLADHYGERLAREQLALEHESYEMGEARFRKMFERQLKAGEVADNAAAKPLITTLLPKMIARINDWFEEVKAKRGKRPTAFQFLQEIKPEAVAYITIKTTLACLTSADNTTVQAVASAIGRAIEDEARFGRIRDLEAKHFKKNVEEQLNKRVGHVYKKAFEQVVEADMLSKGLLGGEAWSSWHKEDSVHVGVRCIEMLIESTGMVSLHRQNAGVVGQDSETIELAPEYAEAIATRAGALAGISPMFQPCVVPPKPWTGITGGGYWANGRRPLALVRTHSKKALMRYEDVYMPEVYKAINIAQNTAWKINKKVLAVANVITKWKHCPVEDIPAIEREELPMKPEDIDMNPEALTAWKRAAAAVYNKDKARKSRRISLEFMLEQANKFANHKAIWFPYNMDWRGRVYAVSMFNPQGNDMTKGLLTLAKGKPIGKEGYYWLKIHGANCAGVDKVPFPERIKFIEENHENIMACAKSPLENTWWAEQDSPFCFLAFCFEYAGVQHHGLSYNCSLPLAFDGSCSGIQHFSAMLRDEVGGRAVNLLPSETVQDIYGIVAKKVNEILQADAINGTDNEVVTVTDENTGEISEKVKLGTKALAGQWLAYGVTRSVTKRSVMTLAYGSKEFGFRQQVLEDTIQPAIDSGKGLMFTQPNQAAGYMAKLIWESVSVTVVAAVEAMNWLKSAAKLLAAEVKDKKTGEILRKRCAVHWVTPDGFPVWQEYKKPIQTRLNLMFLGQFRLQPTINTNKDSEIDAHKQESGIAPNFVHSQDGSHLRKTVVWAHEKYGIESFALIHDSFGTIPADAANLFKAVRETMVDTYESCDVLADFYDQFADQLHESQLDKMPALPAKGNLNLRDILESDFAFA

SEQ ID NO: 57 - protein, 883 aa, synthetic construct
MNTINIAKNDFSDIELAAIPFNTLADHYGERLAREQLALEHESYEMGEARFAKMFERQLKAGEVADNAAAKPLITTLLPKMIARINDWFEEVKAKRGKRPTAFQFLQEIKPEAVAYITIKTTLACLTSADNTTVQAVASAIGRAIEDEARFGRIRDLEAKHFKKNVEEQLNKRVGHVYDKAFMQVVEADMLSKGLLGGEAWSSWHKEDSIHVGVRCIEMLIESTGMVSLHRQNAGVVGQDSETIELAPEYAEAIATRAGALAGISPMFQPCVVPPKPWTGITGGGYWANGRRPLALVRTHSKKALMRYEDVYMPEVYKAINIAQNTAWKINKKVLAVANVITKWKHCPVEDIPAIEREELPMKPEDIDMNPEALTAWKRAAAAVYRKDKARKSRRISLEFMLEQANKFANHKAIWFPYNMDWRGRVYAVSMFNPQGNDMTKGLLTLAKGKPIGKEGYYWLKIHGANCAGVDKVPFPERIKFIEENHENIMACAKSPLENTWWAEQDSPFCFLAFCFEYAGVQHHGLSYNCSLPLAFDGSCSGIQHFSAMLRDEVGGRAVNLLPSETVQDIYGIVAKKVNEILQADAINGTDNEVVTVTDENTGEISEKVKLGTKALAGQWLAYGVTRSVTKRSVMTLAYGSKEFGFRQQVLEDTIQPAIDSGKGLMFTQPNQAAGYMAKLIWESVSVTVVAAVEAMNWLKSAAKLLAAEVKDKKTGEILRKRCAVHWVTPDGFPVWQEYKKPIQTRLNLMFLGQFRLQPTINTNKDSEIDAHKQESGIAPNFVHSQDGSHLRKTVVWAHEKYGIESFALIHDSFGTIPADAANLFKAVRETMVDTYESCDVLADFYDQFADQLHESQLDKMPALPAKGNLNLRDILESDFAFA

SEQ ID NO: 58 - protein, 883 aa, synthetic construct
MNTINIAKNDFSDIELAAIPFNTLADHYGERLAREQLALEHESYEMGEARFAKMFERQLKAGEVADNAAAKPLITTLLPKMIARINDWFEEVKAKRGKRPTAFQFLQEIKPEAVAYITIKTTLACLTSADNTTVQAVASAIGRAIEDEARFGRIRDLEAKHFKKNVEEQENKRVGHVYKKAFMQVVEADMLSKGLLGGEAWSSWHKEDSIHVGVRCIEMLIESTGMVSLHRQNAGVVGQDSETIELAPEYAEAIATRAGALAGISPMFQPCVVPPKPWTGITGGGYWANGRRPLALVRTHSKKALMRYEDVYMPEVYKAINIAQNTAWKINKKVLAVANVITKWKHCPVEDIPAIEREELPMKPEDIDMNPEALTAWKRAAAAVYRKDKARKSRRISLEFMLEQANKFANHKAIWFPYNMDWRGRVYAVSMFNPQGNDMTKGLLTLAKGKPIGKEGYYWLKIHGANCAGVDKVPFPERIKFIEENHENIMACAKSPLENTWWAEQDSPFCFLAFCFEYAGVQHHGLSYNCSLPLAFDGSCSGIQHFSAMLRDEVGGRAVNLLPSETVQDIYGIVAKKVNEILQADAINGTDNEVVTVTDENTGEISEKVKLGTKALAGQWLAYGVTRSVTKRSVMTLAYGSKEFGFRQQVLEDTIQPAIDSGKGLMFTQPNQAAGYMAKLIWESVSVTVVAAVEAMNWLKSAAKLLAAEVKDKKTGEILRKRCAVHWVTPDGFPVWQEYKKPIQTRLNLMFLGQFRLQPTINTNKDSEIDAHKQESGIAPNFVHSQDGSHLRKTVVWAHEKYGIESFALIHDSFGTIPADAANLFKAVRETMVDTYESCDVLADFYDQFADQLHESQLDKMPALPAKGNLNLRDILESDFAFA

SEQ ID NO: 59 - DNA, 2652 bp, synthetic construct
  source 1..2652: mol_type = other DNA
atgaatacaattaacatagctaaaaatgatttcagcgatattgaactggctgcgatcccgtttaataccttggcggaccattatggtgagcgtctggcgcgtgagcaacttgctctggagcacgaatcctacgagatgggtgaagcgcgtttccggaagatgttcgagcgccagcttaaggctggcgaggtggcggataacgctgctgcgaagccgttgattacgaccctgctgccgaaaatgattgcgcgtattaacgattggttcgaggaagtgaaagcaaagcgtggtaaacgtccaaccgcattccagtttctgcaagagatcaagccggaggcggtggcatacattacgatcaaaaccactctcgcatgtctcaccagcgcggataatactacggtccaagcggtggccagcgcgattggccgcgcgattgaggacgaagcgcgttttggtcgcattcgtgacctggaagcgaaacattttaagaagaacgttgaagaacaattgaataaacgcgtgggccacgtttacaagaaagcgttcatgcaagtcgttgaagctgatatgctgagcaaaggcctgttaggtggtgaagcatggagcagctggcataaggaggactcaattcacgtcggcgtgcggtgcattgaaatgctgatcgaatcgaccggtatggttagcctgcatcgccaaaacgccggcgtggtgggtcaagatagcgaaacgattgaactggcgccagagtacgcggaagctatcgctaccagagccggcgcattggcggggatcagcccgatgttccagccgtgtgttgtaccaccgaagccgtggaccggtatcaccggtggaggttactgggcgaatggtagacgtccgttggcgttggttcgtacccatagcaaaaaggctctgatgcgttatgaagacgtttacatgccggaagtgtacaaagccatcaacatcgcgcagaacactgcgtggaaaatcaacaaaaaggtgttagctgtggcgaacgtaattacaaaatggaagcactgcccggttgaggacatcccggctattgaacgtgaagagctgccaatgaaaccagaggacattgacatgaatccggaggcgctgaccgcatggaaacgtgcggcagcagcggtctatcgtaaggataaagccagaaagagccgtcgtatctccctggaattcatgcttgagcaggcgaacaaattcgctaaccacaaagccatctggtttccgtataatatggattggcgtggtcgtgtttacgcggtatcgatgttcaacccgcagggtaatgacatgaccaagggtttgttgaccttggccaaaggtaaaccgattggcaaagaaggttactattggttgaagatccacggtgcgaactgcgcaggggtggataaggtaccgttcccggaacgtattaaattcatcgaggaaaaccacgaaaacattatggcgtgcgcaaagagcccgctggaaaacacgtggtgggcagagcaggacagtccattctgcttcttggcgttctgtttcgaatatgcaggtgtccagcaccacggcctgagctataactgcagcctgccgctggcctttgatggttcttgtagcggtattcaacactttagcgccatgctgcgcgatgaggttggtggcagagcagtgaatctgctgccaagcgaaaccgtgcaagatatctatggcattgtggctaagaaggttaatgaaatcctgcaagcagacgcgattaacggcacggacaacgaggttgtcaccgtgaccgatgaaaacaccggtgagatctcggagaaagtgaaactgggcaccaaagccttggctggccaatggctggcatacggcgttactcgctccgtgaccaagcgttcggtgatgacccttgcttacggcagcaaagagtttggtttccgccaacaggttctggaggatactatccaaccggccatcgactctggtaaaggcctgatgttcacgcagccgaatcaggcagcgggctatatggcgaagctgatttgggaatcggttagcgttaccgttgttgcagcggtggaggctatgaactggctgaaatctgcggcgaagctgttagctgcggaggtgaaggacaagaagacgggcgaaatcctgcgtaagcgctgcgcagtgcattgggttacgccggatggttttccggtatggcaggagtacaaaaagcctattcagacccgtctgaacctgatgtttctgggtcaatttcgtctgcagccgacgatcaacaccaataaggactccgagatcgacgcgcacaaacaggagtctggcatcgcacccaatttcgttcactcacaggacggttcccatctgcgtaagaccgtcgtgtgggcacacgagaagtatggcattgagtcgtttgcattgatccacgattcctttggtaccatcccggcggacgctgcgaacctgtttaaagcggttcgcgaaaccatggttgacacctatgaaagttgcgatgttctggcagacttttatgatcagttcgccgaccaactgcatgagtcccagctggataaaatgccggcgttaccggcgaagggcaacttaaatctccgcgacatcctggaatctgatttcgccttcgcgtaa

SEQ ID NO: 60 - DNA, 2652 bp, synthetic construct
  source 1..2652: mol_type = other DNA
atgaatacaattaacatagctaaaaatgatttcagcgatattgaactggctgcgatcccgtttaataccttggcggaccattatggtgagcgtctggcggctgagcaacttgctctggagcacgaatcctacgagatgggtgaagcgcgtttccggaagatgttcgagcgccagcttaaggctggcgaggtggcggataacgctgctgcgaagccgttgattacgaccctgctgccgaaaatgattgcgcgtattaacgattggttcgaggaagtgaaagcaaagcgtggtaaacgtccaaccgcattccagtttctgcaagagatcaagccggaggcggtggcatacattacgatcaaaaccactctcgcatgtctcaccagcgcggataatactacggtccaagcggtggccagcgcgattggccgcgcgattgaggacgaagcgcgttttggtcgcattcgtgacctggaagcgaaacattttaagaagaacgttgaagaacaattgaataaacgcgtgggccacgtttacaagaaagcgttcatgcaagtcgttgaagctgatatgctgagcaaaggcctgttaggtggtgaagcatggagcagctggcataaggaggactcaattcacgtcggcgtgcggtgcattgaaatgctgatcgaatcgaccggtatggttagcctgcatcgccaaaacgccggcgtggtgggtcaagatagcgaaacgattgaactggcgccagagtacgcggaagctatcgctaccagagccggcgcattggcggggatcagcccgatgttccagccgtgtgttgtaccaccgaagccgtggaccggtatcaccggtggaggttactgggcgaatggtagacgtccgttggcgttggttcgtacccatagcaaaaaggctctgatgcgttatgaagacgtttacatgccggaagtgtacaaagccatcaacatcgcgcagaacactgcgtggaaaatcaacaaaaaggtgttagctgtggcgaacgtaattacaaaatggaagcactgcccggttgaggacatcccggctattgaacgtgaagagctgccaatgaaaccagaggacattgacatgaatccggaggcgctgaccgcatggaaacgtgcggcagcagcggtctatcgtaaggataaagccagaaagagccgtcgtatctccctggaattcatgcttgagcaggcgaacaaattcgctaaccacaaagccatctggtttccgtataatatggattggcgtggtcgtgtttacgcggtatcgatgttcaacccgcagggtaatgacatgaccaagggtttgttgaccttggccaaaggtaaaccgattggcaaagaaggttactattggttgaagatccacggtgcgaactgcgcaggggtggataaggtaccgttcccggaacgtattaaattcatcgaggaaaaccacgaaaacattatggcgtgcgcaaagagcccgctggaaaacacgtggtgggcagagcaggacagtccattctgcttcttggcgttctgtttcgaatatgcaggtgtccagcaccacggcctgagctataactgcagcctgccgctggcctttgatggttcttgtagcggtattcaacactttagcgccatgctgcgcgatgaggttggtggcagagcagtgaatctgctgccaagcgaaaccgtgcaagatatctatggcattgtggctaagaaggttaatgaaatcctgcaagcagacgcgattaacggcacggacaacgaggttgtcaccgtgaccgatgaaaacaccggtgagatctcggagaaagtgaaactgggcaccaaagccttggctggccaatggctggcatacggcgttactcgctccgtgaccaagcgttcggtgatgacccttgcttacggcagcaaagagtttggtttccgccaacaggttctggaggatactatccaaccggccatcgactctggtaaaggcctgatgttcacgcagccgaatcaggcagcgggctatatggcgaagctgatttgggaatcggttagcgttaccgttgttgcagcggtggaggctatgaactggctgaaatctgcggcgaagctgttagctgcggaggtgaaggacaagaagacgggcgaaatcctgcgtaagcgctgcgcagtgcattgggttacgccggatggttttccggtatggcaggagtacaaaaagcctattcagacccgtctgaacctgatgtttctgggtcaatttcgtctgcagccgacgatcaacaccaataaggactccgagatcgacgcgcacaaacaggagtctggcatcgcacccaatttcgttcactcacaggacggttcccatctgcgtaagaccgtcgtgtgggcacacgagaagtatggcattgagtcgtttgcattgatccacgattcctttggtaccatcccggcggacgctgcgaacctgtttaaagcggttcgcgaaaccatggttgacacctatgaaagttgcgatgttctggcagacttttatgatcagttcgccgaccaactgcatgagtcccagctggataaaatgccggcgttaccggcgaagggcaacttaaatctccgcgacatcctggaatctgatttcgccttcgcgtaa

SEQ ID NO: 61 - DNA, 2652 bp, synthetic construct
  source 1..2652: mol_type = other DNA
atgaatacaattaacatagctaaaaatgatttcagcgatattgaactggctgcgatcccgtttaataccttggcggaccattatggtgagcgtctggcgcgtgagcaacttgctctggagcacgaatcctacgagatgggtgaagcgcgtttccggaagatggaggagcgccagcttaaggctggcgaggtggcggataacgctgctgcgaagccgttgattacgaccctgctgccgaaaatgattgcgcgtattaacgattggttcgaggaagtgaaagcaaagcgtggtaaacgtccaaccgcattccagtttctgcaagagatcaagccggaggcggtggcatacattacgatcaaaaccactctcgcatgtctcaccagcgcggataatactacggtccaagcggtggccagcgcgattggccgcgcgattgaggacgaagcgcgttttggtcgcattcgtgacctggaagcgaaacattttaagaagaacgttgaagaacaattgaataaacgcgtgggccacgtttacaagaaagcgttcatgcaagtcgttgaagctgatatgctgagcaaaggcctgttaggtggtgaagcatggagcagctggcataaggaggactcaattcacgtcggcgtgcggtgcattgaaatgctgatcgaatcgaccggtatggttagcctgcatcgccaaaacgccggcgtggtgggtcaagatagcgaaacgattgaactggcgccagagtacgcggaagctatcgctaccagagccggcgcattggcggggatcagcccgatgttccagccgtgtgttgtaccaccgaagccgtggaccggtatcaccggtggaggttactgggcgaatggtagacgtccgttggcgttggttcgtacccatagcaaaaaggctctgatgcgttatgaagacgtttacatgccggaagtgtacaaagccatcaacatcgcgcagaacactgcgtggaaaatcaacaaaaaggtgttagctgtggcgaacgtaattacaaaatggaagcactgcccggttgaggacatcccggctattgaacgtgaagagctgccaatgaaaccagaggacattgacatgaatccggaggcgctgaccgcatggaaacgtgcggcagcagcggtctatcgtaaggataaagccagaaagagccgtcgtatctccctggaattcatgcttgagcaggcgaacaaattcgctaaccacaaagccatctggtttccgtataatatggattggcgtggtcgtgtttacgcggtatcgatgttcaacccgcagggtaatgacatgaccaagggtttgttgaccttggccaaaggtaaaccgattggcaaagaaggttactattggttgaagatccacggtgcgaactgcgcaggggtggataaggtaccgttcccggaacgtattaaattcatcgaggaaaaccacgaaaacattatggcgtgcgcaaagagcccgctggaaaacacgtggtgggcagagcaggacagtccattctgcttcttggcgttctgtttcgaatatgcaggtgtccagcaccacggcctgagctataactgcagcctgccgctggcctttgatggttcttgtagcggtattcaacactttagcgccatgctgcgcgatgaggttggtggcagagcagtgaatctgctgccaagcgaaaccgtgcaagatatctatggcattgtggctaagaaggttaatgaaatcctgcaagcagacgcgattaacggcacggacaacgaggttgtcaccgtgaccgatgaaaacaccggtgagatctcggagaaagtgaaactgggcaccaaagccttggctggccaatggctggcatacggcgttactcgctccgtgaccaagcgttcggtgatgacccttgcttacggcagcaaagagtttggtttccgccaacaggttctggaggatactatccaaccggccatcgactctggtaaaggcctgatgttcacgcagccgaatcaggcagcgggctatatggcgaagctgatttgggaatcggttagcgttaccgttgttgcagcggtggaggctatgaactggctgaaatctgcggcgaagctgttagctgcggaggtgaaggacaagaagacgggcgaaatcctgcgtaagcgctgcgcagtgcattgggttacgccggatggttttccggtatggcaggagtacaaaaagcctattcagacccgtctgaacctgatgtttctgggtcaatttcgtctgcagccgacgatcaacaccaataaggactccgagatcgacgcgcacaaacaggagtctggcatcgcacccaatttcgttcactcacaggacggttcccatctgcgtaagaccgtcgtgtgggcacacgagaagtatggcattgagtcgtttgcattgatccacgattcctttggtaccatcccggcggacgctgcgaacctgtttaaagcggttcgcgaaaccatggttgacacctatgaaagttgcgatgttctggcagacttttatgatcagttcgccgaccaactgcatgagtcccagctggataaaatgccggcgttaccggcgaagggcaacttaaatctccgcgacatcctggaatctgatttcgccttcgcgtaa

SEQ ID NO: 62 - DNA, 2652 bp, synthetic construct
  source 1..2652: mol_type = other DNA
atgaatacaattaacatagctaaaaatgatttcagcgatattgaactggctgcgatcccgtttaataccttggcggaccattatggtgagcgtctggcgcgtgagcaacttgctctggagcacgaatcctacgagatgggtgaagcgcgtttccggaagatgggagagcgccagcttaaggctggcgaggtggcggataacgctgctgcgaagccgttgattacgaccctgctgccgaaaatgattgcgcgtattaacgattggttcgaggaagtgaaagcaaagcgtggtaaacgtccaaccgcattccagtttctgcaagagatcaagccggaggcggtggcatacattacgatcaaaaccactctcgcatgtctcaccagcgcggataatactacggtccaagcggtggccagcgcgattggccgcgcgattgaggacgaagcgcgttttggtcgcattcgtgacctggaagcgaaacattttaagaagaacgttgaagaacaattgaataaacgcgtgggccacgtttacaagaaagcgttcatgcaagtcgttgaagctgatatgctgagcaaaggcctgttaggtggtgaagcatggagcagctggcataaggaggactcaattcacgtcggcgtgcggtgcattgaaatgctgatcgaatcgaccggtatggttagcctgcatcgccaaaacgccggcgtggtgggtcaagatagcgaaacgattgaactggcgccagagtacgcggaagctatcgctaccagagccggcgcattggcggggatcagcccgatgttccagccgtgtgttgtaccaccgaagccgtggaccggtatcaccggtggaggttactgggcgaatggtagacgtccgttggcgttggttcgtacccatagcaaaaaggctctgatgcgttatgaagacgtttacatgccggaagtgtacaaagccatcaacatcgcgcagaacactgcgtggaaaatcaacaaaaaggtgttagctgtggcgaacgtaattacaaaatggaagcactgcccggttgaggacatcccggctattgaacgtgaagagctgccaatgaaaccagaggacattgacatgaatccggaggcgctgaccgcatggaaacgtgcggcagcagcggtctatcgtaaggataaagccagaaagagccgtcgtatctccctggaattcatgcttgagcaggcgaacaaattcgctaaccacaaagccatctggtttccgtataatatggattggcgtggtcgtgtttacgcggtatcgatgttcaacccgcagggtaatgacatgaccaagggtttgttgaccttggccaaaggtaaaccgattggcaaagaaggttactattggttgaagatccacggtgcgaactgcgcaggggtggataaggtaccgttcccggaacgtattaaattcatcgaggaaaaccacgaaaacattatggcgtgcgcaaagagcccgctggaaaacacgtggtgggcagagcaggacagtccattctgcttcttggcgttctgtttcgaatatgcaggtgtccagcaccacggcctgagctataactgcagcctgccgctggcctttgatggttcttgtagcggtattcaacactttagcgccatgctgcgcgatgaggttggtggcagagcagtgaatctgctgccaagcgaaaccgtgcaagatatctatggcattgtggctaagaaggttaatgaaatcctgcaagcagacgcgattaacggcacggacaacgaggttgtcaccgtgaccgatgaaaacaccggtgagatctcggagaaagtgaaactgggcaccaaagccttggctggccaatggctggcatacggcgttactcgctccgtgaccaagcgttcggtgatgacccttgcttacggcagcaaagagtttggtttccgccaacaggttctggaggatactatccaaccggccatcgactctggtaaaggcctgatgttcacgcagccgaatcaggcagcgggctatatggcgaagctgatttgggaatcggttagcgttaccgttgttgcagcggtggaggctatgaactggctgaaatctgcggcgaagctgttagctgcggaggtgaaggacaagaagacgggcgaaatcctgcgtaagcgctgcgcagtgcattgggttacgccggatggttttccggtatggcaggagtacaaaaagcctattcagacccgtctgaacctgatgtttctgggtcaatttcgtctgcagccgacgatcaacaccaataaggactccgagatcgacgcgcacaaacaggagtctggcatcgcacccaatttcgttcactcacaggacggttcccatctgcgtaagaccgtcgtgtgggcacacgagaagtatggcattgagtcgtttgcattgatccacgattcctttggtaccatcccggcggacgctgcgaacctgtttaaagcggttcgcgaaaccatggttgacacctatgaaagttgcgatgttctggcagacttttatgatcagttcgccgaccaactgcatgagtcccagctggataaaatgccggcgttaccggcgaagggcaacttaaatctccgcgacatcctggaatctgatttcgccttcgcgtaa

SEQ ID NO: 63 - DNA, 2652 bp, synthetic construct
  source 1..2652: mol_type = other DNA
atgaatacaattaacatagctaaaaatgatttcagcgatattgaactggctgcgatcccgtttaataccttggcggaccattatggtgagcgtctggcgcgtgagcaacttgctctggagcacgaatcctacgagatgggtgaagcgcgtttccggaagatgaaagagcgccagcttaaggctggcgaggtggcggataacgctgctgcgaagccgttgattacgaccctgctgccgaaaatgattgcgcgtattaacgattggttcgaggaagtgaaagcaaagcgtggtaaacgtccaaccgcattccagtttctgcaagagatcaagccggaggcggtggcatacattacgatcaaaaccactctcgcatgtctcaccagcgcggataatactacggtccaagcggtggccagcgcgattggccgcgcgattgaggacgaagcgcgttttggtcgcattcgtgacctggaagcgaaacattttaagaagaacgttgaagaacaattgaataaacgcgtgggccacgtttacaagaaagcgttcatgcaagtcgttgaagctgatatgctgagcaaaggcctgttaggtggtgaagcatggagcagctggcataaggaggactcaattcacgtcggcgtgcggtgcattgaaatgctgatcgaatcgaccggtatggttagcctgcatcgccaaaacgccggcgtggtgggtcaagatagcgaaacgattgaactggcgccagagtacgcggaagctatcgctaccagagccggcgcattggcggggatcagcccgatgttccagccgtgtgttgtaccaccgaagccgtggaccggtatcaccggtggaggttactgggcgaatggtagacgtccgttggcgttggttcgtacccatagcaaaaaggctctgatgcgttatgaagacgtttacatgccggaagtgtacaaagccatcaacatcgcgcagaacactgcgtggaaaatcaacaaaaaggtgttagctgtggcgaacgtaattacaaaatggaagcactgcccggttgaggacatcccggctattgaacgtgaagagctgccaatgaaaccagaggacattgacatgaatccggaggcgctgaccgcatggaaacgtgcggcagcagcggtctatcgtaaggataaagccagaaagagccgtcgtatctccctggaattcatgcttgagcaggcgaacaaattcgctaaccacaaagccatctggtttccgtataatatggattggcgtggtcgtgtttacgcggtatcgatgttcaacccgcagggtaatgacatgaccaagggtttgttgaccttggccaaaggtaaaccgattggcaaagaaggttactattggttgaagatccacggtgcgaactgcgcaggggtggataaggtaccgttcccggaacgtattaaattcatcgaggaaaaccacgaaaacattatggcgtgcgcaaagagcccgctggaaaacacgtggtgggcagagcaggacagtccattctgcttcttggcgttctgtttcgaatatgcaggtgtccagcaccacggcctgagctataactgcagcctgccgctggcctttgatggttcttgtagcggtattcaacactttagcgccatgctgcgcgatgaggttggtggcagagcagtgaatctgctgccaagcgaaaccgtgcaagatatctatggcattgtggctaagaaggttaatgaaatcctgcaagcagacgcgattaacggcacggacaacgaggttgtcaccgtgaccgatgaaaacaccggtgagatctcggagaaagtgaaactgggcaccaaagccttggctggccaatggctggcatacggcgttactcgctccgtgaccaagcgttcggtgatgacccttgcttacggcagcaaagagtttggtttccgccaacaggttctggaggatactatccaaccggccatcgactctggtaaaggcctgatgttcacgcagccgaatcaggcagcgggctatatggcgaagctgatttgggaatcggttagcgttaccgttgttgcagcggtggaggctatgaactggctgaaatctgcggcgaagctgttagctgcggaggtgaaggacaagaagacgggcgaaatcctgcgtaagcgctgcgcagtgcattgggttacgccggatggttttccggtatggcaggagtacaaaaagcctattcagacccgtctgaacctgatgtttctgggtcaatttcgtctgcagccgacgatcaacaccaataaggactccgagatcgacgcgcacaaacaggagtctggcatcgcacccaatttcgttcactcacaggacggttcccatctgcgtaagaccgtcgtgtgggcacacgagaagtatggcattgagtcgtttgcattgatccacgattcctttggtaccatcccggcggacgctgcgaacctgtttaaagcggttcgcgaaaccatggttgacacctatgaaagttgcgatgttctggcagacttttatgatcagttcgccgaccaactgcatgagtcccagctggataaaatgccggcgttaccggcgaagggcaacttaaatctccgcgacatcctggaatctgatttcgccttcgcgtaa

SEQ ID NO: 64 - DNA, 2652 bp, synthetic construct
  source 1..2652: mol_type = other DNA
atgaatacaattaacatagctaaaaatgatttcagcgatattgaactggctgcgatcccgtttaataccttggcggaccattatggtgagcgtctggcgcgtgagcaacttgctctggagcacgaatcctacgagatgggtgaagcgcgtttccggaagatgcttgagcgccagcttaaggctggcgaggtggcggataacgctgctgcgaagccgttgattacgaccctgctgccgaaaatgattgcgcgtattaacgattggttcgaggaagtgaaagcaaagcgtggtaaacgtccaaccgcattccagtttctgcaagagatcaagccggaggcggtggcatacattacgatcaaaaccactctcgcatgtctcaccagcgcggataatactacggtccaagcggtggccagcgcgattggccgcgcgattgaggacgaagcgcgttttggtcgcattcgtgacctggaagcgaaacattttaagaagaacgttgaagaacaattgaataaacgcgtgggccacgtttacaagaaagcgttcatgcaagtcgttgaagctgatatgctgagcaaaggcctgttaggtggtgaagcatggagcagctggcataaggaggactcaattcacgtcggcgtgcggtgcattgaaatgctgatcgaatcgaccggtatggttagcctgcatcgccaaaacgccggcgtggtgggtcaagatagcgaaacgattgaactggcgccagagtacgcggaagctatcgctaccagagccggcgcattggcggggatcagcccgatgttccagccgtgtgttgtaccaccgaagccgtggaccggtatcaccggtggaggttactgggcgaatggtagacgtccgttggcgttggttcgtacccatagcaaaaaggctctgatgcgttatgaagacgtttacatgccggaagtgtacaaagccatcaacatcgcgcagaacactgcgtggaaaatcaacaaaaaggtgttagctgtggcgaacgtaattacaaaatggaagcactgcccggttgaggacatcccggctattgaacgtgaagagctgccaatgaaaccagaggacattgacatgaatccggaggcgctgaccgcatggaaacgtgcggcagcagcggtctatcgtaaggataaagccagaaagagccgtcgtatctccctggaattcatgcttgagcaggcgaacaaattcgctaaccacaaagccatctggtttccgtataatatggattggcgtggtcgtgtttacgcggtatcgatgttcaacccgcagggtaatgacatgaccaagggtttgttgaccttggccaaaggtaaaccgattggcaaagaaggttactattggttgaagatccacggtgcgaactgcgcaggggtggataaggtaccgttcccggaacgtattaaattcatcgaggaaaaccacgaaaacattatggcgtgcgcaaagagcccgctggaaaacacgtggtgggcagagcaggacagtccattctgcttcttggcgttctgtttcgaatatgcaggtgtccagcaccacggcctgagctataactgcagcctgccgctggcctttgatggttcttgtagcggtattcaacactttagcgccatgctgcgcgatgaggttggtggcagagcagtgaatctgctgccaagcgaaaccgtgcaagatatctatggcattgtggctaagaaggttaatgaaatcctgcaagcagacgcgattaacggcacggacaacgaggttgtcaccgtgaccgatgaaaacaccggtgagatctcggagaaagtgaaactgggcaccaaagccttggctggccaatggctggcatacggcgttactcgctccgtgaccaagcgttcggtgatgacccttgcttacggcagcaaagagtttggtttccgccaacaggttctggaggatactatccaaccggccatcgactctggtaaaggcctgatgttcacgcagccgaatcaggcagcgggctatatggcgaagctgatttgggaatcggttagcgttaccgttgttgcagcggtggaggctatgaactggctgaaatctgcggcgaagctgttagctgcggaggtgaaggacaagaagacgggcgaaatcctgcgtaagcgctgcgcagtgcattgggttacgccggatggttttccggtatggcaggagtacaaaaagcctattcagacccgtctgaacctgatgtttctgggtcaatttcgtctgcagccgacgatcaacaccaataaggactccgagatcgacgcgcacaaacaggagtctggcatcgcacccaatttcgttcactcacaggacggttcccatctgcgtaagaccgtcgtgtgggcacacgagaagtatggcattgagtcgtttgcattgatccacgattcctttggtaccatcccggcggacgctgcgaacctgtttaaagcggttcgcgaaaccatggttgacacctatgaaagttgcgatgttctggcagacttttatgatcagttcgccgaccaactgcatgagtcccagctggataaaatgccggcgttaccggcgaagggcaacttaaatctccgcgacatcctggaatctgatttcgccttcgcgtaa

SEQ ID NO: 65 - DNA, 2652 bp, synthetic construct
  source 1..2652: mol_type = other DNA
atgaatacaattaacatagctaaaaatgatttcagcgatattgaactggctgcgatcccgtttaataccttggcggaccattatggtgagcgtctggcgcgtgagcaacttgctctggagcacgaatcctacgagatgggtgaagcgcgtttccggaagatgaatgagcgccagcttaaggctggcgaggtggcggataacgctgctgcgaagccgttgattacgaccctgctgccgaaaatgattgcgcgtattaacgattggttcgaggaagtgaaagcaaagcgtggtaaacgtccaaccgcattccagtttctgcaagagatcaagccggaggcggtggcatacattacgatcaaaaccactctcgcatgtctcaccagcgcggataatactacggtccaagcggtggccagcgcgattggccgcgcgattgaggacgaagcgcgttttggtcgcattcgtgacctggaagcgaaacattttaagaagaacgttgaagaacaattgaataaacgcgtgggccacgtttacaagaaagcgttcatgcaagtcgttgaagctgatatgctgagcaaaggcctgttaggtggtgaagcatggagcagctggcataaggaggactcaattcacgtcggcgtgcggtgcattgaaatgctgatcgaatcgaccggtatggttagcctgcatcgccaaaacgccggcgtggtgggtcaagatagcgaaacgattgaactggcgccagagtacgcggaagctatcgctaccagagccggcgcattggcggggatcagcccgatgttccagccgtgtgttgtaccaccgaagccgtggaccggtatcaccggtggaggttactgggcgaatggtagacgtccgttggcgttggttcgtacccatagcaaaaaggctctgatgcgttatgaagacgtttacatgccggaagtgtacaaagccatcaacatcgcgcagaacactgcgtggaaaatcaacaaaaaggtgttagctgtggcgaacgtaattacaaaatggaagcactgcccggttgaggacatcccggctattgaacgtgaagagctgccaatgaaaccagaggacattgacatgaatccggaggcgctgaccgcatggaaacgtgcggcagcagcggtctatcgtaaggataaagccagaaagagccgtcgtatctccctggaattcatgcttgagcaggcgaacaaattcgctaaccacaaagccatctggtttccgtataatatggattggcgtggtcgtgtttacgcggtatcgatgttcaacccgcagggtaatgacatgaccaagggtttgttgaccttggccaaaggtaaaccgattggcaaagaaggttactattggttgaagatccacggtgcgaactgcgcaggggtggataaggtaccgttcccggaacgtattaaattcatcgaggaaaaccacgaaaacattatggcgtgcgcaaagagcccgctggaaaacacgtggtgggcagagcaggacagtccattctgcttcttggcgttctgtttcgaatatgcaggtgtccagcaccacggcctgagctataactgcagcctgccgctggcctttgatggttcttgtagcggtattcaacactttagcgccatgctgcgcgatgaggttggtggcagagcagtgaatctgctgccaagcgaaaccgtgcaagatatctatggcattgtggctaagaaggttaatgaaatcctgcaagcagacgcgattaacggcacggacaacgaggttgtcaccgtgaccgatgaaaacaccggtgagatctcggagaaagtgaaactgggcaccaaagccttggctggccaatggctggcatacggcgttactcgctccgtgaccaagcgttcggtgatgacccttgcttacggcagcaaagagtttggtttccgccaacaggttctggaggatactatccaaccggccatcgactctggtaaaggcctgatgttcacgcagccgaatcaggcagcgggctatatggcgaagctgatttgggaatcggttagcgttaccgttgttgcagcggtggaggctatgaactggctgaaatctgcggcgaagctgttagctgcggaggtgaaggacaagaagacgggcgaaatcctgcgtaagcgctgcgcagtgcattgggttacgccggatggttttccggtatggcaggagtacaaaaagcctattcagacccgtctgaacctgatgtttctgggtcaatttcgtctgcagccgacgatcaacaccaataaggactccgagatcgacgcgcacaaacaggagtctggcatcgcacccaatttcgttcactcacaggacggttcccatctgcgtaagaccgtcgtgtgggcacacgagaagtatggcattgagtcgtttgcattgatccacgattcctttggtaccatcccggcggacgctgcgaacctgtttaaagcggttcgcgaaaccatggttgacacctatgaaagttgcgatgttctggcagacttttatgatcagttcgccgaccaactgcatgagtcccagctggataaaatgccggcgttaccggcgaagggcaacttaaatctccgcgacatcctggaatctgatttcgccttcgcgtaa

SEQ ID NO: 66 - DNA, 2652 bp, synthetic construct
  source 1..2652: mol_type = other DNA
atgaatacaattaacatagctaaaaatgatttcagcgatattgaactggctgcgatcccgtttaataccttggcggaccattatggtgagcgtctggcgcgtgagcaacttgctctggagcacgaatcctacgagatgggtgaagcgcgtttccggaagatgttcgagcgccagcttaaggctggcgaggtggcggataacgctgctgcgaagccgttgattacgaccctgctgccgaaaatgattgcgcgtattaacgattggttcgaggaagtgaaagcaaagcgtggtaaacgtccaaccgcattccagtttctgcaagagatcaagccggaggcggtggcatacattacgatcaaaaccactctcgcatgtctcaccagcgcggataatactacggtccaagcggtggccagcgcgattggccgcgcgattgaggacgaagcgcgttttggtcgcattcgtgacctggaagcgaaacattttaagaagaacgttgaagaacaattgaataaacgcgtgggccacgtttacaagaaagcgttcatgcaagtcgttgaagctgatatgctgagcaaaggcctgttaggtggtgaagcatggagcagctggcataaggaggactcaattcacgtcggcgtgcggtgcattgaaatgctgatcgaatcgaccggtatggttagcctgcatcgccaaaacgccggcgtggtgggtcaagatagcgaaacgattgaactggcgccagagtacgcggaagctatcgctaccagagccggcgcattggcggggatcagcccgatgttccagccgtgtgttgtaccaccgaagccgtggaccggtatcaccggtggaggttactgggcgaatggtagacgtccgttggcgttggttcgtacccatagcaaaaaggctctgatgcgttatgaagacgtttacatgccggaagtgtacaaagccatcaacatcgcgcagaacactgcgtggaaaatcaacaaaaaggtgttagctgtggcgaacgtaattacaaaatggaagcactgcccggttgaggacatcccggctattgaacgtgaagagctgccaatgaaaccagaggacattgacatgaatccggaggcgctgaccgcatggaaacgtgcggcagcagcggtctatcgtaaggataaagccagaaagagccgtcgtatctccctggaattcatgcttgagcaggcgaacaaattcgctaaccacaaagccatctggtttccgtataatatggattggcgtggtcgtgtttacgcggtatcgatgttcaacccgcagggtaatgacatgaccaagggtttgttgaccttggccaaaggtaaaccgattggcaaagaaggttactattggttgaagatccacggtgcgaactgcgcaggggtggataaggtaccgttcccggaacgtattaaattcatcgaggaaaaccacgaaaacattatggcgtgcgcaaagagcccgctggaaaacacgtggtgggcagagcaggacagtccattctgcttcttggcgttctgtttcgaatatgcaggtgtccagcaccacggcctgagctataactgcagcctgccgctggcctttgatggttcttgtagcggtattcaacactttagcgccatgctgcgcgatgaggttggtggcagagcagtgaatctgctgccaagcgaaaccgtgcaagatatctatggcattgtggctaagaaggttaatgaaatcctgcaagcagacgcgattaacggcacggacaacgaggttgtcaccgtgaccgatgaaaacaccggtgagatctcggagaaagtgaaactgggcaccaaagccttggctggccaatggctggcatacggcgttactcgctccgtgaccaagcgttcggtgatgacccttgcttacggcagcaaagagtttggtttccgccaacaggttctggaggatactatccaaccggccatcgactctggtaaaggcctgatgttcacgcagccgaatcaggcagcgggctatatggcgaagctgatttgggaatcggttagcgttaccgttgttgcagcggtggaggctatgaactggctgaaatctgcggcgaagctgttagctgcggaggtgaaggacaagaagacgggcgaaatcctgcgtaagcgctgcgcagtgcattgggttacgccggatggttttccggtatggcaggagtacaaaaagcctattcagacccgtctgaacctgatgtttctggatcaatttcgtctgcagccgacgatcaacaccaataaggactccgagatcgacgcgcacaaacaggagtctggcatcgcacccaatttcgttcactcacaggacggttcccatctgcgtaagaccgtcgtgtgggcacacgagaagtatggcattgagtcgtttgcattgatccacgattcctttggtaccatcccggcggacgctgcgaacctgtttaaagcggttcgcgaaaccatggttgacacctatgaaagttgcgatgttctggcagacttttatgatcagttcgccgaccaactgcatgagtcccagctggataaaatgccggcgttaccggcgaagggcaacttaaatctccgcgacatcctggaatctgatttcgccttcgcgtaa

SEQ ID NO: 67 - DNA, 2652 bp, synthetic construct
  source 1..2652: mol_type = other DNA
atgaatacaattaacatagctaaaaatgatttcagcgatattgaactggctgcgatcccgtttaataccttggcggaccattatggtgagcgtctggcgcgtgagcaacttgctctggagcacgaatcctacgagatgggtgaagcgcgtttccggaagatgttcgagcgccagcttaaggctggcgaggtggcggataacgctgctgcgaagccgttgattacgaccctgctgccgaaaatgattgcgcgtattaacgattggttcgaggaagtgaaagcaaagcgtggtaaacgtccaaccgcattccagtttctgcaagagatcaagccggaggcggtggcatacattacgatcaaaaccactctcgcatgtctcaccagcgcggataatactacggtccaagcggtggccagcgcgattggccgcgcgattgaggacgaagcgcgttttggtcgcgatcgtgacctggaagcgaaacattttaagaagaacgttgaagaacaattgaataaacgcgtgggccacgtttacaagaaagcgttcatgcaagtcgttgaagctgatatgctgagcaaaggcctgttaggtggtgaagcatggagcagctggcataaggaggactcaattcacgtcggcgtgcggtgcattgaaatgctgatcgaatcgaccggtatggttagcctgcatcgccaaaacgccggcgtggtgggtcaagatagcgaaacgattgaactggcgccagagtacgcggaagctatcgctaccagagccggcgcattggcggggatcagcccgatgttccagccgtgtgttgtaccaccgaagccgtggaccggtatcaccggtggaggttactgggcgaatggtagacgtccgttggcgttggttcgtacccatagcaaaaaggctctgatgcgttatgaagacgtttacatgccggaagtgtacaaagccatcaacatcgcgcagaacactgcgtggaaaatcaacaaaaaggtgttagctgtggcgaacgtaattacaaaatggaagcactgcccggttgaggacatcccggctattgaacgtgaagagctgccaatgaaaccagaggacattgacatgaatccggaggcgctgaccgcatggaaacgtgcggcagcagcggtctatcgtaaggataaagccagaaagagccgtcgtatctccctggaattcatgcttgagcaggcgaacaaattcgctaaccacaaagccatctggtttccgtataatatggattggcgtggtcgtgtttacgcggtatcgatgttcaacccgcagggtaatgacatgaccaagggtttgttgaccttggccaaaggtaaaccgattggcaaagaaggttactattggttgaagatccacggtgcgaactgcgcaggggtggataaggtaccgttcccggaacgtattaaattcatcgaggaaaaccacgaaaacattatggcgtgcgcaaagagcccgctggaaaacacgtggtgggcagagcaggacagtccattctgcttcttggcgttctgtttcgaatatgcaggtgtccagcaccacggcctgagctataactgcagcctgccgctggcctttgatggttcttgtagcggtattcaacactttagcgccatgctgcgcgatgaggttggtggcagagcagtgaatctgctgccaagcgaaaccgtgcaagatatctatggcattgtggctaagaaggttaatgaaatcctgcaagcagacgcgattaacggcacggacaacgaggttgtcaccgtgaccgatgaaaacaccggtgagatctcggagaaagtgaaactgggcaccaaagccttggctggccaatggctggcatacggcgttactcgctccgtgaccaagcgttcggtgatgacccttgcttacggcagcaaagagtttggtttccgccaacaggttctggaggatactatccaaccggccatcgactctggtaaaggcctgatgttcacgcagccgaatcaggcagcgggctatatggcgaagctgatttgggaatcggttagcgttaccgttgttgcagcggtggaggctatgaactggctgaaatctgcggcgaagctgttagctgcggaggtgaaggacaagaagacgggcgaaatcctgcgtaagcgctgcgcagtgcattgggttacgccggatggttttccggtatggcaggagtacaaaaagcctattcagacccgtctgaacctgatgtttctgggtcaatttcgtctgcagccgacgatcaacaccaataaggactccgagatcgacgcgcacaaacaggagtctggcatcgcacccaatttcgttcactcacaggacggttcccatctgcgtaagaccgtcgtgtgggcacacgagaagtatggcattgagtcgtttgcattgatccacgattcctttggtaccatcccggcggacgctgcgaacctgtttaaagcggttcgcgaaaccatggttgacacctatgaaagttgcgatgttctggcagacttttatgatcagttcgccgaccaactgcatgagtcccagctggataaaatgccggcgttaccggcgaagggcaacttaaatctccgcgacatcctggaatctgatttcgccttcgcgtaa

SEQ ID NO: 68 - DNA, 2652 bp, synthetic construct
  source 1..2652: mol_type = other DNA
atgaatacaattaacatagctaaaaatgatttcagcgatattgaactggctgcgatcccgtttaataccttggcggaccattatggtgagcgtctggcgcgtgagcaacttgctctggagcacgaatcctacgagatgggtgaagcgcgtttccggaagatgttcgagcgccagcttaaggctggcgaggtggcggataacgctgctgcgaagccgttgattacgaccctgctgccgaaaatgattgcgcgtattaacgattggttcgaggaagtgaaagcaaagcgtggtaaacgtccaaccgcattccagtttctgcaagagatcaagccggaggcggtggcatacattacgatcaaaaccactctcgcatgtctcaccagcgcggataatactacggtccaagcggtggccagcgcgattggccgcgcgattgaggacgaagcgcgttttggtcgcattcgtgacctggaagcgaaacattttaagaagaacgttgaagaacaagcgaataaacgcgtgggccacgtttacaagaaagcgttcatgcaagtcgttgaagctgatatgctgagcaaaggcctgttaggtggtgaagcatggagcagctggcataaggaggactcaattcacgtcggcgtgcggtgcattgaaatgctgatcgaatcgaccggtatggttagcctgcatcgccaaaacgccggcgtggtgggtcaagatagcgaaacgattgaactggcgccagagtacgcggaagctatcgctaccagagccggcgcattggcggggatcagcccgatgttccagccgtgtgttgtaccaccgaagccgtggaccggtatcaccggtggaggttactgggcgaatggtagacgtccgttggcgttggttcgtacccatagcaaaaaggctctgatgcgttatgaagacgtttacatgccggaagtgtacaaagccatcaacatcgcgcagaacactgcgtggaaaatcaacaaaaaggtgttagctgtggcgaacgtaattacaaaatggaagcactgcccggttgaggacatcccggctattgaacgtgaagagctgccaatgaaaccagaggacattgacatgaatccggaggcgctgaccgcatggaaacgtgcggcagcagcggtctatcgtaaggataaagccagaaagagccgtcgtatctccctggaattcatgcttgagcaggcgaacaaattcgctaaccacaaagccatctggtttccgtataatatggattggcgtggtcgtgtttacgcggtatcgatgttcaacccgcagggtaatgacatgaccaagggtttgttgaccttggccaaaggtaaaccgattggcaaagaaggttactattggttgaagatccacggtgcgaactgcgcaggggtggataaggtaccgttcccggaacgtattaaattcatcgaggaaaaccacgaaaacattatggcgtgcgcaaagagcccgctggaaaacacgtggtgggcagagcaggacagtccattctgcttcttggcgttctgtttcgaatatgcaggtgtccagcaccacggcctgagctataactgcagcctgccgctggcctttgatggttcttgtagcggtattcaacactttagcgccatgctgcgcgatgaggttggtggcagagcagtgaatctgctgccaagcgaaaccgtgcaagatatctatggcattgtggctaagaaggttaatgaaatcctgcaagcagacgcgattaacggcacggacaacgaggttgtcaccgtgaccgatgaaaacaccggtgagatctcggagaaagtgaaactgggcaccaaagccttggctggccaatggctggcatacggcgttactcgctccgtgaccaagcgttcggtgatgacccttgcttacggcagcaaagagtttggtttccgccaacaggttctggaggatactatccaaccggccatcgactctggtaaaggcctgatgttcacgcagccgaatcaggcagcgggctatatggcgaagctgatttgggaatcggttagcgttaccgttgttgcagcggtggaggctatgaactggctgaaatctgcggcgaagctgttagctgcggaggtgaaggacaagaagacgggcgaaatcctgcgtaagcgctgcgcagtgcattgggttacgccggatggttttccggtatggcaggagtacaaaaagcctattcagacccgtctgaacctgatgtttctgggtcaatttcgtctgcagccgacgatcaacaccaataaggactccgagatcgacgcgcacaaacaggagtctggcatcgcacccaatttcgttcactcacaggacggttcccatctgcgtaagaccgtcgtgtgggcacacgagaagtatggcattgagtcgtttgcattgatccacgattcctttggtaccatcccggcggacgctgcgaacctgtttaaagcggttcgcgaaaccatggttgacacctatgaaagttgcgatgttctggcagacttttatgatcagttcgccgaccaactgcatgagtcccagctggataaaatgccggcgttaccggcgaagggcaacttaaatctccgcgacatcctggaatctgatttcgccttcgcgtaa

SEQ ID NO: 69 - DNA, 2649 bp, synthetic construct
  source 1..2649: mol_type = other DNA
atgaatacaattaacatagctaaaaatgatttcagcgatattgaactggctgcgatcccgtttaataccttggcggaccattatggtgagcgtctggcgcgtgagcaacttgctctggagcacgaatcctacgagatgggtgaagcgcgtttccggaagatgttcgagcgccagcttaaggctggcgaggtggcggataacgctgctgcgaagccgttgattacgaccctgctgccgaaaatgattgcgcgtattaacgattggttcgaggaagtgaaagcaaagcgtggtaaacgtccaaccgcattccagtttctgcaagagatcaagccggaggcggtggcatacattacgatcaaaaccactctcgcatgtctcaccagcgcggataatactacggtccaagcggtggccagcgcgattggccgcgcgattgaggacgaagcgcgttttggtcgcattcgtgacctggaagcgaaacattttaagaagaacgttgaagaacaattgaatcgcgtgggccacgtttacaagaaagcgttcatgcaagtcgttgaagctgatatgctgagcaaaggcctgttaggtggtgaagcatggagcagctggcataaggaggactcaattcacgtcggcgtgcggtgcattgaaatgctgatcgaatcgaccggtatggttagcctgcatcgccaaaacgccggcgtggtgggtcaagatagcgaaacgattgaactggcgccagagtacgcggaagctatcgctaccagagccggcgcattggcggggatcagcccgatgttccagccgtgtgttgtaccaccgaagccgtggaccggtatcaccggtggaggttactgggcgaatggtagacgtccgttggcgttggttcgtacccatagcaaaaaggctctgatgcgttatgaagacgtttacatgccggaagtgtacaaagccatcaacatcgcgcagaacactgcgtggaaaatcaacaaaaaggtgttagctgtggcgaacgtaattacaaaatggaagcactgcccggttgaggacatcccggctattgaacgtgaagagctgccaatgaaaccagaggacattgacatgaatccggaggcgctgaccgcatggaaacgtgcggcagcagcggtctatcgtaaggataaagccagaaagagccgtcgtatctccctggaattcatgcttgagcaggcgaacaaattcgctaaccacaaagccatctggtttccgtataatatggattggcgtggtcgtgtttacgcggtatcgatgttcaacccgcagggtaatgacatgaccaagggtttgttgaccttggccaaaggtaaaccgattggcaaagaaggttactattggttgaagatccacggtgcgaactgcgcaggggtggataaggtaccgttcccggaacgtattaaattcatcgaggaaaaccacgaaaacattatggcgtgcgcaaagagcccgctggaaaacacgtggtgggcagagcaggacagtccattctgcttcttggcgttctgtttcgaatatgcaggtgtccagcaccacggcctgagctataactgcagcctgccgctggcctttgatggttcttgtagcggtattcaacactttagcgccatgctgcgcgatgaggttggtggcagagcagtgaatctgctgccaagcgaaaccgtgcaagatatctatggcattgtggctaagaaggttaatgaaatcctgcaagcagacgcgattaacggcacggacaacgaggttgtcaccgtgaccgatgaaaacaccggtgagatctcggagaaagtgaaactgggcaccaaagccttggctggccaatggctggcatacggcgttactcgctccgtgaccaagcgttcggtgatgacccttgcttacggcagcaaagagtttggtttccgccaacaggttctggaggatactatccaaccggccatcgactctggtaaaggcctgatgttcacgcagccgaatcaggcagcgggctatatggcgaagctgatttgggaatcggttagcgttaccgttgttgcagcggtggaggctatgaactggctgaaatctgcggcgaagctgttagctgcggaggtgaaggacaagaagacgggcgaaatcctgcgtaagcgctgcgcagtgcattgggttacgccggatggttttccggtatggcaggagtacaaaaagcctattcagacccgtctgaacctgatgtttctgggtcaatttcgtctgcagccgacgatcaacaccaataaggactccgagatcgacgcgcacaaacaggagtctggcatcgcacccaatttcgttcactcacaggacggttcccatctgcgtaagaccgtcgtgtgggcacacgagaagtatggcattgagtcgtttgcattgatccacgattcctttggtaccatcccggcggacgctgcgaacctgtttaaagcggttcgcgaaaccatggttgacacctatgaaagttgcgatgttctggcagacttttatgatcagttcgccgaccaactgcatgagtcccagctggataaaatgccggcgttaccggcgaagggcaacttaaatctccgcgacatcctggaatctgatttcgccttcgcgtaa

SEQ ID NO: 70 - DNA, 2652 bp, synthetic construct
  source 1..2652: mol_type = other DNA
atgaatacaattaacatagctaaaaatgatttcagcgatattgaactggctgcgatcccgtttaataccttggcggaccattatggtgagcgtctggcgcgtgagcaacttgctctggagcacgaatcctacgagatgggtgaagcgcgtttccggaagatgttcgagcgccagcttaaggctggcgaggtggcggataacgctgctgcgaagccgttgattacgaccctgctgccgaaaatgattgcgcgtattaacgattggttcgaggaagtgaaagcaaagcgtggtaaacgtccaaccgcattccagtttctgcaagagatcaagccggaggcggtggcatacattacgatcaaaaccactctcgcatgtctcaccagcgcggataatactacggtccaagcggtggccagcgcgattggccgcgcgattgaggacgaagcgcgttttggtcgcattcgtgacctggaagcgaaacattttaagaagaacgttgaagaacaattgaatgcacgcgtgggccacgtttacaagaaagcgttcatgcaagtcgttgaagctgatatgctgagcaaaggcctgttaggtggtgaagcatggagcagctggcataaggaggactcaattcacgtcggcgtgcggtgcattgaaatgctgatcgaatcgaccggtatggttagcctgcatcgccaaaacgccggcgtggtgggtcaagatagcgaaacgattgaactggcgccagagtacgcggaagctatcgctaccagagccggcgcattggcggggatcagcccgatgttccagccgtgtgttgtaccaccgaagccgtggaccggtatcaccggtggaggttactgggcgaatggtagacgtccgttggcgttggttcgtacccatagcaaaaaggctctgatgcgttatgaagacgtttacatgccggaagtgtacaaagccatcaacatcgcgcagaacactgcgtggaaaatcaacaaaaaggtgttagctgtggcgaacgtaattacaaaatggaagcactgcccggttgaggacatcccggctattgaacgtgaagagctgccaatgaaaccagaggacattgacatgaatccggaggcgctgaccgcatggaaacgtgcggcagcagcggtctatcgtaaggataaagccagaaagagccgtcgtatctccctggaattcatgcttgagcaggcgaacaaattcgctaaccacaaagccatctggtttccgtataatatggattggcgtggtcgtgtttacgcggtatcgatgttcaacccgcagggtaatgacatgaccaagggtttgttgaccttggccaaaggtaaaccgattggcaaagaaggttactattggttgaagatccacggtgcgaactgcgcaggggtggataaggtaccgttcccggaacgtattaaattcatcgaggaaaaccacgaaaacattatggcgtgcgcaaagagcccgctggaaaacacgtggtgggcagagcaggacagtccattctgcttcttggcgttctgtttcgaatatgcaggtgtccagcaccacggcctgagctataactgcagcctgccgctggcctttgatggttcttgtagcggtattcaacactttagcgccatgctgcgcgatgaggttggtggcagagcagtgaatctgctgccaagcgaaaccgtgcaagatatctatggcattgtggctaagaaggttaatgaaatcctgcaagcagacgcgattaacggcacggacaacgaggttgtcaccgtgaccgatgaaaacaccggtgagatctcggagaaagtgaaactgggcaccaaagccttggctggccaatggctggcatacggcgttactcgctccgtgaccaagcgttcggtgatgacccttgcttacggcagcaaagagtttggtttccgccaacaggttctggaggatactatccaaccggccatcgactctggtaaaggcctgatgttcacgcagccgaatcaggcagcgggctatatggcgaagctgatttgggaatcggttagcgttaccgttgttgcagcggtggaggctatgaactggctgaaatctgcggcgaagctgttagctgcggaggtgaaggacaagaagacgggcgaaatcctgcgtaagcgctgcgcagtgcattgggttacgccggatggttttccggtatggcaggagtacaaaaagcctattcagacccgtctgaacctgatgtttctgggtcaatttcgtctgcagccgacgatcaacaccaataaggactccgagatcgacgcgcacaaacaggagtctggcatcgcacccaatttcgttcactcacaggacggttcccatctgcgtaagaccgtcgtgtgggcacacgagaagtatggcattgagtcgtttgcattgatccacgattcctttggtaccatcccggcggacgctgcgaacctgtttaaagcggttcgcgaaaccatggttgacacctatgaaagttgcgatgttctggcagacttttatgatcagttcgccgaccaactgcatgagtcccagctggataaaatgccggcgttaccggcgaagggcaacttaaatctccgcgacatcctggaatctgatttcgccttcgcgtaa

SEQ ID NO: 71 - DNA, 2652 bp, synthetic construct
  source 1..2652: mol_type = other DNA
atgaatacaattaacatagctaaaaatgatttcagcgatattgaactggctgcgatcccgtttaataccttggcggaccattatggtgagcgtctggcgcgtgagcaacttgctctggagcacgaatcctacgagatgggtgaagcgcgtttccggaagatgttcgagcgccagcttaaggctggcgaggtggcggataacgctgctgcgaagccgttgattacgaccctgctgccgaaaatgattgcgcgtattaacgattggttcgaggaagtgaaagcaaagcgtggtaaacgtccaaccgcattccagtttctgcaagagatcaagccggaggcggtggcatacattacgatcaaaaccactctcgcatgtctcaccagcgcggataatactacggtccaagcggtggccagcgcgattggccgcgcgattgaggacgaagcgcgttttggtcgcattcgtgacctggaagcgaaacattttaagaagaacgttgaagaacaattgaatggacgcgtgggccacgtttacaagaaagcgttcatgcaagtcgttgaagctgatatgctgagcaaaggcctgttaggtggtgaagcatggagcagctggcataaggaggactcaattcacgtcggcgtgcggtgcattgaaatgctgatcgaatcgaccggtatggttagcctgcatcgccaaaacgccggcgtggtgggtcaagatagcgaaacgattgaactggcgccagagtacgcggaagctatcgctaccagagccggcgcattggcggggatcagcccgatgttccagccgtgtgttgtaccaccgaagccgtggaccggtatcaccggtggaggttactgggcgaatggtagacgtccgttggcgttggttcgtacccatagcaaaaaggctctgatgcgttatgaagacgtttacatgccggaagtgtacaaagccatcaacatcgcgcagaacactgcgtggaaaatcaacaaaaaggtgttagctgtggcgaacgtaattacaaaatggaagcactgcccggttgaggacatcccggctattgaacgtgaagagctgccaatgaaaccagaggacattgacatgaatccggaggcgctgaccgcatggaaacgtgcggcagcagcggtctatcgtaaggataaagccagaaagagccgtcgtatctccctggaattcatgcttgagcaggcgaacaaattcgctaaccacaaagccatctggtttccgtataatatggattggcgtggtcgtgtttacgcggtatcgatgttcaacccgcagggtaatgacatgaccaagggtttgttgaccttggccaaaggtaaaccgattggcaaagaaggttactattggttgaagatccacggtgcgaactgcgcaggggtggataaggtaccgttcccggaacgtattaaattcatcgaggaaaaccacgaaaacattatggcgtgcgcaaagagcccgctggaaaacacgtggtgggcagagcaggacagtccattctgcttcttggcgttctgtttcgaatatgcaggtgtccagcaccacggcctgagctataactgcagcctgccgctggcctttgatggttcttgtagcggtattcaacactttagcgccatgctgcgcgatgaggttggtggcagagcagtgaatctgctgccaagcgaaaccgtgcaagatatctatggcattgtggctaagaaggttaatgaaatcctgcaagcagacgcgattaacggcacggacaacgaggttgtcaccgtgaccgatgaaaacaccggtgagatctcggagaaagtgaaactgggcaccaaagccttggctggccaatggctggcatacggcgttactcgctccgtgaccaagcgttcggtgatgacccttgcttacggcagcaaagagtttggtttccgccaacaggttctggaggatactatccaaccggccatcgactctggtaaaggcctgatgttcacgcagccgaatcaggcagcgggctatatggcgaagctgatttgggaatcggttagcgttaccgttgttgcagcggtggaggctatgaactggctgaaatctgcggcgaagctgttagctgcggaggtgaaggacaagaagacgggcgaaatcctgcgtaagcgctgcgcagtgcattgggttacgccggatggttttccggtatggcaggagtacaaaaagcctattcagacccgtctgaacctgatgtttctgggtcaatttcgtctgcagccgacgatcaacaccaataaggactccgagatcgacgcgcacaaacaggagtctggcatcgcacccaatttcgttcactcacaggacggttcccatctgcgtaagaccgtcgtgtgggcacacgagaagtatggcattgagtcgtttgcattgatccacgattcctttggtaccatcccggcggacgctgcgaacctgtttaaagcggttcgcgaaaccatggttgacacctatgaaagttgcgatgttctggcagacttttatgatcagttcgccgaccaactgcatgagtcccagctggataaaatgccggcgttaccggcgaagggcaacttaaatctccgcgacatcctggaatctgatttcgccttcgcgtaa

SEQ ID NO: 72 - DNA, 2652 bp, synthetic construct
  source 1..2652: mol_type = other DNA
atgaatacaattaacatagctaaaaatgatttcagcgatattgaactggctgcgatcccgtttaataccttggcggaccattatggtgagcgtctggcgcgtgagcaacttgctctggagcacgaatcctacgagatgggtgaagcgcgtttccggaagatgttcgagcgccagcttaaggctggcgaggtggcggataacgctgctgcgaagccgttgattacgaccctgctgccgaaaatgattgcgcgtattaacgattggttcgaggaagtgaaagcaaagcgtggtaaacgtccaaccgcattccagtttctgcaagagatcaagccggaggcggtggcatacattacgatcaaaaccactctcgcatgtctcaccagcgcggataatactacggtccaagcggtggccagcgcgattggccgcgcgattgaggacgaagcgcgttttggtcgcattcgtgacctggaagcgaaacattttaagaagaacgttgaagaacaattgaatccacgcgtgggccacgtttacaagaaagcgttcatgcaagtcgttgaagctgatatgctgagcaaaggcctgttaggtggtgaagcatggagcagctggcataaggaggactcaattcacgtcggcgtgcggtgcattgaaatgctgatcgaatcgaccggtatggttagcctgcatcgccaaaacgccggcgtggtgggtcaagatagcgaaacgattgaactggcgccagagtacgcggaagctatcgctaccagagccggcgcattggcggggatcagcccgatgttccagccgtgtgttgtaccaccgaagccgtggaccggtatcaccggtggaggttactgggcgaatggtagacgtccgttggcgttggttcgtacccatagcaaaaaggctctgatgcgttatgaagacgtttacatgccggaagtgtacaaagccatcaacatcgcgcagaacactgcgtggaaaatcaacaaaaaggtgttagctgtggcgaacgtaattacaaaatggaagcactgcccggttgaggacatcccggctattgaacgtgaagagctgccaatgaaaccagaggacattgacatgaatccggaggcgctgaccgcatggaaacgtgcggcagcagcggtctatcgtaaggataaagccagaaagagccgtcgtatctccctggaattcatgcttgagcaggcgaacaaattcgctaaccacaaagccatctggtttccgtataatatggattggcgtggtcgtgtttacgcggtatcgatgttcaacccgcagggtaatgacatgaccaagggtttgttgaccttggccaaaggtaaaccgattggcaaagaaggttactattggttgaagatccacggtgcgaactgcgcaggggtggataaggtaccgttcccggaacgtattaaattcatcgaggaaaaccacgaaaacattatggcgtgcgcaaagagcccgctggaaaacacgtggtgggcagagcaggacagtccattctgcttcttggcgttctgtttcgaatatgcaggtgtccagcaccacggcctgagctataactgcagcctgccgctggcctttgatggttcttgtagcggtattcaacactttagcgccatgctgcgcgatgaggttggtggcagagcagtgaatctgctgccaagcgaaaccgtgcaagatatctatggcattgtggctaagaaggttaatgaaatcctgcaagcagacgcgattaacggcacggacaacgaggttgtcaccgtgaccgatgaaaacaccggtgagatctcggagaaagtgaaactgggcaccaaagccttggctggccaatggctggcatacggcgttactcgctccgtgaccaagcgttcggtgatgacccttgcttacggcagcaaagagtttggtttccgccaacaggttctggaggatactatccaaccggccatcgactctggtaaaggcctgatgttcacgcagccgaatcaggcagcgggctatatggcgaagctgatttgggaatcggttagcgttaccgttgttgcagcggtggaggctatgaactggctgaaatctgcggcgaagctgttagctgcggaggtgaaggacaagaagacgggcgaaatcctgcgtaagcgctgcgcagtgcattgggttacgccggatggttttccggtatggcaggagtacaaaaagcctattcagacccgtctgaacctgatgtttctgggtcaatttcgtctgcagccgacgatcaacaccaataaggactccgagatcgacgcgcacaaacaggagtctggcatcgcacccaatttcgttcactcacaggacggttcccatctgcgtaagaccgtcgtgtgggcacacgagaagtatggcattgagtcgtttgcattgatccacgattcctttggtaccatcccggcggacgctgcgaacctgtttaaagcggttcgcgaaaccatggttgacacctatgaaagttgcgatgttctggcagacttttatgatcagttcgccgaccaactgcatgagtcccagctggataaaatgccggcgttaccggcgaagggcaacttaaatctccgcgacatcctggaatctgatttcgccttcgcgtaa

SEQ ID NO: 73 - DNA, 2652 bp, synthetic construct
  source 1..2652: mol_type = other DNA
atgaatacaattaacatagctaaaaatgatttcagcgatattgaactggctgcgatcccgtttaataccttggcggaccattatggtgagcgtctggcgcgtgagcaacttgctctggagcacgaatcctacgagatgggtgaagcgcgtttccggaagatgttcgagcgccagcttaaggctggcgaggtggcggataacgctgctgcgaagccgttgattacgaccctgctgccgaaaatgattgcgcgtattaacgattggttcgaggaagtgaaagcaaagcgtggtaaacgtccaaccgcattccagtttctgcaagagatcaagccggaggcggtggcatacattacgatcaaaaccactctcgcatgtctcaccagcgcggataatactacggtccaagcggtggccagcgcgattggccgcgcgattgaggacgaagcgcgttttggtcgcattcgtgacctggaagcgaaacattttaagaagaacgttgaagaacaagataataaacgcgtgggccacgtttacaagaaagcgttcatgcaagtcgttgaagctgatatgctgagcaaaggcctgttaggtggtgaagcatggagcagctggcataaggaggactcaattcacgtcggcgtgcggtgcattgaaatgctgatcgaatcgaccggtatggttagcctgcatcgccaaaacgccggcgtggtgggtcaagatagcgaaacgattgaactggcgccagagtacgcggaagctatcgctaccagagccggcgcattggcggggatcagcccgatgttccagccgtgtgttgtaccaccgaagccgtggaccggtatcaccggtggaggttactgggcgaatggtagacgtccgttggcgttggttcgtacccatagcaaaaaggctctgatgcgttatgaagacgtttacatgccggaagtgtacaaagccatcaacatcgcgcagaacactgcgtggaaaatcaacaaaaaggtgttagctgtggcgaacgtaattacaaaatggaagcactgcccggttgaggacatcccggctattgaacgtgaagagctgccaatgaaaccagaggacattgacatgaatccggaggcgctgaccgcatggaaacgtgcggcagcagcggtctatcgtaaggataaagccagaaagagccgtcgtatctccctggaattcatgcttgagcaggcgaacaaattcgctaaccacaaagccatctggtttccgtataatatggattggcgtggtcgtgtttacgcggtatcgatgttcaacccgcagggtaatgacatgaccaagggtttgttgaccttggccaaaggtaaaccgattggcaaagaaggttactattggttgaagatccacggtgcgaactgcgcaggggtggataaggtaccgttcccggaacgtattaaattcatcgaggaaaaccacgaaaacattatggcgtgcgcaaagagcccgctggaaaacacgtggtgggcagagcaggacagtccattctgcttcttggcgttctgtttcgaatatgcaggtgtccagcaccacggcctgagctataactgcagcctgccgctggcctttgatggttcttgtagcggtattcaacactttagcgccatgctgcgcgatgaggttggtggcagagcagtgaatctgctgccaagcgaaaccgtgcaagatatctatggcattgtggctaagaaggttaatgaaatcctgcaagcagacgcgattaacggcacggacaacgaggttgtcaccgtgaccgatgaaaacaccggtgagatctcggagaaagtgaaactgggcaccaaagccttggctggccaatggctggcatacggcgttactcgctccgtgaccaagcgttcggtgatgacccttgcttacggcagcaaagagtttggtttccgccaacaggttctggaggatactatccaaccggccatcgactctggtaaaggcctgatgttcacgcagccgaatcaggcagcgggctatatggcgaagctgatttgggaatcggttagcgttaccgttgttgcagcggtggaggctatgaactggctgaaatctgcggcgaagctgttagctgcggaggtgaaggacaagaagacgggcgaaatcctgcgtaagcgctgcgcagtgcattgggttacgccggatggttttccggtatggcaggagtacaaaaagcctattcagacccgtctgaacctgatgtttctgggtcaatttcgtctgcagccgacgatcaacaccaataaggactccgagatcgacgcgcacaaacaggagtctggcatcgcacccaatttcgttcactcacaggacggttcccatctgcgtaagaccgtcgtgtgggcacacgagaagtatggcattgagtcgtttgcattgatccacgattcctttggtaccatcccggcggacgctgcgaacctgtttaaagcggttcgcgaaaccatggttgacacctatgaaagttgcgatgttctggcagacttttatgatcagttcgccgaccaactgcatgagtcccagctggataaaatgccggcgttaccggcgaagggcaacttaaatctccgcgacatcctggaatctgatttcgccttcgcgtaa

SEQ ID NO: 74 - DNA, 2652 bp, synthetic construct
  source 1..2652: mol_type = other DNA
atgaatacaattaacatagctaaaaatgatttcagcgatattgaactggctgcgatcccgtttaataccttggcggaccattatggtgagcgtctggcgcgtgagcaacttgctctggagcacgaatcctacgagatgggtgaagcgcgtttccggaagatgttcgagcgccaggctaaggctggcgaggtggcggataacgctgctgcgaagccgttgattacgaccctgctgccgaaaatgattgcgcgtattaacgattggttcgaggaagtgaaagcaaagcgtggtaaacgtccaaccgcattccagtttctgcaagagatcaagccggaggcggtggcatacattacgatcaaaaccactctcgcatgtctcaccagcgcggataatactacggtccaagcggtggccagcgcgattggccgcgcgattgaggacgaagcgcgttttggtcgcattcgtgacctggaagcgaaacattttaagaagaacgttgaagaacaattgaataaacgcgtgggccacgtttacaagaaagcgttcatgcaagtcgttgaagctgatatgctgagcaaaggcctgttaggtggtgaagcatggagcagctggcataaggaggactcaattcacgtcggcgtgcggtgcattgaaatgctgatcgaatcgaccggtatggttagcctgcatcgccaaaacgccggcgtggtgggtcaagatagcgaaacgattgaactggcgccagagtacgcggaagctatcgctaccagagccggcgcattggcggggatcagcccgatgttccagccgtgtgttgtaccaccgaagccgtggaccggtatcaccggtggaggttactgggcgaatggtagacgtccgttggcgttggttcgtacccatagcaaaaaggctctgatgcgttatgaagacgtttacatgccggaagtgtacaaagccatcaacatcgcgcagaacactgcgtggaaaatcaacaaaaaggtgttagctgtggcgaacgtaattacaaaatggaagcactgcccggttgaggacatcccggctattgaacgtgaagagctgccaatgaaaccagaggacattgacatgaatccggaggcgctgaccgcatggaaacgtgcggcagcagcggtctatcgtaaggataaagccagaaagagccgtcgtatctccctggaattcatgcttgagcaggcgaacaaattcgctaaccacaaagccatctggtttccgtataatatggattggcgtggtcgtgtttacgcggtatcgatgttcaacccgcagggtaatgacatgaccaagggtttgttgaccttggccaaaggtaaaccgattggcaaagaaggttactattggttgaagatccacggtgcgaactgcgcaggggtggataaggtaccgttcccggaacgtattaaattcatcgaggaaaaccacgaaaacattatggcgtgcgcaaagagcccgctggaaaacacgtggtgggcagagcaggacagtccattctgcttcttggcgttctgtttcgaatatgcaggtgtccagcaccacggcctgagctataactgcagcctgccgctggcctttgatggttcttgtagcggtattcaacactttagcgccatgctgcgcgatgaggttggtggcagagcagtgaatctgctgccaagcgaaaccgtgcaagatatctatggcattgtggctaagaaggttaatgaaatcctgcaagcagacgcgattaacggcacggacaacgaggttgtcaccgtgaccgatgaaaacaccggtgagatctcggagaaagtgaaactgggcaccaaagccttggctggccaatggctggcatacggcgttactcgctccgtgaccaagcgttcggtgatgacccttgcttacggcagcaaagagtttggtttccgccaacaggttctggaggatactatccaaccggccatcgactctggtaaaggcctgatgttcacgcagccgaatcaggcagcgggctatatggcgaagctgatttgggaatcggttagcgttaccgttgttgcagcggtggaggctatgaactggctgaaatctgcggcgaagctgttagctgcggaggtgaaggacaagaagacgggcgaaatcctgcgtaagcgctgcgcagtgcattgggttacgccggatggttttccggtatggcaggagtacaaaaagcctattcagacccgtctgaacctgatgtttctgggtcaatttcgtctgcagccgacgatcaacaccaataaggactccgagatcgacgcgcacaaacaggagtctggcatcgcacccaatttcgttcactcacaggacggttcccatctgcgtaagaccgtcgtgtgggcacacgagaagtatggcattgagtcgtttgcattgatccacgattcctttggtaccatcccggcggacgctgcgaacctgtttaaagcggttcgcgaaaccatggttgacacctatgaaagttgcgatgttctggcagacttttatgatcagttcgccgaccaactgcatgagtcccagctggataaaatgccggcgttaccggcgaagggcaacttaaatctccgcgacatcctggaatctgatttcgccttcgcgtaa

SEQ ID NO: 75 - DNA, 2652 bp, synthetic construct
  source 1..2652: mol_type = other DNA
atgaatacaattaacatagctaaaaatgatttcagcgatattgaactggctgcgatcccgtttaataccttggcggaccattatggtgagcgtctggcgcgtgagcaacttgctctggagcacgaatcctacgagatgggtgaagcgcgtttccggaagatgttcgagcgccagcttaaggctggcgaggtggcggataacgctgctgcgaagccgttgattacgaccctgctgccgaaaatgattgcgcgtattaacgattggttcgaggaagtgaaagcaaagcgtggtaaacgtccaaccgcattccagtttctgcaagagatcaagccggaggcggtggcatacattacgatcaaaaccactctcgcatgtctcaccagcgcggataatactacggtccaagcggtggccagcgcgattggccgcgcgattgaggacgaagcgcgttttggtcgcattcgtgacctggaagcgaaacattttaagaagaacgttgaagaacaattgaataaacgcgtgggccacgttcctaagaaagcgttcatgcaagtcgttgaagctgatatgctgagcaaaggcctgttaggtggtgaagcatggagcagctggcataaggaggactcaattcacgtcggcgtgcggtgcattgaaatgctgatcgaatcgaccggtatggttagcctgcatcgccaaaacgccggcgtggtgggtcaagatagcgaaacgattgaactggcgccagagtacgcggaagctatcgctaccagagccggcgcattggcggggatcagcccgatgttccagccgtgtgttgtaccaccgaagccgtggaccggtatcaccggtggaggttactgggcgaatggtagacgtccgttggcgttggttcgtacccatagcaaaaaggctctgatgcgttatgaagacgtttacatgccggaagtgtacaaagccatcaacatcgcgcagaacactgcgtggaaaatcaacaaaaaggtgttagctgtggcgaacgtaattacaaaatggaagcactgcccggttgaggacatcccggctattgaacgtgaagagctgccaatgaaaccagaggacattgacatgaatccggaggcgctgaccgcatggaaacgtgcggcagcagcggtctatcgtaaggataaagccagaaagagccgtcgtatctccctggaattcatgcttgagcaggcgaacaaattcgctaaccacaaagccatctggtttccgtataatatggattggcgtggtcgtgtttacgcggtatcgatgttcaacccgcagggtaatgacatgaccaagggtttgttgaccttggccaaaggtaaaccgattggcaaagaaggttactattggttgaagatccacggtgcgaactgcgcaggggtggataaggtaccgttcccggaacgtattaaattcatcgaggaaaaccacgaaaacattatggcgtgcgcaaagagcccgctggaaaacacgtggtgggcagagcaggacagtccattctgcttcttggcgttctgtttcgaatatgcaggtgtccagcaccacggcctgagctataactgcagcctgccgctggcctttgatggttcttgtagcggtattcaacactttagcgccatgctgcgcgatgaggttggtggcagagcagtgaatctgctgccaagcgaaaccgtgcaagatatctatggcattgtggctaagaaggttaatgaaatcctgcaagcagacgcgattaacggcacggacaacgaggttgtcaccgtgaccgatgaaaacaccggtgagatctcggagaaagtgaaactgggcaccaaagccttggctggccaatggctggcatacggcgttactcgctccgtgaccaagcgttcggtgatgacccttgcttacggcagcaaagagtttggtttccgccaacaggttctggaggatactatccaaccggccatcgactctggtaaaggcctgatgttcacgcagccgaatcaggcagcgggctatatggcgaagctgatttgggaatcggttagcgttaccgttgttgcagcggtggaggctatgaactggctgaaatctgcggcgaagctgttagctgcggaggtgaaggacaagaagacgggcgaaatcctgcgtaagcgctgcgcagtgcattgggttacgccggatggttttccggtatggcaggagtacaaaaagcctattcagacccgtctgaacctgatgtttctgggtcaatttcgtctgcagccgacgatcaacaccaataaggactccgagatcgacgcgcacaaacaggagtctggcatcgcacccaatttcgttcactcacaggacggttcccatctgcgtaagaccgtcgtgtgggcacacgagaagtatggcattgagtcgtttgcattgatccacgattcctttggtaccatcccggcggacgctgcgaacctgtttaaagcggttcgcgaaaccatggttgacacctatgaaagttgcgatgttctggcagacttttatgatcagttcgccgaccaactgcatgagtcccagctggataaaatgccggcgttaccggcgaagggcaacttaaatctccgcgacatcctggaatctgatttcgccttcgcgtaa

SEQ ID NO: 76 - DNA, 2652 bp, synthetic construct
  source 1..2652: mol_type = other DNA
atgaatacaattaacatagctaaaaatgatttcagcgatattgaactggctgcgatcccgtttaataccttggcggaccattatggtgagcgtctggcgcgtgagcaacttgctctggagcacgaatcctacgagatgggtgaagcgcgtttccggaagatgttcgagcgccagcttaaggctggcgaggtggcggataacgctgctgcgaagccgttgattacgaccctgctgccgaaaatgattgcgcgtattaacgattggttcgaggaagtgaaagcaaagcgtggtaaacgtccaaccgcattccagtttctgcaagagatcaagccggaggcggtggcatacattacgatcaaaaccactctcgcatgtctcaccagcgcggataatactacggtccaagcggtggccagcgcgattggccgcgcgattgaggacgaagcgcgttttggtcgcattcgtgacctggaagcgaaacattttaagaagaacgttgaagaacaattgaataaacgcgtgggccacgttggaaagaaagcgttcatgcaagtcgttgaagctgatatgctgagcaaaggcctgttaggtggtgaagcatggagcagctggcataaggaggactcaattcacgtcggcgtgcggtgcattgaaatgctgatcgaatcgaccggtatggttagcctgcatcgccaaaacgccggcgtggtgggtcaagatagcgaaacgattgaactggcgccagagtacgcggaagctatcgctaccagagccggcgcattggcggggatcagcccgatgttccagccgtgtgttgtaccaccgaagccgtggaccggtatcaccggtggaggttactgggcgaatggtagacgtccgttggcgttggttcgtacccatagcaaaaaggctctgatgcgttatgaagacgtttacatgccggaagtgtacaaagccatcaacatcgcgcagaacactgcgtggaaaatcaacaaaaaggtgttagctgtggcgaacgtaattacaaaatggaagcactgcccggttgaggacatcccggctattgaacgtgaagagctgccaatgaaaccagaggacattgacatgaatccggaggcgctgaccgcatggaaacgtgcggcagcagcggtctatcgtaaggataaagccagaaagagccgtcgtatctccctggaattcatgcttgagcaggcgaacaaattcgctaaccacaaagccatctggtttccgtataatatggattggcgtggtcgtgtttacgcggtatcgatgttcaacccgcagggtaatgacatgaccaagggtttgttgaccttggccaaaggtaaaccgattggcaaagaaggttactattggttgaagatccacggtgcgaactgcgcaggggtggataaggtaccgttcccggaacgtattaaattcatcgaggaaaaccacgaaaacattatggcgtgcgcaaagagcccgctggaaaacacgtggtgggcagagcaggacagtccattctgcttcttggcgttctgtttcgaatatgcaggtgtccagcaccacggcctgagctataactgcagcctgccgctggcctttgatggttcttgtagcggtattcaacactttagcgccatgctgcgcgatgaggttggtggcagagcagtgaatctgctgccaagcgaaaccgtgcaagatatctatggcattgtggctaagaaggttaatgaaatcctgcaagcagacgcgattaacggcacggacaacgaggttgtcaccgtgaccgatgaaaacaccggtgagatctcggagaaagtgaaactgggcaccaaagccttggctggccaatggctggcatacggcgttactcgctccgtgaccaagcgttcggtgatgacccttgcttacggcagcaaagagtttggtttccgccaacaggttctggaggatactatccaaccggccatcgactctggtaaaggcctgatgttcacgcagccgaatcaggcagcgggctatatggcgaagctgatttgggaatcggttagcgttaccgttgttgcagcggtggaggctatgaactggctgaaatctgcggcgaagctgttagctgcggaggtgaaggacaagaagacgggcgaaatcctgcgtaagcgctgcgcagtgcattgggttacgccggatggttttccggtatggcaggagtacaaaaagcctattcagacccgtctgaacctgatgtttctgggtcaatttcgtctgcagccgacgatcaacaccaataaggactccgagatcgacgcgcacaaacaggagtctggcatcgcacccaatttcgttcactcacaggacggttcccatctgcgtaagaccgtcgtgtgggcacacgagaagtatggcattgagtcgtttgcattgatccacgattcctttggtaccatcccggcggacgctgcgaacctgtttaaagcggttcgcgaaaccatggttgacacctatgaaagttgcgatgttctggcagacttttatgatcagttcgccgaccaactgcatgagtcccagctggataaaatgccggcgttaccggcgaagggcaacttaaatctccgcgacatcctggaatctgatttcgccttcgcgtaa

SEQ ID NO: 77 - DNA, 2652 bp, synthetic construct
  source 1..2652: mol_type = other DNA
atgaatacaattaacatagctaaaaatgatttcagcgatattgaactggctgcgatcccgtttaataccttggcggaccattatggtgagcgtctggcgcgtgagcaacttgctctggagcacgaatcctacgagatgggtgaagcgcgtttccggaagatgttcgagcgccagcttaaggctggcgaggtggcggataacgctgctgcgaagccgttgattacgaccctgctgccgaaaatgattgcgcgtattaacgattggttcgaggaagtgaaagcaaagcgtggtaaacgtccaaccgcattccagtttctgcaagagatcaagccggaggcggtggcatacattacgatcaaaaccactctcgcatgtctcaccagcgcggataatactacggtccaagcggtggccagcgcgattggccgcgcgattgaggacgaagcgcgttttggtcgcattcgtgacctggaagcgaaacattttaagaagaacgttgaagaacaattgaataaacgcgtgggccacgtttacaagaaagcgttcgaacaagtcgttgaagctgatatgctgagcaaaggcctgttaggtggtgaagcatggagcagctggcataaggaggactcaattcacgtcggcgtgcggtgcattgaaatgctgatcgaatcgaccggtatggttagcctgcatcgccaaaacgccggcgtggtgggtcaagatagcgaaacgattgaactggcgccagagtacgcggaagctatcgctaccagagccggcgcattggcggggatcagcccgatgttccagccgtgtgttgtaccaccgaagccgtggaccggtatcaccggtggaggttactgggcgaatggtagacgtccgttggcgttggttcgtacccatagcaaaaaggctctgatgcgttatgaagacgtttacatgccggaagtgtacaaagccatcaacatcgcgcagaacactgcgtggaaaatcaacaaaaaggtgttagctgtggcgaacgtaattacaaaatggaagcactgcccggttgaggacatcccggctattgaacgtgaagagctgccaatgaaaccagaggacattgacatgaatccggaggcgctgaccgcatggaaacgtgcggcagcagcggtctatcgtaaggataaagccagaaagagccgtcgtatctccctggaattcatgcttgagcaggcgaacaaattcgctaaccacaaagccatctggtttccgtataatatggattggcgtggtcgtgtttacgcggtatcgatgttcaacccgcagggtaatgacatgaccaagggtttgttgaccttggccaaaggtaaaccgattggcaaagaaggttactattggttgaagatccacggtgcgaactgcgcaggggtggataaggtaccgttcccggaacgtattaaattcatcgaggaaaaccacgaaaacattatggcgtgcgcaaagagcccgctggaaaacacgtggtgggcagagcaggacagtccattctgcttcttggcgttctgtttcgaatatgcaggtgtccagcaccacggcctgagctataactgcagcctgccgctggcctttgatggttcttgtagcggtattcaacactttagcgccatgctgcgcgatgaggttggtggcagagcagtgaatctgctgccaagcgaaaccgtgcaagatatctatggcattgtggctaagaaggttaatgaaatcctgcaagcagacgcgattaacggcacggacaacgaggttgtcaccgtgaccgatgaaaacaccggtgagatctcggagaaagtgaaactgggcaccaaagccttggctggccaatggctggcatacggcgttactcgctccgtgaccaagcgttcggtgatgacccttgcttacggcagcaaagagtttggtttccgccaacaggttctggaggatactatccaaccggccatcgactctggtaaaggcctgatgttcacgcagccgaatcaggcagcgggctatatggcgaagctgatttgggaatcggttagcgttaccgttgttgcagcggtggaggctatgaactggctgaaatctgcggcgaagctgttagctgcggaggtgaaggacaagaagacgggcgaaatcctgcgtaagcgctgcgcagtgcattgggttacgccggatggttttccggtatggcaggagtacaaaaagcctattcagacccgtctgaacctgatgtttctgggtcaatttcgtctgcagccgacgatcaacaccaataaggactccgagatcgacgcgcacaaacaggagtctggcatcgcacccaatttcgttcactcacaggacggttcccatctgcgtaagaccgtcgtgtgggcacacgagaagtatggcattgagtcgtttgcattgatccacgattcctttggtaccatcccggcggacgctgcgaacctgtttaaagcggttcgcgaaaccatggttgacacctatgaaagttgcgatgttctggcagacttttatgatcagttcgccgaccaactgcatgagtcccagctggataaaatgccggcgttaccggcgaagggcaacttaaatctccgcgacatcctggaatctgatttcgccttcgcgtaa

SEQ ID NO: 78 - DNA, 2652 bp, synthetic construct
  source 1..2652: mol_type = other DNA
atgaatacaattaacatagctaaaaatgatttcagcgatattgaactggctgcgatcccgtttaataccttggcggaccattatggtgagcgtctggcgcgtgagcaacttgctctggagcacgaatcctacgagatgggtgaagcgcgtttcgcgaagatgttcgagcgccagcttaaggctggcgaggtggcggataacgctgctgcgaagccgttgattacgaccctgctgccgaaaatgattgcgcgtattaacgattggttcgaggaagtgaaagcaaagcgtggtaaacgtccaaccgcattccagtttctgcaagagatcaagccggaggcggtggcatacattacgatcaaaaccactctcgcatgtctcaccagcgcggataatactacggtccaagcggtggccagcgcgattggccgcgcgattgaggacgaagcgcgttttggtcgcattcgtgacctggaagcgaaacattttaagaagaacgttgaagaacaattgaataaacgcgtgggccacgtttacaagaaagcgttcatgcaagtcgttgaagctgatatgctgagcaaaggcctgttaggtggtgaagcatggagcagctggcataaggaggactcaattcacgtcggcgtgcggtgcattgaaatgctgatcgaatcgaccggtatggttagcctgcatcgccaaaacgccggcgtggtgggtcaagatagcgaaacgattgaactggcgccagagtacgcggaagctatcgctaccagagccggcgcattggcggggatcagcccgatgttccagccgtgtgttgtaccaccgaagccgtggaccggtatcaccggtggaggttactgggcgaatggtagacgtccgttggcgttggttcgtacccatagcaaaaaggctctgatgcgttatgaagacgtttacatgccggaagtgtacaaagccatcaacatcgcgcagaacactgcgtggaaaatcaacaaaaaggtgttagctgtggcgaacgtaattacaaaatggaagcactgcccggttgaggacatcccggctattgaacgtgaagagctgccaatgaaaccagaggacattgacatgaatccggaggcgctgaccgcatggaaacgtgcggcagcagcggtctatcgtaaggataaagccagaaagagccgtcgtatctccctggaattcatgcttgagcaggcgaacaaattcgctaaccacaaagccatctggtttccgtataatatggattggcgtggtcgtgtttacgcggtatcgatgttcaacccgcagggtaatgacatgaccaagggtttgttgaccttggccaaaggtaaaccgattggcaaagaaggttactattggttgaagatccacggtgcgaactgcgcaggggtggataaggtaccgttcccggaacgtattaaattcatcgaggaaaaccacgaaaacattatggcgtgcgcaaagagcccgctggaaaacacgtggtgggcagagcaggacagtccattctgcttcttggcgttctgtttcgaatatgcaggtgtccagcaccacggcctgagctataactgcagcctgccgctggcctttgatggttcttgtagcggtattcaacactttagcgccatgctgcgcgatgaggttggtggcagagcagtgaatctgctgccaagcgaaaccgtgcaagatatctatggcattgtggctaagaaggttaatgaaatcctgcaagcagacgcgattaacggcacggacaacgaggttgtcaccgtgaccgatgaaaacaccggtgagatctcggagaaagtgaaactgggcaccaaagccttggctggccaatggctggcatacggcgttactcgctccgtgaccaagcgttcggtgatgacccttgcttacggcagcaaagagtttggtttccgccaacaggttctggaggatactatccaaccggccatcgactctggtaaaggcctgatgttcacgcagccgaatcaggcagcgggctatatggcgaagctgatttgggaatcggttagcgttaccgttgttgcagcggtggaggctatgaactggctgaaatctgcggcgaagctgttagctgcggaggtgaaggacaagaagacgggcgaaatcctgcgtaagcgctgcgcagtgcattgggttacgccggatggttttccggtatggcaggagtacaaaaagcctattcagacccgtctgaacctgatgtttctgggtcaatttcgtctgcagccgacgatcaacaccaataaggactccgagatcgacgcgcacaaacaggagtctggcatcgcacccaatttcgttcactcacaggacggttcccatctgcgtaagaccgtcgtgtgggcacacgagaagtatggcattgagtcgtttgcattgatccacgattcctttggtaccatcccggcggacgctgcgaacctgtttaaagcggttcgcgaaaccatggttgacacctatgaaagttgcgatgttctggcagacttttatgatcagttcgccgaccaactgcatgagtcccagctggataaaatgccggcgttaccggcgaagggcaacttaaatctccgcgacatcctggaatctgatttcgccttcgcgtaa

SEQ ID NO: 79 - DNA, 2652 bp, synthetic construct
  source 1..2652: mol_type = other DNA
atgaatacaattaacatagctaaaaatgatttcagcgatattgaactggctgcgatcccgtttaataccttggcggaccattatggtgagcgtctggcgcgtgagcaacttgctctggagcacgaatcctacgagatgggtgaagcgcgtttccggaagatgttcgagcgccagcttaaggctggcgaggtggcggataacgctgctgcgaagccgttgattacgaccctgctgccgaaaatgattgcgcgtattaacgattggttcgaggaagtgaaagcaaagcgtggtaaacgtccaaccgcattccagtttctgcaagagatcaagccggaggcggtggcatacattacgatcaaaaccactctcgcatgtctcaccagcgcggataatactacggtccaagcggtggccagcgcgattggccgcgcgattgaggacgaagcgcgttttggtcgcattcgtgacctggaagcgaaacattttaagaagaacgttgaagaacaattgaataaacgcgtgggccacgttcacaagaaagcgttcatgcaagtcgttgaagctgatatgctgagcaaaggcctgttaggtggtgaagcatggagcagctggcataaggaggactcaattcacgtcggcgtgcggtgcattgaaatgctgatcgaatcgaccggtatggttagcctgcatcgccaaaacgccggcgtggtgggtcaagatagcgaaacgattgaactggcgccagagtacgcggaagctatcgctaccagagccggcgcattggcggggatcagcccgatgttccagccgtgtgttgtaccaccgaagccgtggaccggtatcaccggtggaggttactgggcgaatggtagacgtccgttggcgttggttcgtacccatagcaaaaaggctctgatgcgttatgaagacgtttacatgccggaagtgtacaaagccatcaacatcgcgcagaacactgcgtggaaaatcaacaaaaaggtgttagctgtggcgaacgtaattacaaaatggaagcactgcccggttgaggacatcccggctattgaacgtgaagagctgccaatgaaaccagaggacattgacatgaatccggaggcgctgaccgcatggaaacgtgcggcagcagcggtctatcgtaaggataaagccagaaagagccgtcgtatctccctggaattcatgcttgagcaggcgaacaaattcgctaaccacaaagccatctggtttccgtataatatggattggcgtggtcgtgtttacgcggtatcgatgttcaacccgcagggtaatgacatgaccaagggtttgttgaccttggccaaaggtaaaccgattggcaaagaaggttactattggttgaagatccacggtgcgaactgcgcaggggtggataaggtaccgttcccggaacgtattaaattcatcgaggaaaaccacgaaaacattatggcgtgcgcaaagagcccgctggaaaacacgtggtgggcagagcaggacagtccattctgcttcttggcgttctgtttcgaatatgcaggtgtccagcaccacggcctgagctataactgcagcctgccgctggcctttgatggttcttgtagcggtattcaacactttagcgccatgctgcgcgatgaggttggtggcagagcagtgaatctgctgccaagcgaaaccgtgcaagatatctatggcattgtggctaagaaggttaatgaaatcctgcaagcagacgcgattaacggcacggacaacgaggttgtcaccgtgaccgatgaaaacaccggtgagatctcggagaaagtgaaactgggcaccaaagccttggctggccaatggctggcatacggcgttactcgctccgtgaccaagcgttcggtgatgacccttgcttacggcagcaaagagtttggtttccgccaacaggttctggaggatactatccaaccggccatcgactctggtaaaggcctgatgttcacgcagccgaatcaggcagcgggctatatggcgaagctgatttgggaatcggttagcgttaccgttgttgcagcggtggaggctatgaactggctgaaatctgcggcgaagctgttagctgcggaggtgaaggacaagaagacgggcgaaatcctgcgtaagcgctgcgcagtgcattgggttacgccggatggttttccggtatggcaggagtacaaaaagcctattcagacccgtctgaacctgatgtttctgggtcaatttcgtctgcagccgacgatcaacaccaataaggactccgagatcgacgcgcacaaacaggagtctggcatcgcacccaatttcgttcactcacaggacggttcccatctgcgtaagaccgtcgtgtgggcacacgagaagtatggcattgagtcgtttgcattgatccacgattcctttggtaccatcccggcggacgctgcgaacctgtttaaagcggttcgcgaaaccatggttgacacctatgaaagttgcgatgttctggcagacttttatgatcagttcgccgaccaactgcatgagtcccagctggataaaatgccggcgttaccggcgaagggcaacttaaatctccgcgacatcctggaatctgatttcgccttcgcgtaa

SEQ ID NO: 80 - DNA, 2652 bp, synthetic construct
  source 1..2652: mol_type = other DNA
atgaatacaattaacatagctaaaaatgatttcagcgatattgaactggctgcgatcccgtttaataccttggcggaccattatggtgagcgtctggcgcgtgagcaacttgctctggagcacgaatcctacgagatgggtgaagcgcgtttccggaagatgttcgagcgccagcttaaggctggcgaggtggcggataacgctgctgcgaagccgttgattacgaccctgctgccgaaaatgattgcgcgtattaacgattggttcgaggaagtgaaagcaaagcgtggtaaacgtccaaccgcattccagtttctgcaagagatcaagccggaggcggtggcatacattacgatcaaaaccactctcgcatgtctcaccagcgcggataatactacggtccaagcggtggccagcgcgattggccgcgcgattgaggacgaagcgcgttttggtcgcattcgtgacctggaagcgaaacattttaagaagaacgttgaagaacaattgaataaacgcgtgggccacgtttacaagaaagcgttcatgcaagtcgttgatgctgatatgctgagcaaaggcctgttaggtggtgaagcatggagcagctggcataaggaggactcaattcacgtcggcgtgcggtgcattgaaatgctgatcgaatcgaccggtatggttagcctgcatcgccaaaacgccggcgtggtgggtcaagatagcgaaacgattgaactggcgccagagtacgcggaagctatcgctaccagagccggcgcattggcggggatcagcccgatgttccagccgtgtgttgtaccaccgaagccgtggaccggtatcaccggtggaggttactgggcgaatggtagacgtccgttggcgttggttcgtacccatagcaaaaaggctctgatgcgttatgaagacgtttacatgccggaagtgtacaaagccatcaacatcgcgcagaacactgcgtggaaaatcaacaaaaaggtgttagctgtggcgaacgtaattacaaaatggaagcactgcccggttgaggacatcccggctattgaacgtgaagagctgccaatgaaaccagaggacattgacatgaatccggaggcgctgaccgcatggaaacgtgcggcagcagcggtctatcgtaaggataaagccagaaagagccgtcgtatctccctggaattcatgcttgagcaggcgaacaaattcgctaaccacaaagccatctggtttccgtataatatggattggcgtggtcgtgtttacgcggtatcgatgttcaacccgcagggtaatgacatgaccaagggtttgttgaccttggccaaaggtaaaccgattggcaaagaaggttactattggttgaagatccacggtgcgaactgcgcaggggtggataaggtaccgttcccggaacgtattaaattcatcgaggaaaaccacgaaaacattatggcgtgcgcaaagagcccgctggaaaacacgtggtgggcagagcaggacagtccattctgcttcttggcgttctgtttcgaatatgcaggtgtccagcaccacggcctgagctataactgcagcctgccgctggcctttgatggttcttgtagcggtattcaacactttagcgccatgctgcgcgatgaggttggtggcagagcagtgaatctgctgccaagcgaaaccgtgcaagatatctatggcattgtggctaagaaggttaatgaaatcctgcaagcagacgcgattaacggcacggacaacgaggttgtcaccgtgaccgatgaaaacaccggtgagatctcggagaaagtgaaactgggcaccaaagccttggctggccaatggctggcatacggcgttactcgctccgtgaccaagcgttcggtgatgacccttgcttacggcagcaaagagtttggtttccgccaacaggttctggaggatactatccaaccggccatcgactctggtaaaggcctgatgttcacgcagccgaatcaggcagcgggctatatggcgaagctgatttgggaatcggttagcgttaccgttgttgcagcggtggaggctatgaactggctgaaatctgcggcgaagctgttagctgcggaggtgaaggacaagaagacgggcgaaatcctgcgtaagcgctgcgcagtgcattgggttacgccggatggttttccggtatggcaggagtacaaaaagcctattcagacccgtctgaacctgatgtttctgggtcaatttcgtctgcagccgacgatcaacaccaataaggactccgagatcgacgcgcacaaacaggagtctggcatcgcacccaatttcgttcactcacaggacggttcccatctgcgtaagaccgtcgtgtgggcacacgagaagtatggcattgagtcgtttgcattgatccacgattcctttggtaccatcccggcggacgctgcgaacctgtttaaagcggttcgcgaaaccatggttgacacctatgaaagttgcgatgttctggcagacttttatgatcagttcgccgaccaactgcatgagtcccagctggataaaatgccggcgttaccggcgaagggcaacttaaatctccgcgacatcctggaatctgatttcgccttcgcgtaa

SEQ ID NO: 81 - DNA, 2652 bp, synthetic construct
  source 1..2652: mol_type = other DNA
atgaatacaattaacatagctaaaaatgatttcagcgatattgaactggctgcgatcccgtttaataccttggcggaccattatggtgagcgtctggcgcgtgagcaacttgctctggagcacgaatcctacgagatgggtgaagcgcgtttccggaagatgttcgagcgccagcttaaggctggcgaggtggcggataacgctgctgcgaagccgttgattacgaccctgctgccgaaaatgattgcgcgtattaacgattggttcgaggaagtgaaagcaaagcgtggtaaacgtccaaccgcattccagtttctgcaagagatcaagccggaggcggtggcatacattacgatcaaaaccactctcgcatgtctcaccagcgcggataatactacggtccaagcggtggccagcgcgattggccgcgcgattgaggacgaagcgcgttttggtcgcattcgtgacctggaagcgaaacattttaagaagaacgttgaagaacaattgaataaacgcgtgggccacgtttacaagaaagcgttcatgcaagtcgttgaagctgatatgctgagcaaaggcctgttaggtggtgaagcatggagcagctggcataaggaggactcaattcacgtcggcgtgcggtgcattgaaatgctgatcgaatcgaccggtatggttagcctgcatcgccaaaacgccggcgtggtgggtcaagatagcgaaacgattgaactggcgccagagtacgcggaagctatcgctaccagagccggcgcattggcggggatcagcccgatgttccagccgtgtgttgtaccaccgaagccgtggaccggtatcaccggtggaggttactgggcgaatggtagacgtccgttggcgttggttcgtacccatagcaaaaaggctctgatgcgttatgaagacgtttacatgccggaagtgtacaaagccatcaacatcgcgcagaacactgcgtggaaaatcaacaaaaaggtgttagctgtggcgaacgtaattacaaaatggaagcactgcccggttgaggacatcccggctattgaacgtgaagagctgccaatgaaaccagaggacattgacatgaatccggaggcgctgaccgcatggaaacgtgcggcagcagcggtctatcgtaaggataaagccagaaagagccgtcgtatctccctggaattcatgcttgagcaggcgaacaaattcgctaaccacaaagccatctggtttccgtataatatggattggcgtggtcgtgtttacgcggtatcgatgttcaacccgcagggtaatgacatgaccaagggtttgttgacctttgccaaaggtaaaccgattggcaaagaaggttactattggttgaagatccacggtgcgaactgcgcaggggtggataaggtaccgttcccggaacgtattaaattcatcgaggaaaaccacgaaaacattatggcgtgcgcaaagagcccgctggaaaacacgtggtgggcagagcaggacagtccattctgcttcttggcgttctgtttcgaatatgcaggtgtccagcaccacggcctgagctataactgcagcctgccgctggcctttgatggttcttgtagcggtattcaacactttagcgccatgctgcgcgatgaggttggtggcagagcagtgaatctgctgccaagcgaaaccgtgcaagatatctatggcattgtggctaagaaggttaatgaaatcctgcaagcagacgcgattaacggcacggacaacgaggttgtcaccgtgaccgatgaaaacaccggtgagatctcggagaaagtgaaactgggcaccaaagccttggctggccaatggctggcatacggcgttactcgctccgtgaccaagcgttcggtgatgacccttgcttacggcagcaaagagtttggtttccgccaacaggttctggaggatactatccaaccggccatcgactctggtaaaggcctgatgttcacgcagccgaatcaggcagcgggctatatggcgaagctgatttgggaatcggttagcgttaccgttgttgcagcggtggaggctatgaactggctgaaatctgcggcgaagctgttagctgcggaggtgaaggacaagaagacgggcgaaatcctgcgtaagcgctgcgcagtgcattgggttacgccggatggttttccggtatggcaggagtacaaaaagcctattcagacccgtctgaacctgatgtttctgggtcaatttcgtctgcagccgacgatcaacaccaataaggactccgagatcgacgcgcacaaacaggagtctggcatcgcacccaatttcgttcactcacaggacggttcccatctgcgtaagaccgtcgtgtgggcacacgagaagtatggcattgagtcgtttgcattgatccacgattcctttggtaccatcccggcggacgctgcgaacctgtttaaagcggttcgcgaaaccatggttgacacctatgaaagttgcgatgttctggcagacttttatgatcagttcgccgaccaactgcatgagtcccagctggataaaatgccggcgttaccggcgaagggcaacttaaatctccgcgacatcctggaatctgatttcgccttcgcgtaa

SEQ ID NO: 82 - DNA, 2652 bp, synthetic construct
  source 1..2652: mol_type = other DNA
atgaatacaattaacatagctaaaaatgatttcagcgatattgaactggctgcgatcccgtttaataccttggcggaccattatggtgagcgtctggcgcgtgagcaacttgctctggagcacgaatcctacgagatgggtgaagcgcgtttccggaagatgttcgagcgccagcttaaggctggcgaggtggcggataacgctgctgcgaagccgttgattacgaccctgctgccgaaaatgattgcgcgtattaacgattggttcgaggaagtgaaagcaaagcgtggtaaacgtccaaccgcattccagtttctgcaagagatcaagccggaggcggtggcatacattacgatcaaaaccactctcgcatgtctcaccagcgcggataatactacggtccaagcggtggccagcgcgattggccgcgcgattgaggacgaagcgcgttttggtcgcattcgtgacctggaagcgaaacattttaagaagaacgttgaagaacaattgaataaacgcgtgggccacgtttacaagaaagcgttcatgcaagtcgttgaagctgatatgctgagcaaaggcctgttaggtggtgaagcatggagcagctggcataaggaggactcaattcacgtcggcgtgcggtgcattgaaatgctgatcgaatcgaccggtatggttagcctgcatcgccaaaacgccggcgtggtgggtcaagatagcgaaacgattgaactggcgccagagtacgcggaagctatcgctaccagagccggcgcattggcggggatcagcccgatgttccagccgtgtgttgtaccaccgaagccgtggaccggtatcaccggtggaggttactgggcgaatggtagacgtccgttggcgttggttcgtacccatagcaaaaaggctctgatgcgttatgaagacgtttacatgccggaagtgtacaaagccatcaacatcgcgcagaacactgcgtggaaaatcaacaaaaaggtgttagctgtggcgaacgtaattacaaaatggaagcactgcccggttgaggacatcccggctattgaacgtgaagagctgccaatgaaaccagaggacattgacatgaatccggaggcgctgaccgcatggaaacgtgcggcagcagcggtctatcgttctgataaagccagaaagagccgtcgtatctccctggaattcatgcttgagcaggcgaacaaattcgctaaccacaaagccatctggtttccgtataatatggattggcgtggtcgtgtttacgcggtatcgatgttcaacccgcagggtaatgacatgaccaagggtttgttgaccttggccaaaggtaaaccgattggcaaagaaggttactattggttgaagatccacggtgcgaactgcgcaggggtggataaggtaccgttcccggaacgtattaaattcatcgaggaaaaccacgaaaacattatggcgtgcgcaaagagcccgctggaaaacacgtggtgggcagagcaggacagtccattctgcttcttggcgttctgtttcgaatatgcaggtgtccagcaccacggcctgagctataactgcagcctgccgctggcctttgatggttcttgtagcggtattcaacactttagcgccatgctgcgcgatgaggttggtggcagagcagtgaatctgctgccaagcgaaaccgtgcaagatatctatggcattgtggctaagaaggttaatgaaatcctgcaagcagacgcgattaacggcacggacaacgaggttgtcaccgtgaccgatgaaaacaccggtgagatctcggagaaagtgaaactgggcaccaaagccttggctggccaatggctggcatacggcgttactcgctccgtgaccaagcgttcggtgatgacccttgcttacggcagcaaagagtttggtttccgccaacaggttctggaggatactatccaaccggccatcgactctggtaaaggcctgatgttcacgcagccgaatcaggcagcgggctatatggcgaagctgatttgggaatcggttagcgttaccgttgttgcagcggtggaggctatgaactggctgaaatctgcggcgaagctgttagctgcggaggtgaaggacaagaagacgggcgaaatcctgcgtaagcgctgcgcagtgcattgggttacgccggatggttttccggtatggcaggagtacaaaaagcctattcagacccgtctgaacctgatgtttctgggtcaatttcgtctgcagccgacgatcaacaccaataaggactccgagatcgacgcgcacaaacaggagtctggcatcgcacccaatttcgttcactcacaggacggttcccatctgcgtaagaccgtcgtgtgggcacacgagaagtatggcattgagtcgtttgcattgatccacgattcctttggtaccatcccggcggacgctgcgaacctgtttaaagcggttcgcgaaaccatggttgacacctatgaaagttgcgatgttctggcagacttttatgatcagttcgccgaccaactgcatgagtcccagctggataaaatgccggcgttaccggcgaagggcaacttaaatctccgcgacatcctggaatctgatttcgccttcgcgtaa

SEQ ID NO: 83 - DNA, 2652 bp, synthetic construct
  source 1..2652: mol_type = other DNA
atgaatacaattaacatagctaaaaatgatttcagcgatattgaactggctgcgatcccgtttaataccttggcggaccattatggtgagcgtctggcgcgtgagcaacttgctctggagcacgaatcctacgagatgggtgaagcgcgtttccggaagatgttcgagcgccagcttaaggctggcgaggtggcggataacgctgctgcgaagccgttgattacgaccctgctgccgaaaatgattgcgcgtattaacgattggttcgaggaagtgaaagcaaagcgtggtaaacgtccaaccgcattccagtttctgcaagagatcaagccggaggcggtggcatacattacgatcaaaaccactctcgcatgtctcaccagcgcggataatactacggtccaagcggtggccagcgcgattggccgcgcgattgaggacgaagcgcgttttggtcgcattcgtgacctggaagcgaaacattttaagaagaacgttgaagaacaattgaataaacgcgtgggccacgtttacaagaaagcgttcatgcaagtcgttgaagctgatatgctgagcaaaggcctgttaggtggtgaagcatggagcagctggcataaggaggactcaattcacgtcggcgtgcggtgcattgaaatgctgatcgaatcgaccggtatggttagcctgcatcgccaaaacgccggcgtggtgggtcaagatagcgaaacgattgaactggcgccagagtacgcggaagctatcgctaccagagccggcgcattggcggggatcagcccgatgttccagccgtgtgttgtaccaccgaagccgtggaccggtatcaccggtggaggttactgggcgaatggtagacgtccgttggcgttggttcgtacccatagcaaaaaggctctgatgcgttatgaagacgtttacatgccggaagtgtacaaagccatcaacatcgcgcagaacactgcgtggaaaatcaacaaaaaggtgttagctgtggcgaacgtaattacaaaatggaagcactgcccggttgaggacatcccggctattgaacgtgaagagctgccaatgaaaccagaggacattgacatgaatccggaggcgctgaccgcatggaaacgtgcggcagcagcggtctatcgtaaggatgcagccagaaagagccgtcgtatctccctggaattcatgcttgagcaggcgaacaaattcgctaaccacaaagccatctggtttccgtataatatggattggcgtggtcgtgtttacgcggtatcgatgttcaacccgcagggtaatgacatgaccaagggtttgttgaccttggccaaaggtaaaccgattggcaaagaaggttactattggttgaagatccacggtgcgaactgcgcaggggtggataaggtaccgttcccggaacgtattaaattcatcgaggaaaaccacgaaaacattatggcgtgcgcaaagagcccgctggaaaacacgtggtgggcagagcaggacagtccattctgcttcttggcgttctgtttcgaatatgcaggtgtccagcaccacggcctgagctataactgcagcctgccgctggcctttgatggttcttgtagcggtattcaacactttagcgccatgctgcgcgatgaggttggtggcagagcagtgaatctgctgccaagcgaaaccgtgcaagatatctatggcattgtggctaagaaggttaatgaaatcctgcaagcagacgcgattaacggcacggacaacgaggttgtcaccgtgaccgatgaaaacaccggtgagatctcggagaaagtgaaactgggcaccaaagccttggctggccaatggctggcatacggcgttactcgctccgtgaccaagcgttcggtgatgacccttgcttacggcagcaaagagtttggtttccgccaacaggttctggaggatactatccaaccggccatcgactctggtaaaggcctgatgttcacgcagccgaatcaggcagcgggctatatggcgaagctgatttgggaatcggttagcgttaccgttgttgcagcggtggaggctatgaactggctgaaatctgcggcgaagctgttagctgcggaggtgaaggacaagaagacgggcgaaatcctgcgtaagcgctgcgcagtgcattgggttacgccggatggttttccggtatggcaggagtacaaaaagcctattcagacccgtctgaacctgatgtttctgggtcaatttcgtctgcagccgacgatcaacaccaataaggactccgagatcgacgcgcacaaacaggagtctggcatcgcacccaatttcgttcactcacaggacggttcccatctgcgtaagaccgtcgtgtgggcacacgagaagtatggcattgagtcgtttgcattgatccacgattcctttggtaccatcccggcggacgctgcgaacctgtttaaagcggttcgcgaaaccatggttgacacctatgaaagttgcgatgttctggcagacttttatgatcagttcgccgaccaactgcatgagtcccagctggataaaatgccggcgttaccggcgaagggcaacttaaatctccgcgacatcctggaatctgatttcgccttcgcgtaa

SEQ ID NO: 84 - DNA, 2652 bp, synthetic construct
  source 1..2652: mol_type = other DNA
atgaatacaattaacatagctaaaaatgatttcagcgatattgaactggctgcgatcccgtttaataccttggcggaccattatggtgagcgtctggcgcgtgagcaacttgctctggagcacgaatcctacgagatgggtgaagcgcgtttccggaagatgttcgagcgccagcttaaggctggcgaggtggcggataacgctgctgcgaagccgttgattacgaccctgctgccgaaaatgattgcgcgtattaacgattggttcgaggaagtgaaagcaaagcgtggtaaacgtccaaccgcattccagtttctgcaagagatcaagccggaggcggtggcatacattacgatcaaaaccactctcgcatgtctcaccagcgcggataatactacggtccaagcggtggccagcgcgattggccgcgcgattgaggacgaagcgcgttttggtcgcattcgtgacctggaagcgaaacattttaagaagaacgttgaagaacaattgaataaacgcgtgggccacgtttacaagaaagcgttcatgcaagtcgttgaagctgatatgctgagcaaaggcctgttaggtggtgaagcatggagcagctggcataaggaggactcaattcacgtcggcgtgcggtgcattgaaatgctgatcgaatcgaccggtatggttagcctgcatcgccaaaacgccggcgtggtgggtcaagatagcgaaacgattgaactggcgccagagtacgcggaagctatcgctaccagagccggcgcattggcggggatcagcccgatgttccagccgtgtgttgtaccaccgaagccgtggaccggtatcaccggtggaggttactgggcgaatggtagacgtccgttggcgttggttcgtacccatagcaaaaaggctctgatgcgttatgaagacgtttacatgccggaagtgtacaaagccatcaacatcgcgcagaacactgcgtggaaaatcaacaaaaaggtgttagctgtggcgaacgtaattacaaaatggaagcactgcccggttgaggacatcccggctattgaacgtgaagagctgccaatgaaaccagaggacattgacatgaatccggaggcgctgaccgcatggaaacgtgcggcagcagcggtctatcgtaaggataaagccagaaagagccgtcgtatctccctggaattcatgcttgagcaggcgaacaaattcgctaaccacaaagccatctggtttccgtataatatggattggcgtggtcgtgtttacgcggtatcgatgttcaacccgcagggtaatgacatgaccaagggtttgttgaccttggccaaaggtaaaccgattggcaaagaaggttactattggttgaagatccacggtgcgaactgcgcaggggtggataaggtaccgttcccggaacgtattaaattcatcgaggaaaaccacgaaaacattatggcgtgcgcaaagagcccgctggaaaacacgtggtgggcagagcaggacagtccattctgcttcttggcgttctgtttcgaatatgcaggtgtccagcaccacggcctgagctataacagcagcctgccgctggcctttgatggttcttgtagcggtattcaacactttagcgccatgctgcgcgatgaggttggtggcagagcagtgaatctgctgccaagcgaaaccgtgcaagatatctatggcattgtggctaagaaggttaatgaaatcctgcaagcagacgcgattaacggcacggacaacgaggttgtcaccgtgaccgatgaaaacaccggtgagatctcggagaaagtgaaactgggcaccaaagccttggctggccaatggctggcatacggcgttactcgctccgtgaccaagcgttcggtgatgacccttgcttacggcagcaaagagtttggtttccgccaacaggttctggaggatactatccaaccggccatcgactctggtaaaggcctgatgttcacgcagccgaatcaggcagcgggctatatggcgaagctgatttgggaatcggttagcgttaccgttgttgcagcggtggaggctatgaactggctgaaatctgcggcgaagctgttagctgcggaggtgaaggacaagaagacgggcgaaatcctgcgtaagcgctgcgcagtgcattgggttacgccggatggttttccggtatggcaggagtacaaaaagcctattcagacccgtctgaacctgatgtttctgggtcaatttcgtctgcagccgacgatcaacaccaataaggactccgagatcgacgcgcacaaacaggagtctggcatcgcacccaatttcgttcactcacaggacggttcccatctgcgtaagaccgtcgtgtgggcacacgagaagtatggcattgagtcgtttgcattgatccacgattcctttggtaccatcccggcggacgctgcgaacctgtttaaagcggttcgcgaaaccatggttgacacctatgaaagttgcgatgttctggcagacttttatgatcagttcgccgaccaactgcatgagtcccagctggataaaatgccggcgttaccggcgaagggcaacttaaatctccgcgacatcctggaatctgatttcgccttcgcgtaa

SEQ ID NO: 85 - DNA, 2652 bp, synthetic construct
  source 1..2652: mol_type = other DNA
atgaatacaattaacatagctaaaaatgatttcagcgatattgaactggctgcgatcccgtttaataccttggcggaccattatggtgagcgtctggcgcgtgagcaacttgctctggagcacgaatcctacgagatgggtgaagcgcgtttccggaagatgttcgagcgccagcttaaggctggcgaggtggcggataacgctgctgcgaagccgttgattacgaccctgctgccgaaaatgattgcgcgtattaacgattggttcgaggaagtgaaagcaaagcgtggtaaacgtccaaccgcattccagtttctgcaagagatcaagccggaggcggtggcatacattacgatcaaaaccactctcgcatgtctcaccagcgcggataatactacggtccaagcggtggccagcgcgattggccgcgcgattgaggacgaagcgcgttttggtcgcattcgtgacctggaagcgaaacattttaagaagaacgttgaagaacaattgaataaacgcgtgggccacgtttacaagaaagcgttcatgcaagtcgttgaagctgatatgctgagcaaaggcctgttaggtggtgaagcatggagcagctggcataaggaggactcaattcacgtcggcgtgcggtgcattgaaatgctgatcgaatcgaccggtatggttagcctgcatcgccaaaacgccggcgtggtgggtcaagatagcgaaacgattgaactggcgccagagtacgcggaagctatcgctaccagagccggcgcattggcggggatcagcccgatgttccagccgtgtgttgtaccaccgaagccgtggaccggtatcaccggtggaggttactgggcgaatggtagacgtccgttggcgttggttcgtacccatagcaaaaaggctctgatgcgttatgaagacgtttacatgccggaagtgtacaaagccatcaacatcgcgcagaacactgcgtggaaaatcaacaaaaaggtgttagctgtggcgaacgtaattacaaaatggaagcactgcccggttgaggacatcccggctattgaacgtgaagagctgccaatgaaaccagaggacattgacatgaatccggaggcgctgaccgcatggaaacgtgcggcagcagcggtctatcgtaaggataaagccagaaagagccgtcgtatctccctggaattcatgcttgagcaggcgaacaaattcgctaaccacaaagccatctggtttccgtataatatggattggcgtggtcgtgtttacgcggtatcgatgttcaacccgcagggtaatgacatgaccaagggtttgttgaccttggccaaaggtaaaccgattggcaaagaaggttactattggttgaagatccacggtgcgaactgcgcaggggtggataaggtaccgttcccggaacgtattaaattcatcgaggaaaaccacgaaaacattatggcgtgcgcaaagagcccgctggaaaacacgtggtgggcagagcaggacagtccattctgcttcttggcgttctgtttcgaatatgcaggtgtccagcaccacggcctgagctataactgcagcctgccgctggcctttgatggttcttgtagcggtattcaacactttagcgccatgctgcgcgatgaggttggtggcagagcagtgaatctgctgccaagcgaaaccgtgcaagatatctatggcattgtggctaagaaggttaatgaaatcctgcaagcagacgcgattaacggcacggacaacgaggttgtcaccgtgaccgatgaaaacaccggtgagatctcggagaaagtgaaactgggcaccaaagccttggctggccaatggctggcatacggcgttactcgctccgtgaccaagcgttcggtgatgacccttgcttacggcagcaaagagtttggtttccgccaacaggttctggaggatactatccaaccggccatcgactctggtaaaggcctgatgttcacgcagccgaatcaggcagcgggctatatggcgaagctgatttgggaatcggttagcgttaccgttgttgcagcggtggaggctatgaactggctgaaatctgcggcgaagctgttagctgcggaggtgaaggacaagaagacgggcgaaatcctgcgtaagcgctgcgcagtgcattgggttacgccggatggttttccggtatggcaggagtacaaaaagcctattcagacccgtctgaacctgatgtttctgggtcaatttcgtctgcagccgacgatcaacaccaataaggactccgagatcgacgcgcacaaacaggagtctggcatcgcacccaatttcgttcactcacaggacggttcccatctgcgtaagaccgtcgtgtgggcacacgagaagtatggcattgagtcgtttgcattgatccacgattcctttggtaccatcccggcggacgctgcgaacctgtttaaagcggttcgcgaaaccatggttgacacctatgaaagttgcgatgttctggcagacttttatgatcagttcgccgaccaactgcatgagtcccagctggataaaatgccggcgttaccggcgaagggcaacttagatctccgcgacatcctggaatctgatttcgccttcgcgtaa

SEQ ID NO: 86 - DNA, 2646 bp, synthetic construct
  source 1..2646: mol_type = other DNA
atgaatacaattaacatagctaaaaatgatttcagcgatattgaactggctgcgatcccgtttaataccttggcggaccattatggtgagcgtctggcgcgtgagcaacttgctctggagcacgaatcctacgagatgggtgaagcgcgtttccggaagatgttcgagcgccagcttaaggctggcgaggtggcggataacgctgctgcgaagccgttgattacgaccctgctgccgaaaatgattgcgcgtattaacgattggttcgaggaagtgaaagcaaagcgtggtaaacgtccaaccgcattccagtttctgcaagagatcaagccggaggcggtggcatacattacgatcaaaaccactctcgcatgtctcaccagcgcggataatactacggtccaagcggtggccagcgcgattggccgcgcgattgaggacgaagcgcgttttggtcgcattcgtgacctggaagcgaaacattttaagaagaacgttgaagaacaattgaatgtgggccacgtttacaagaaagcgttcatgcaagtcgttgaagctgatatgctgagcaaaggcctgttaggtggtgaagcatggagcagctggcataaggaggactcaattcacgtcggcgtgcggtgcattgaaatgctgatcgaatcgaccggtatggttagcctgcatcgccaaaacgccggcgtggtgggtcaagatagcgaaacgattgaactggcgccagagtacgcggaagctatcgctaccagagccggcgcattggcggggatcagcccgatgttccagccgtgtgttgtaccaccgaagccgtggaccggtatcaccggtggaggttactgggcgaatggtagacgtccgttggcgttggttcgtacccatagcaaaaaggctctgatgcgttatgaagacgtttacatgccggaagtgtacaaagccatcaacatcgcgcagaacactgcgtggaaaatcaacaaaaaggtgttagctgtggcgaacgtaattacaaaatggaagcactgcccggttgaggacatcccggctattgaacgtgaagagctgccaatgaaaccagaggacattgacatgaatccggaggcgctgaccgcatggaaacgtgcggcagcagcggtctatcgtaaggataaagccagaaagagccgtcgtatctccctggaattcatgcttgagcaggcgaacaaattcgctaaccacaaagccatctggtttccgtataatatggattggcgtggtcgtgtttacgcggtatcgatgttcaacccgcagggtaatgacatgaccaagggtttgttgaccttggccaaaggtaaaccgattggcaaagaaggttactattggttgaagatccacggtgcgaactgcgcaggggtggataaggtaccgttcccggaacgtattaaattcatcgaggaaaaccacgaaaacattatggcgtgcgcaaagagcccgctggaaaacacgtggtgggcagagcaggacagtccattctgcttcttggcgttctgtttcgaatatgcaggtgtccagcaccacggcctgagctataactgcagcctgccgctggcctttgatggttcttgtagcggtattcaacactttagcgccatgctgcgcgatgaggttggtggcagagcagtgaatctgctgccaagcgaaaccgtgcaagatatctatggcattgtggctaagaaggttaatgaaatcctgcaagcagacgcgattaacggcacggacaacgaggttgtcaccgtgaccgatgaaaacaccggtgagatctcggagaaagtgaaactgggcaccaaagccttggctggccaatggctggcatacggcgttactcgctccgtgaccaagcgttcggtgatgacccttgcttacggcagcaaagagtttggtttccgccaacaggttctggaggatactatccaaccggccatcgactctggtaaaggcctgatgttcacgcagccgaatcaggcagcgggctatatggcgaagctgatttgggaatcggttagcgttaccgttgttgcagcggtggaggctatgaactggctgaaatctgcggcgaagctgttagctgcggaggtgaaggacaagaagacgggcgaaatcctgcgtaagcgctgcgcagtgcattgggttacgccggatggttttccggtatggcaggagtacaaaaagcctattcagacccgtctgaacctgatgtttctgggtcaatttcgtctgcagccgacgatcaacaccaataaggactccgagatcgacgcgcacaaacaggagtctggcatcgcacccaatttcgttcactcacaggacggttcccatctgcgtaagaccgtcgtgtgggcacacgagaagtatggcattgagtcgtttgcattgatccacgattcctttggtaccatcccggcggacgctgcgaacctgtttaaagcggttcgcgaaaccatggttgacacctatgaaagttgcgatgttctggcagacttttatgatcagttcgccgaccaactgcatgagtcccagctggataaaatgccggcgttaccggcgaagggcaacttaaatctccgcgacatcctggaatctgatttcgccttcgcgtaa

SEQ ID NO: 87 - DNA, 2652 bp, synthetic construct
  source 1..2652: mol_type = other DNA
atgaatacaattaacatagctaaaaatgatttcagcgatattgaactggctgcgatcccgtttaataccttggcggaccattatggtgagcgtctggcgcgtgagcaacttgctctggagcacgaatcctacgagatgggtgaagcgcgtttccggaagatgttcgagcgccagcttaaggctggcgaggtggcggataacgctgctgcgaagccgttgattacgaccctgctgccgaaaatgattgcgcgtattaacgattggttcgaggaagtgaaagcaaagcgtggtaaacgtccaaccgcattccagtttctgcaagagatcaagccggaggcggtggcatacattacgatcaaaaccactctcgcatgtctcaccagcgcggataatactacggtccaagcggtggccagcgcgattggccgcgcgattgaggacgaagcgcgttttggtcgcattcgtgacctggaagcgaaacattttaagaagaacgttgaagaacaattgaatgctggagtgggccacgtttacaagaaagcgttcatgcaagtcgttgaagctgatatgctgagcaaaggcctgttaggtggtgaagcatggagcagctggcataaggaggactcaattcacgtcggcgtgcggtgcattgaaatgctgatcgaatcgaccggtatggttagcctgcatcgccaaaacgccggcgtggtgggtcaagatagcgaaacgattgaactggcgccagagtacgcggaagctatcgctaccagagccggcgcattggcggggatcagcccgatgttccagccgtgtgttgtaccaccgaagccgtggaccggtatcaccggtggaggttactgggcgaatggtagacgtccgttggcgttggttcgtacccatagcaaaaaggctctgatgcgttatgaagacgtttacatgccggaagtgtacaaagccatcaacatcgcgcagaacactgcgtggaaaatcaacaaaaaggtgttagctgtggcgaacgtaattacaaaatggaagcactgcccggttgaggacatcccggctattgaacgtgaagagctgccaatgaaaccagaggacattgacatgaatccggaggcgctgaccgcatggaaacgtgcggcagcagcggtctatcgtaaggataaagccagaaagagccgtcgtatctccctggaattcatgcttgagcaggcgaacaaattcgctaaccacaaagccatctggtttccgtataatatggattggcgtggtcgtgtttacgcggtatcgatgttcaacccgcagggtaatgacatgaccaagggtttgttgaccttggccaaaggtaaaccgattggcaaagaaggttactattggttgaagatccacggtgcgaactgcgcaggggtggataaggtaccgttcccggaacgtattaaattcatcgaggaaaaccacgaaaacattatggcgtgcgcaaagagcccgctggaaaacacgtggtgggcagagcaggacagtccattctgcttcttggcgttctgtttcgaatatgcaggtgtccagcaccacggcctgagctataactgcagcctgccgctggcctttgatggttcttgtagcggtattcaacactttagcgccatgctgcgcgatgaggttggtggcagagcagtgaatctgctgccaagcgaaaccgtgcaagatatctatggcattgtggctaagaaggttaatgaaatcctgcaagcagacgcgattaacggcacggacaacgaggttgtcaccgtgaccgatgaaaacaccggtgagatctcggagaaagtgaaactgggcaccaaagccttggctggccaatggctggcatacggcgttactcgctccgtgaccaagcgttcggtgatgacccttgcttacggcagcaaagagtttggtttccgccaacaggttctggaggatactatccaaccggccatcgactctggtaaaggcctgatgttcacgcagccgaatcaggcagcgggctatatggcgaagctgatttgggaatcggttagcgttaccgttgttgcagcggtggaggctatgaactggctgaaatctgcggcgaagctgttagctgcggaggtgaaggacaagaagacgggcgaaatcctgcgtaagcgctgcgcagtgcattgggttacgccggatggttttccggtatggcaggagtacaaaaagcctattcagacccgtctgaacctgatgtttctgggtcaatttcgtctgcagccgacgatcaacaccaataaggactccgagatcgacgcgcacaaacaggagtctggcatcgcacccaatttcgttcactcacaggacggttcccatctgcgtaagaccgtcgtgtgggcacacgagaagtatggcattgagtcgtttgcattgatccacgattcctttggtaccatcccggcggacgctgcgaacctgtttaaagcggttcgcgaaaccatggttgacacctatgaaagttgcgatgttctggcagacttttatgatcagttcgccgaccaactgcatgagtcccagctggataaaatgccggcgttaccggcgaagggcaacttaaatctccgcgacatcctggaatctgatttcgccttcgcgtaa

SEQ ID NO: 88 - DNA, 2652 bp, synthetic construct
  source 1..2652: mol_type = other DNA
atgaatacaattaacatagctaaaaatgatttcagcgatattgaactggctgcgatcccgtttaataccttggcggaccattatggtgagcgtctggcgcgtgagcaacttgctctggagcacgaatcctacgagatgggtgaagcgcgtttccggaagatgttcgagcgccagcttaaggctggcgaggtggcggataacgctgctgcgaagccgttgattacgaccctgctgccgaaaatgattgcgcgtattaacgattggttcgaggaagtgaaagcaaagcgtggtaaacgtccaaccgcattccagtttctgcaagagatcaagccggaggcggtggcatacattacgatcaaaaccactctcgcatgtctcaccagcgcggataatactacggtccaagcggtggccagcgcgattggccgcgcgattgaggacgaagcgcgttttggtcgcattcgtgacctggaagcgaaacattttaagaagaacgttgaagaacaattgaatgctggagtgggccacgtttacaagaaagcgttcatgcaagtcgttgaagctgatatgctgagcaaaggcctgttaggtggtgaagcatggagcagctggcataaggaggactcaattcacgtcggcgtgcggtgcattgaaatgctgatcgaatcgaccggtatggttagcctgcatcgccaaaacgccggcgtggtgggtcaagatagcgaaacgattgaactggcgccagagtacgcggaagctatcgctaccagagccggcgcattggcggggatcagcccgatgttccagccgtgtgttgtaccaccgaagccgtggaccggtatcaccggtggaggttactgggcgaatggtagacgtccgttggcgttggttcgtacccatagcaaaaaggctctgatgcgttatgaagacgtttacatgccggaagtgtacaaagccatcaacatcgcgcagaacactgcgtggaaaatcaacaaaaaggtgttagctgtggcgaacgtaattacaaaatggaagcactgcccggttgaggacatcccggctattgaacgtgaagagctgccaatgaaaccagaggacattgacatgaatccggaggcgctgaccgcatggaaacgtgcggcagcagcggtctatcgttacgataaagccagaaagagccgtcgtatctccctggaattcatgcttgagcaggcgaacaaattcgctaaccacaaagccatctggtttccgtataatatggattggcgtggtcgtgtttacgcggtatcgatgttcaacccgcagggtaatgacatgaccaagggtttgttgaccttggccaaaggtaaaccgattggcaaagaaggttactattggttgaagatccacggtgcgaactgcgcaggggtggataaggtaccgttcccggaacgtattaaattcatcgaggaaaaccacgaaaacattatggcgtgcgcaaagagcccgctggaaaacacgtggtgggcagagcaggacagtccattctgcttcttggcgttctgtttcgaatatgcaggtgtccagcaccacggcctgagctataactgcagcctgccgctggcctttgatggttcttgtagcggtattcaacactttagcgccatgctgcgcgatgaggttggtggcagagcagtgaatctgctgccaagcgaaaccgtgcaagatatctatggcattgtggctaagaaggttaatgaaatcctgcaagcagacgcgattaacggcacggacaacgaggttgtcaccgtgaccgatgaaaacaccggtgagatctcggagaaagtgaaactgggcaccaaagccttggctggccaatggctggcatacggcgttactcgctccgtgaccaagcgttcggtgatgacccttgcttacggcagcaaagagtttggtttccgccaacaggttctggaggatactatccaaccggccatcgactctggtaaaggcctgatgttcacgcagccgaatcaggcagcgggctatatggcgaagctgatttgggaatcggttagcgttaccgttgttgcagcggtggaggctatgaactggctgaaatctgcggcgaagctgttagctgcggaggtgaaggacaagaagacgggcgaaatcctgcgtaagcgctgcgcagtgcattgggttacgccggatggttttccggtatggcaggagtacaaaaagcctattcagacccgtctgaacctgatgtttctgggtcaatttcgtctgcagccgacgatcaacaccaataaggactccgagatcgacgcgcacaaacaggagtctggcatcgcacccaatttcgttcactcacaggacggttcccatctgcgtaagaccgtcgtgtgggcacacgagaagtatggcattgagtcgtttgcattgatccacgattcctttggtaccatcccggcggacgctgcgaacctgtttaaagcggttcgcgaaaccatggttgacacctatgaaagttgcgatgttctggcagacttttatgatcagttcgccgaccaactgcatgagtcccagctggataaaatgccggcgttaccggcgaagggcaacttaaatctccgcgacatcctggaatctgatttcgccttcgcgtaa

SEQ ID NO: 89 - DNA, 2652 bp, synthetic construct
  source 1..2652: mol_type = other DNA
atgaatacaattaacatagctaaaaatgatttcagcgatattgaactggctgcgatcccgtttaataccttggcggaccattatggtgagcgtctggcgcgtgagcaacttgctctggagcacgaatcctacgagatgggtgaagcgcgtttccggaagatgttcgagcgccagcttaaggctggcgaggtggcggataacgctgctgcgaagccgttgattacgaccctgctgccgaaaatgattgcgcgtattaacgattggttcgaggaagtgaaagcaaagcgtggtaaacgtccaaccgcattccagtttctgcaagagatcaagccggaggcggtggcatacattacgatcaaaaccactctcgcatgtctcaccagcgcggataatactacggtccaagcggtggccagcgcgattggccgcgcgattgaggacgaagcgcgttttggtcgcattcgtgacctggaagcgaaacattttaagaagaacgttgaagaacaattgaatgctggagtgggccacgtttacaagaaagcgttcatgcaagtcgttgaagctgatatgctgagcaaaggcctgttaggtggtgaagcatggagcagctggcataaggaggactcaattcacgtcggcgtgcggtgcattgaaatgctgatcgaatcgaccggtatggttagcctgcatcgccaaaacgccggcgtggtgggtcaagatagcgaaacgattgaactggcgccagagtacgcggaagctatcgctaccagagccggcgcattggcggggatcagcccgatgttccagccgtgtgttgtaccaccgaagccgtggaccggtatcaccggtggaggttactgggcgaatggtagacgtccgttggcgttggttcgtacccatagcaaaaaggctctgatgcgttatgaagacgtttacatgccggaagtgtacaaagccatcaacatcgcgcagaacactgcgtggaaaatcaacaaaaaggtgttagctgtggcgaacgtaattacaaaatggaagcactgcccggttgaggacatcccggctattgaacgtgaagagctgccaatgaaaccagaggacattgacatgaatccggaggcgctgaccgcatggaaacgtgcggcagcagcggtctatcgttctgataaagccagaaagagccgtcgtatctccctggaattcatgcttgagcaggcgaacaaattcgctaaccacaaagccatctggtttccgtataatatggattggcgtggtcgtgtttacgcggtatcgatgttcaacccgcagggtaatgacatgaccaagggtttgttgaccttggccaaaggtaaaccgattggcaaagaaggttactattggttgaagatccacggtgcgaactgcgcaggggtggataaggtaccgttcccggaacgtattaaattcatcgaggaaaaccacgaaaacattatggcgtgcgcaaagagcccgctggaaaacacgtggtgggcagagcaggacagtccattctgcttcttggcgttctgtttcgaatatgcaggtgtccagcaccacggcctgagctataactgcagcctgccgctggcctttgatggttcttgtagcggtattcaacactttagcgccatgctgcgcgatgaggttggtggcagagcagtgaatctgctgccaagcgaaaccgtgcaagatatctatggcattgtggctaagaaggttaatgaaatcctgcaagcagacgcgattaacggcacggacaacgaggttgtcaccgtgaccgatgaaaacaccggtgagatctcggagaaagtgaaactgggcaccaaagccttggctggccaatggctggcatacggcgttactcgctccgtgaccaagcgttcggtgatgacccttgcttacggcagcaaagagtttggtttccgccaacaggttctggaggatactatccaaccggccatcgactctggtaaaggcctgatgttcacgcagccgaatcaggcagcgggctatatggcgaagctgatttgggaatcggttagcgttaccgttgttgcagcggtggaggctatgaactggctgaaatctgcggcgaagctgttagctgcggaggtgaaggacaagaagacgggcgaaatcctgcgtaagcgctgcgcagtgcattgggttacgccggatggttttccggtatggcaggagtacaaaaagcctattcagacccgtctgaacctgatgtttctgggtcaatttcgtctgcagccgacgatcaacaccaataaggactccgagatcgacgcgcacaaacaggagtctggcatcgcacccaatttcgttcactcacaggacggttcccatctgcgtaagaccgtcgtgtgggcacacgagaagtatggcattgagtcgtttgcattgatccacgattcctttggtaccatcccggcggacgctgcgaacctgtttaaagcggttcgcgaaaccatggttgacacctatgaaagttgcgatgttctggcagacttttatgatcagttcgccgaccaactgcatgagtcccagctggataaaatgccggcgttaccggcgaagggcaacttaaatctccgcgacatcctggaatctgatttcgccttcgcgtaa

SEQ ID NO: 90 - DNA, 2649 bp, synthetic construct
  source 1..2649: mol_type = other DNA
atgaatacaattaacatagctaaaaatgatttcagcgatattgaactggctgcgatcccgtttaataccttggcggaccattatggtgagcgtctggcgcgtgagcaacttgctctggagcacgaatcctacgagatgggtgaagcgcgtttccggaagatgttcgagcgccagcttaaggctggcgaggtggcggataacgctgctgcgaagccgttgattacgaccctgctgccgaaaatgattgcgcgtattaacgattggttcgaggaagtgaaagcaaagcgtggtaaacgtccaaccgcattccagtttctgcaagagatcaagccggaggcggtggcatacattacgatcaaaaccactctcgcatgtctcaccagcgcggataatactacggtccaagcggtggccagcgcgattggccgcgcgattgaggacgaagcgcgttttggtcgcattcgtgacctggaagcgaaacattttaagaagaacgttgatgaacaattgaatcgcgtgggccacgtttacaagaaagcgttcatgcaagtcgttgaagctgatatgctgagcaaaggcctgttaggtggtgaagcatggagcagctggcataaggaggactcaattcacgtcggcgtgcggtgcattgaaatgctgatcgaatcgaccggtatggttagcctgcatcgccaaaacgccggcgtggtgggtcaagatagcgaaacgattgaactggcgccagagtacgcggaagctatcgctaccagagccggcgcattggcggggatcagcccgatgttccagccgtgtgttgtaccaccgaagccgtggaccggtatcaccggtggaggttactgggcgaatggtagacgtccgttggcgttggttcgtacccatagcaaaaaggctctgatgcgttatgaagacgtttacatgccggaagtgtacaaagccatcaacatcgcgcagaacactgcgtggaaaatcaacaaaaaggtgttagctgtggcgaacgtaattacaaaatggaagcactgcccggttgaggacatcccggctattgaacgtgaagagctgccaatgaaaccagaggacattgacatgaatccggaggcgctgaccgcatggaaacgtgcggcagcagcggtctatcgtaaggataaagccagaaagagccgtcgtatctccctggaattcatgcttgagcaggcgaacaaattcgctaaccacaaagccatctggtttccgtataatatggattggcgtggtcgtgtttacgcggtatcgatgttcaacccgcagggtaatgacatgaccaagggtttgttgaccttggccaaaggtaaaccgattggcaaagaaggttactattggttgaagatccacggtgcgaactgcgcaggggtggataaggtaccgttcccggaacgtattaaattcatcgaggaaaaccacgaaaacattatggcgtgcgcaaagagcccgctggaaaacacgtggtgggcagagcaggacagtccattctgcttcttggcgttctgtttcgaatatgcaggtgtccagcaccacggcctgagctataactgcagcctgccgctggcctttgatggttcttgtagcggtattcaacactttagcgccatgctgcgcgatgaggttggtggcagagcagtgaatctgctgccaagcgaaaccgtgcaagatatctatggcattgtggctaagaaggttaatgaaatcctgcaagcagacgcgattaacggcacggacaacgaggttgtcaccgtgaccgatgaaaacaccggtgagatctcggagaaagtgaaactgggcaccaaagccttggctggccaatggctggcatacggcgttactcgctccgtgaccaagcgttcggtgatgacccttgcttacggcagcaaagagtttggtttccgccaacaggttctggaggatactatccaaccggccatcgactctggtaaaggcctgatgttcacgcagccgaatcaggcagcgggctatatggcgaagctgatttgggaatcggttagcgttaccgttgttgcagcggtggaggctatgaactggctgaaatctgcggcgaagctgttagctgcggaggtgaaggacaagaagacgggcgaaatcctgcgtaagcgctgcgcagtgcattgggttacgccggatggttttccggtatggcaggagtacaaaaagcctattcagacccgtctgaacctgatgtttctgggtcaatttcgtctgcagccgacgatcaacaccaataaggactccgagatcgacgcgcacaaacaggagtctggcatcgcacccaatttcgttcactcacaggacggttcccatctgcgtaagaccgtcgtgtgggcacacgagaagtatggcattgagtcgtttgcattgatccacgattcctttggtaccatcccggcggacgctgcgaacctgtttaaagcggttcgcgaaaccatggttgacacctatgaaagttgcgatgttctggcagacttttatgatcagttcgccgaccaactgcatgagtcccagctggataaaatgccggcgttaccggcgaagggcaacttaaatctccgcgacatcctggaatctgatttcgccttcgcgtaa

SEQ ID NO: 91 - DNA, 2646 bp, synthetic construct
  source 1..2646: mol_type = other DNA
atgaatacaattaacatagctaaaaatgatttcagcgatattgaactggctgcgatcccgtttaataccttggcggaccattatggtgagcgtctggcgcgtgagcaacttgctctggagcacgaatcctacgagatgggtgaagcgcgtttccggaagatgttcgagcgccagcttaaggctggcgaggtggcggataacgctgctgcgaagccgttgattacgaccctgctgccgaaaatgattgcgcgtattaacgattggttcgaggaagtgaaagcaaagcgtggtaaacgtccaaccgcattccagtttctgcaagagatcaagccggaggcggtggcatacattacgatcaaaaccactctcgcatgtctcaccagcgcggataatactacggtccaagcggtggccagcgcgattggccgcgcgattgaggacgaagcgcgttttggtcgcattcgtgacctggaagcgaaacattttaagaagaacgttgaagatcaattgaatgtgggccacgtttacaagaaagcgttcatgcaagtcgttgaagctgatatgctgagcaaaggcctgttaggtggtgaagcatggagcagctggcataaggaggactcaattcacgtcggcgtgcggtgcattgaaatgctgatcgaatcgaccggtatggttagcctgcatcgccaaaacgccggcgtggtgggtcaagatagcgaaacgattgaactggcgccagagtacgcggaagctatcgctaccagagccggcgcattggcggggatcagcccgatgttccagccgtgtgttgtaccaccgaagccgtggaccggtatcaccggtggaggttactgggcgaatggtagacgtccgttggcgttggttcgtacccatagcaaaaaggctctgatgcgttatgaagacgtttacatgccggaagtgtacaaagccatcaacatcgcgcagaacactgcgtggaaaatcaacaaaaaggtgttagctgtggcgaacgtaattacaaaatggaagcactgcccggttgaggacatcccggctattgaacgtgaagagctgccaatgaaaccagaggacattgacatgaatccggaggcgctgaccgcatggaaacgtgcggcagcagcggtctatcgtaaggataaagccagaaagagccgtcgtatctccctggaattcatgcttgagcaggcgaacaaattcgctaaccacaaagccatctggtttccgtataatatggattggcgtggtcgtgtttacgcggtatcgatgttcaacccgcagggtaatgacatgaccaagggtttgttgaccttggccaaaggtaaaccgattggcaaagaaggttactattggttgaagatccacggtgcgaactgcgcaggggtggataaggtaccgttcccggaacgtattaaattcatcgaggaaaaccacgaaaacattatggcgtgcgcaaagagcccgctggaaaacacgtggtgggcagagcaggacagtccattctgcttcttggcgttctgtttcgaatatgcaggtgtccagcaccacggcctgagctataactgcagcctgccgctggcctttgatggttcttgtagcggtattcaacactttagcgccatgctgcgcgatgaggttggtggcagagcagtgaatctgctgccaagcgaaaccgtgcaagatatctatggcattgtggctaagaaggttaatgaaatcctgcaagcagacgcgattaacggcacggacaacgaggttgtcaccgtgaccgatgaaaacaccggtgagatctcggagaaagtgaaactgggcaccaaagccttggctggccaatggctggcatacggcgttactcgctccgtgaccaagcgttcggtgatgacccttgcttacggcagcaaagagtttggtttccgccaacaggttctggaggatactatccaaccggccatcgactctggtaaaggcctgatgttcacgcagccgaatcaggcagcgggctatatggcgaagctgatttgggaatcggttagcgttaccgttgttgcagcggtggaggctatgaactggctgaaatctgcggcgaagctgttagctgcggaggtgaaggacaagaagacgggcgaaatcctgcgtaagcgctgcgcagtgcattgggttacgccggatggttttccggtatggcaggagtacaaaaagcctattcagacccgtctgaacctgatgtttctgggtcaatttcgtctgcagccgacgatcaacaccaataaggactccgagatcgacgcgcacaaacaggagtctggcatcgcacccaatttcgttcactcacaggacggttcccatctgcgtaagaccgtcgtgtgggcacacgagaagtatggcattgagtcgtttgcattgatccacgattcctttggtaccatcccggcggacgctgcgaacctgtttaaagcggttcgcgaaaccatggttgacacctatgaaagttgcgatgttctggcagacttttatgatcagttcgccgaccaactgcatgagtcccagctggataaaatgccggcgttaccggcgaagggcaacttaaatctccgcgacatcctggaatctgatttcgccttcgcgtaa

SEQ ID NO: 92 - DNA, 2646 bp, synthetic construct
  source 1..2646: mol_type = other DNA
atgaatacaattaacatagctaaaaatgatttcagcgatattgaactggctgcgatcccgtttaataccttggcggaccattatggtgagcgtctggcgcgtgagcaacttgctctggagcacgaatcctacgagatgggtgaagcgcgtttccggaagatgttcgagcgccagcttaaggctggcgaggtggcggataacgctgctgcgaagccgttgattacgaccctgctgccgaaaatgattgcgcgtattaacgattggttcgaggaagtgaaagcaaagcgtggtaaacgtccaaccgcattccagtttctgcaagagatcaagccggaggcggtggcatacattacgatcaaaaccactctcgcatgtctcaccagcgcggataatactacggtccaagcggtggccagcgcgattggccgcgcgattgaggacgaagcgcgttttggtcgcattcgtgacctggaagcgaaacattttaagaagaacgttgaagaacaattgaatgtgggccacgtttacaagaaagcgttcatgcaagtcgttgaagctgatatgctgagcaaaggcctgttaggtggtgaagcatggagcagctggcataaggaggactcaattcacgtcggcgtgcggtgcattgaaatgctgatcgaatcgaccggtatggttagcctgcatcgccaaaacgccggcgtggtgggtcaagatagcgaaacgattgaactggcgccagagtacgcggaagctatcgctaccagagccggcgcattggcggggatcagcccgatgttccagccgtgtgttgtaccaccgaagccgtggaccggtatcaccggtggaggttactgggcgaatggtagacgtccgttggcgttggttcgtacccatagcaaaaaggctctgatgcgttatgaagacgtttacatgccggaagtgtacaaagccatcaacatcgcgcagaacactgcgtggaaaatcaacaaaaaggtgttagctgtggcgaacgtaattacaaaatggaagcactgcccggttgaggacatcccggctattgaacgtgaagagctgccaatgaaaccagaggacattgacatgaatccggaggcgctgaccgcatggaaacgtgcggcagcagcggtctatcgtagtgataaagccagaaagagccgtcgtatctccctggaattcatgcttgagcaggcgaacaaattcgctaaccacaaagccatctggtttccgtataatatggattggcgtggtcgtgtttacgcggtatcgatgttcaacccgcagggtaatgacatgaccaagggtttgttgaccttggccaaaggtaaaccgattggcaaagaaggttactattggttgaagatccacggtgcgaactgcgcaggggtggataaggtaccgttcccggaacgtattaaattcatcgaggaaaaccacgaaaacattatggcgtgcgcaaagagcccgctggaaaacacgtggtgggcagagcaggacagtccattctgcttcttggcgttctgtttcgaatatgcaggtgtccagcaccacggcctgagctataactgcagcctgccgctggcctttgatggttcttgtagcggtattcaacactttagcgccatgctgcgcgatgaggttggtggcagagcagtgaatctgctgccaagcgaaaccgtgcaagatatctatggcattgtggctaagaaggttaatgaaatcctgcaagcagacgcgattaacggcacggacaacgaggttgtcaccgtgaccgatgaaaacaccggtgagatctcggagaaagtgaaactgggcaccaaagccttggctggccaatggctggcatacggcgttactcgctccgtgaccaagcgttcggtgatgacccttgcttacggcagcaaagagtttggtttccgccaacaggttctggaggatactatccaaccggccatcgactctggtaaaggcctgatgttcacgcagccgaatcaggcagcgggctatatggcgaagctgatttgggaatcggttagcgttaccgttgttgcagcggtggaggctatgaactggctgaaatctgcggcgaagctgttagctgcggaggtgaaggacaagaagacgggcgaaatcctgcgtaagcgctgcgcagtgcattgggttacgccggatggttttccggtatggcaggagtacaaaaagcctattcagacccgtctgaacctgatgtttctgggtcaatttcgtctgcagccgacgatcaacaccaataaggactccgagatcgacgcgcacaaacaggagtctggcatcgcacccaatttcgttcactcacaggacggttcccatctgcgtaagaccgtcgtgtgggcacacgagaagtatggcattgagtcgtttgcattgatccacgattcctttggtaccatcccggcggacgctgcgaacctgtttaaagcggttcgcgaaaccatggttgacacctatgaaagttgcgatgttctggcagacttttatgatcagttcgccgaccaactgcatgagtcccagctggataaaatgccggcgttaccggcgaagggcaacttaaatctccgcgacatcctggaatctgatttcgccttcgcgtaa

SEQ ID NO: 93 - DNA, 2646 bp, synthetic construct
  source 1..2646: mol_type = other DNA
atgaatacaattaacatagctaaaaatgatttcagcgatattgaactggctgcgatcccgtttaataccttggcggaccattatggtgagcgtctggcgcgtgagcaacttgctctggagcacgaatcctacgagatgggtgaagcgcgtttccggaagatgttcgagcgccagcttaaggctggcgaggtggcggataacgctgctgcgaagccgttgattacgaccctgctgccgaaaatgattgcgcgtattaacgattggttcgaggaagtgaaagcaaagcgtggtaaacgtccaaccgcattccagtttctgcaagagatcaagccggaggcggtggcatacattacgatcaaaaccactctcgcatgtctcaccagcgcggataatactacggtccaagcggtggccagcgcgattggccgcgcgattgaggacgaagcgcgttttggtcgcattcgtgacctggaagcgaaacattttaagaagaacgttgaagaacaattgaatgtgggccacgttggcaagaaagcgttcatgcaagtcgttgaagctgatatgctgagcaaaggcctgttaggtggtgaagcatggagcagctggcataaggaggactcaattcacgtcggcgtgcggtgcattgaaatgctgatcgaatcgaccggtatggttagcctgcatcgccaaaacgccggcgtggtgggtcaagatagcgaaacgattgaactggcgccagagtacgcggaagctatcgctaccagagccggcgcattggcggggatcagcccgatgttccagccgtgtgttgtaccaccgaagccgtggaccggtatcaccggtggaggttactgggcgaatggtagacgtccgttggcgttggttcgtacccatagcaaaaaggctctgatgcgttatgaagacgtttacatgccggaagtgtacaaagccatcaacatcgcgcagaacactgcgtggaaaatcaacaaaaaggtgttagctgtggcgaacgtaattacaaaatggaagcactgcccggttgaggacatcccggctattgaacgtgaagagctgccaatgaaaccagaggacattgacatgaatccggaggcgctgaccgcatggaaacgtgcggcagcagcggtctatcgtaaggataaagccagaaagagccgtcgtatctccctggaattcatgcttgagcaggcgaacaaattcgctaaccacaaagccatctggtttccgtataatatggattggcgtggtcgtgtttacgcggtatcgatgttcaacccgcagggtaatgacatgaccaagggtttgttgaccttggccaaaggtaaaccgattggcaaagaaggttactattggttgaagatccacggtgcgaactgcgcaggggtggataaggtaccgttcccggaacgtattaaattcatcgaggaaaaccacgaaaacattatggcgtgcgcaaagagcccgctggaaaacacgtggtgggcagagcaggacagtccattctgcttcttggcgttctgtttcgaatatgcaggtgtccagcaccacggcctgagctataactgcagcctgccgctggcctttgatggttcttgtagcggtattcaacactttagcgccatgctgcgcgatgaggttggtggcagagcagtgaatctgctgccaagcgaaaccgtgcaagatatctatggcattgtggctaagaaggttaatgaaatcctgcaagcagacgcgattaacggcacggacaacgaggttgtcaccgtgaccgatgaaaacaccggtgagatctcggagaaagtgaaactgggcaccaaagccttggctggccaatggctggcatacggcgttactcgctccgtgaccaagcgttcggtgatgacccttgcttacggcagcaaagagtttggtttccgccaacaggttctggaggatactatccaaccggccatcgactctggtaaaggcctgatgttcacgcagccgaatcaggcagcgggctatatggcgaagctgatttgggaatcggttagcgttaccgttgttgcagcggtggaggctatgaactggctgaaatctgcggcgaagctgttagctgcggaggtgaaggacaagaagacgggcgaaatcctgcgtaagcgctgcgcagtgcattgggttacgccggatggttttccggtatggcaggagtacaaaaagcctattcagacccgtctgaacctgatgtttctgggtcaatttcgtctgcagccgacgatcaacaccaataaggactccgagatcgacgcgcacaaacaggagtctggcatcgcacccaatttcgttcactcacaggacggttcccatctgcgtaagaccgtcgtgtgggcacacgagaagtatggcattgagtcgtttgcattgatccacgattcctttggtaccatcccggcggacgctgcgaacctgtttaaagcggttcgcgaaaccatggttgacacctatgaaagttgcgatgttctggcagacttttatgatcagttcgccgaccaactgcatgagtcccagctggataaaatgccggcgttaccggcgaagggcaacttaaatctccgcgacatcctggaatctgatttcgccttcgcgtaa

SEQ ID NO: 94 - DNA, 2646 bp, synthetic construct
  source 1..2646: mol_type = other DNA
atgaatacaattaacatagctaaaaatgatttcagcgatattgaactggctgcgatcccgtttaataccttggcggaccattatggtgagcgtctggcgcgtgagcaacttgctctggagcacgaatcctacgagatgggtgaagcgcgtttccggaagatgttcgagcgccagcttaaggctggcgaggtggcggataacgctgctgcgaagccgttgattacgaccctgctgccgaaaatgattgcgcgtattaacgattggttcgaggaagtgaaagcaaagcgtggtaaacgtccaaccgcattccagtttctgcaagagatcaagccggaggcggtggcatacattacgatcaaaaccactctcgcatgtctcaccagcgcggataatactacggtccaagcggtggccagcgcgattggccgcgcgattgaggacgaagcgcgttttggtcgcattcgtgacctggaagcgaaacattttaagaagaacgttgaagaacaattgaatgtgggccacgttcccaagaaagcgttcatgcaagtcgttgaagctgatatgctgagcaaaggcctgttaggtggtgaagcatggagcagctggcataaggaggactcaattcacgtcggcgtgcggtgcattgaaatgctgatcgaatcgaccggtatggttagcctgcatcgccaaaacgccggcgtggtgggtcaagatagcgaaacgattgaactggcgccagagtacgcggaagctatcgctaccagagccggcgcattggcggggatcagcccgatgttccagccgtgtgttgtaccaccgaagccgtggaccggtatcaccggtggaggttactgggcgaatggtagacgtccgttggcgttggttcgtacccatagcaaaaaggctctgatgcgttatgaagacgtttacatgccggaagtgtacaaagccatcaacatcgcgcagaacactgcgtggaaaatcaacaaaaaggtgttagctgtggcgaacgtaattacaaaatggaagcactgcccggttgaggacatcccggctattgaacgtgaagagctgccaatgaaaccagaggacattgacatgaatccggaggcgctgaccgcatggaaacgtgcggcagcagcggtctatcgtaaggataaagccagaaagagccgtcgtatctccctggaattcatgcttgagcaggcgaacaaattcgctaaccacaaagccatctggtttccgtataatatggattggcgtggtcgtgtttacgcggtatcgatgttcaacccgcagggtaatgacatgaccaagggtttgttgaccttggccaaaggtaaaccgattggcaaagaaggttactattggttgaagatccacggtgcgaactgcgcaggggtggataaggtaccgttcccggaacgtattaaattcatcgaggaaaaccacgaaaacattatggcgtgcgcaaagagcccgctggaaaacacgtggtgggcagagcaggacagtccattctgcttcttggcgttctgtttcgaatatgcaggtgtccagcaccacggcctgagctataactgcagcctgccgctggcctttgatggttcttgtagcggtattcaacactttagcgccatgctgcgcgatgaggttggtggcagagcagtgaatctgctgccaagcgaaaccgtgcaagatatctatggcattgtggctaagaaggttaatgaaatcctgcaagcagacgcgattaacggcacggacaacgaggttgtcaccgtgaccgatgaaaacaccggtgagatctcggagaaagtgaaactgggcaccaaagccttggctggccaatggctggcatacggcgttactcgctccgtgaccaagcgttcggtgatgacccttgcttacggcagcaaagagtttggtttccgccaacaggttctggaggatactatccaaccggccatcgactctggtaaaggcctgatgttcacgcagccgaatcaggcagcgggctatatggcgaagctgatttgggaatcggttagcgttaccgttgttgcagcggtggaggctatgaactggctgaaatctgcggcgaagctgttagctgcggaggtgaaggacaagaagacgggcgaaatcctgcgtaagcgctgcgcagtgcattgggttacgccggatggttttccggtatggcaggagtacaaaaagcctattcagacccgtctgaacctgatgtttctgggtcaatttcgtctgcagccgacgatcaacaccaataaggactccgagatcgacgcgcacaaacaggagtctggcatcgcacccaatttcgttcactcacaggacggttcccatctgcgtaagaccgtcgtgtgggcacacgagaagtatggcattgagtcgtttgcattgatccacgattcctttggtaccatcccggcggacgctgcgaacctgtttaaagcggttcgcgaaaccatggttgacacctatgaaagttgcgatgttctggcagacttttatgatcagttcgccgaccaactgcatgagtcccagctggataaaatgccggcgttaccggcgaagggcaacttaaatctccgcgacatcctggaatctgatttcgccttcgcgtaa

SEQ ID NO: 95 - DNA, 2652 bp, synthetic construct
  source 1..2652: mol_type = other DNA
atgaatacaattaacatagctaaaaatgatttcagcgatattgaactggctgcgatcccgtttaataccttggcggaccattatggtgagcgtctggcgcgtgagcaacttgctctggagcacgaatcctacgagatgggtgaagcgcgtttccggaagatgggagagcgccagcttaaggctggcgaggtggcggataacgctgctgcgaagccgttgattacgaccctgctgccgaaaatgattgcgcgtattaacgattggttcgaggaagtgaaagcaaagcgtggtaaacgtccaaccgcattccagtttctgcaagagatcaagccggaggcggtggcatacattacgatcaaaaccactctcgcatgtctcaccagcgcggataatactacggtccaagcggtggccagcgcgattggccgcgcgattgaggacgaagcgcgttttggtcgcattcgtgacctggaagcgaaacattttaagaagaacgttgaagaacaattgaataaacgcgtgggccacgttcacaagaaagcgttcatgcaagtcgttgaagctgatatgctgagcaaaggcctgttaggtggtgaagcatggagcagctggcataaggaggactcaattcacgtcggcgtgcggtgcattgaaatgctgatcgaatcgaccggtatggttagcctgcatcgccaaaacgccggcgtggtgggtcaagatagcgaaacgattgaactggcgccagagtacgcggaagctatcgctaccagagccggcgcattggcggggatcagcccgatgttccagccgtgtgttgtaccaccgaagccgtggaccggtatcaccggtggaggttactgggcgaatggtagacgtccgttggcgttggttcgtacccatagcaaaaaggctctgatgcgttatgaagacgtttacatgccggaagtgtacaaagccatcaacatcgcgcagaacactgcgtggaaaatcaacaaaaaggtgttagctgtggcgaacgtaattacaaaatggaagcactgcccggttgaggacatcccggctattgaacgtgaagagctgccaatgaaaccagaggacattgacatgaatccggaggcgctgaccgcatggaaacgtgcggcagcagcggtctatcgtaaggataaagccagaaagagccgtcgtatctccctggaattcatgcttgagcaggcgaacaaattcgctaaccacaaagccatctggtttccgtataatatggattggcgtggtcgtgtttacgcggtatcgatgttcaacccgcagggtaatgacatgaccaagggtttgttgaccttggccaaaggtaaaccgattggcaaagaaggttactattggttgaagatccacggtgcgaactgcgcaggggtggataaggtaccgttcccggaacgtattaaattcatcgaggaaaaccacgaaaacattatggcgtgcgcaaagagcccgctggaaaacacgtggtgggcagagcaggacagtccattctgcttcttggcgttctgtttcgaatatgcaggtgtccagcaccacggcctgagctataactgcagcctgccgctggcctttgatggttcttgtagcggtattcaacactttagcgccatgctgcgcgatgaggttggtggcagagcagtgaatctgctgccaagcgaaaccgtgcaagatatctatggcattgtggctaagaaggttaatgaaatcctgcaagcagacgcgattaacggcacggacaacgaggttgtcaccgtgaccgatgaaaacaccggtgagatctcggagaaagtgaaactgggcaccaaagccttggctggccaatggctggcatacggcgttactcgctccgtgaccaagcgttcggtgatgacccttgcttacggcagcaaagagtttggtttccgccaacaggttctggaggatactatccaaccggccatcgactctggtaaaggcctgatgttcacgcagccgaatcaggcagcgggctatatggcgaagctgatttgggaatcggttagcgttaccgttgttgcagcggtggaggctatgaactggctgaaatctgcggcgaagctgttagctgcggaggtgaaggacaagaagacgggcgaaatcctgcgtaagcgctgcgcagtgcattgggttacgccggatggttttccggtatggcaggagtacaaaaagcctattcagacccgtctgaacctgatgtttctgggtcaatttcgtctgcagccgacgatcaacaccaataaggactccgagatcgacgcgcacaaacaggagtctggcatcgcacccaatttcgttcactcacaggacggttcccatctgcgtaagaccgtcgtgtgggcacacgagaagtatggcattgagtcgtttgcattgatccacgattcctttggtaccatcccggcggacgctgcgaacctgtttaaagcggttcgcgaaaccatggttgacacctatgaaagttgcgatgttctggcagacttttatgatcagttcgccgaccaactgcatgagtcccagctggataaaatgccggcgttaccggcgaagggcaacttaaatctccgcgacatcctggaatctgatttcgccttcgcgtaa

SEQ ID NO: 96 - DNA, 2652 bp, synthetic construct
  source 1..2652: mol_type = other DNA
atgaatacaattaacatagctaaaaatgatttcagcgatattgaactggctgcgatcccgtttaataccttggcggaccattatggtgagcgtctggcgcgtgagcaacttgctctggagcacgaatcctacgagatgggtgaagcgcgtttccggaagatgcttgagcgccagcttaaggctggcgaggtggcggataacgctgctgcgaagccgttgattacgaccctgctgccgaaaatgattgcgcgtattaacgattggttcgaggaagtgaaagcaaagcgtggtaaacgtccaaccgcattccagtttctgcaagagatcaagccggaggcggtggcatacattacgatcaaaaccactctcgcatgtctcaccagcgcggataatactacggtccaagcggtggccagcgcgattggccgcgcgattgaggacgaagcgcgttttggtcgcattcgtgacctggaagcgaaacattttaagaagaacgttgaagaacaattgaataaacgcgtgggccacgtttacaagaaagcggaaatgcaagtcgttgaagctgatatgctgagcaaaggcctgttaggtggtgaagcatggagcagctggcataaggaggactcaattcacgtcggcgtgcggtgcattgaaatgctgatcgaatcgaccggtatggttagcctgcatcgccaaaacgccggcgtggtgggtcaagatagcgaaacgattgaactggcgccagagtacgcggaagctatcgctaccagagccggcgcattggcggggatcagcccgatgttccagccgtgtgttgtaccaccgaagccgtggaccggtatcaccggtggaggttactgggcgaatggtagacgtccgttggcgttggttcgtacccatagcaaaaaggctctgatgcgttatgaagacgtttacatgccggaagtgtacaaagccatcaacatcgcgcagaacactgcgtggaaaatcaacaaaaaggtgttagctgtggcgaacgtaattacaaaatggaagcactgcccggttgaggacatcccggctattgaacgtgaagagctgccaatgaaaccagaggacattgacatgaatccggaggcgctgaccgcatggaaacgtgcggcagcagcggtctatcgtaaggataaagccagaaagagccgtcgtatctccctggaattcatgcttgagcaggcgaacaaattcgctaaccacaaagccatctggtttccgtataatatggattggcgtggtcgtgtttacgcggtatcgatgttcaacccgcagggtaatgacatgaccaagggtttgttgaccttggccaaaggtaaaccgattggcaaagaaggttactattggttgaagatccacggtgcgaactgcgcaggggtggataaggtaccgttcccggaacgtattaaattcatcgaggaaaaccacgaaaacattatggcgtgcgcaaagagcccgctggaaaacacgtggtgggcagagcaggacagtccattctgcttcttggcgttctgtttcgaatatgcaggtgtccagcaccacggcctgagctataactgcagcctgccgctggcctttgatggttcttgtagcggtattcaacactttagcgccatgctgcgcgatgaggttggtggcagagcagtgaatctgctgccaagcgaaaccgtgcaagatatctatggcattgtggctaagaaggttaatgaaatcctgcaagcagacgcgattaacggcacggacaacgaggttgtcaccgtgaccgatgaaaacaccggtgagatctcggagaaagtgaaactgggcaccaaagccttggctggccaatggctggcatacggcgttactcgctccgtgaccaagcgttcggtgatgacccttgcttacggcagcaaagagtttggtttccgccaacaggttctggaggatactatccaaccggccatcgactctggtaaaggcctgatgttcacgcagccgaatcaggcagcgggctatatggcgaagctgatttgggaatcggttagcgttaccgttgttgcagcggtggaggctatgaactggctgaaatctgcggcgaagctgttagctgcggaggtgaaggacaagaagacgggcgaaatcctgcgtaagcgctgcgcagtgcattgggttacgccggatggttttccggtatggcaggagtacaaaaagcctattcagacccgtctgaacctgatgtttctgggtcaatttcgtctgcagccgacgatcaacaccaataaggactccgagatcgacgcgcacaaacaggagtctggcatcgcacccaatttcgttcactcacaggacggttcccatctgcgtaagaccgtcgtgtgggcacacgagaagtatggcattgagtcgtttgcattgatccacgattcctttggtaccatcccggcggacgctgcgaacctgtttaaagcggttcgcgaaaccatggttgacacctatgaaagttgcgatgttctggcagacttttatgatcagttcgccgaccaactgcatgagtcccagctggataaaatgccggcgttaccggcgaagggcaacttaaatctccgcgacatcctggaatctgatttcgccttcgcgtaa

SEQ ID NO: 97 - DNA, 2652 bp, synthetic construct
  source 1..2652: mol_type = other DNA
atgaatacaattaacatagctaaaaatgatttcagcgatattgaactggctgcgatcccgtttaataccttggcggaccattatggtgagcgtctggcgcgtgagcaacttgctctggagcacgaatcctacgagatgggtgaagcgcgtttccggaagatgcttgagcgccagcttaaggctggcgaggtggcggataacgctgctgcgaagccgttgattacgaccctgctgccgaaaatgattgcgcgtattaacgattggttcgaggaagtgaaagcaaagcgtggtaaacgtccaaccgcattccagtttctgcaagagatcaagccggaggcggtggcatacattacgatcaaaaccactctcgcatgtctcaccagcgcggataatactacggtccaagcggtggccagcgcgattggccgcgcgattgaggacgaagcgcgttttggtcgcattcgtgacctggaagcgaaacattttaagaagaacgttgaagaacaagaaaataaacgcgtgggccacgtttacaagaaagcgttcatgcaagtcgttgaagctgatatgctgagcaaaggcctgttaggtggtgaagcatggagcagctggcataaggaggactcaattcacgtcggcgtgcggtgcattgaaatgctgatcgaatcgaccggtatggttagcctgcatcgccaaaacgccggcgtggtgggtcaagatagcgaaacgattgaactggcgccagagtacgcggaagctatcgctaccagagccggcgcattggcggggatcagcccgatgttccagccgtgtgttgtaccaccgaagccgtggaccggtatcaccggtggaggttactgggcgaatggtagacgtccgttggcgttggttcgtacccatagcaaaaaggctctgatgcgttatgaagacgtttacatgccggaagtgtacaaagccatcaacatcgcgcagaacactgcgtggaaaatcaacaaaaaggtgttagctgtggcgaacgtaattacaaaatggaagcactgcccggttgaggacatcccggctattgaacgtgaagagctgccaatgaaaccagaggacattgacatgaatccggaggcgctgaccgcatggaaacgtgcggcagcagcggtctatcgtaaggataaagccagaaagagccgtcgtatctccctggaattcatgcttgagcaggcgaacaaattcgctaaccacaaagccatctggtttccgtataatatggattggcgtggtcgtgtttacgcggtatcgatgttcaacccgcagggtaatgacatgaccaagggtttgttgaccttggccaaaggtaaaccgattggcaaagaaggttactattggttgaagatccacggtgcgaactgcgcaggggtggataaggtaccgttcccggaacgtattaaattcatcgaggaaaaccacgaaaacattatggcgtgcgcaaagagcccgctggaaaacacgtggtgggcagagcaggacagtccattctgcttcttggcgttctgtttcgaatatgcaggtgtccagcaccacggcctgagctataactgcagcctgccgctggcctttgatggttcttgtagcggtattcaacactttagcgccatgctgcgcgatgaggttggtggcagagcagtgaatctgctgccaagcgaaaccgtgcaagatatctatggcattgtggctaagaaggttaatgaaatcctgcaagcagacgcgattaacggcacggacaacgaggttgtcaccgtgaccgatgaaaacaccggtgagatctcggagaaagtgaaactgggcaccaaagccttggctggccaatggctggcatacggcgttactcgctccgtgaccaagcgttcggtgatgacccttgcttacggcagcaaagagtttggtttccgccaacaggttctggaggatactatccaaccggccatcgactctggtaaaggcctgatgttcacgcagccgaatcaggcagcgggctatatggcgaagctgatttgggaatcggttagcgttaccgttgttgcagcggtggaggctatgaactggctgaaatctgcggcgaagctgttagctgcggaggtgaaggacaagaagacgggcgaaatcctgcgtaagcgctgcgcagtgcattgggttacgccggatggttttccggtatggcaggagtacaaaaagcctattcagacccgtctgaacctgatgtttctgggtcaatttcgtctgcagccgacgatcaacaccaataaggactccgagatcgacgcgcacaaacaggagtctggcatcgcacccaatttcgttcactcacaggacggttcccatctgcgtaagaccgtcgtgtgggcacacgagaagtatggcattgagtcgtttgcattgatccacgattcctttggtaccatcccggcggacgctgcgaacctgtttaaagcggttcgcgaaaccatggttgacacctatgaaagttgcgatgttctggcagacttttatgatcagttcgccgaccaactgcatgagtcccagctggataaaatgccggcgttaccggcgaagggcaacttaaatctccgcgacatcctggaatctgatttcgccttcgcgtaa

SEQ ID NO: 98 - DNA, 2652 bp, synthetic construct
  source 1..2652: mol_type = other DNA
atgaatacaattaacatagctaaaaatgatttcagcgatattgaactggctgcgatcccgtttaataccttggcggaccattatggtgagcgtctggcgcgtgagcaacttgctctggagcacgaatcctacgagatgggtgaagcgcgtttccggaagatgcttgagcgccagcttaaggctggcgaggtggcggataacgctgctgcgaagccgttgattacgaccctgctgccgaaaatgattgcgcgtattaacgattggttcgaggaagtgaaagcaaagcgtggtaaacgtccaaccgcattccagtttctgcaagagatcaagccggaggcggtggcatacattacgatcaaaaccactctcgcatgtctcaccagcgcggataatactacggtccaagcggtggccagcgcgattggccgcgcgattgaggacgaagcgcgttttggtcgcattcgtgacctggaagcgaaacattttaagaagaacgttgaagaacaattgaataaacgcgtgggccacgtttacaagaaagcgttcgaacaagtcgttgaagctgatatgctgagcaaaggcctgttaggtggtgaagcatggagcagctggcataaggaggactcaattcacgtcggcgtgcggtgcattgaaatgctgatcgaatcgaccggtatggttagcctgcatcgccaaaacgccggcgtggtgggtcaagatagcgaaacgattgaactggcgccagagtacgcggaagctatcgctaccagagccggcgcattggcggggatcagcccgatgttccagccgtgtgttgtaccaccgaagccgtggaccggtatcaccggtggaggttactgggcgaatggtagacgtccgttggcgttggttcgtacccatagcaaaaaggctctgatgcgttatgaagacgtttacatgccggaagtgtacaaagccatcaacatcgcgcagaacactgcgtggaaaatcaacaaaaaggtgttagctgtggcgaacgtaattacaaaatggaagcactgcccggttgaggacatcccggctattgaacgtgaagagctgccaatgaaaccagaggacattgacatgaatccggaggcgctgaccgcatggaaacgtgcggcagcagcggtctatcgtaaggataaagccagaaagagccgtcgtatctccctggaattcatgcttgagcaggcgaacaaattcgctaaccacaaagccatctggtttccgtataatatggattggcgtggtcgtgtttacgcggtatcgatgttcaacccgcagggtaatgacatgaccaagggtttgttgaccttggccaaaggtaaaccgattggcaaagaaggttactattggttgaagatccacggtgcgaactgcgcaggggtggataaggtaccgttcccggaacgtattaaattcatcgaggaaaaccacgaaaacattatggcgtgcgcaaagagcccgctggaaaacacgtggtgggcagagcaggacagtccattctgcttcttggcgttctgtttcgaatatgcaggtgtccagcaccacggcctgagctataactgcagcctgccgctggcctttgatggttcttgtagcggtattcaacactttagcgccatgctgcgcgatgaggttggtggcagagcagtgaatctgctgccaagcgaaaccgtgcaagatatctatggcattgtggctaagaaggttaatgaaatcctgcaagcagacgcgattaacggcacggacaacgaggttgtcaccgtgaccgatgaaaacaccggtgagatctcggagaaagtgaaactgggcaccaaagccttggctggccaatggctggcatacggcgttactcgctccgtgaccaagcgttcggtgatgacccttgcttacggcagcaaagagtttggtttccgccaacaggttctggaggatactatccaaccggccatcgactctggtaaaggcctgatgttcacgcagccgaatcaggcagcgggctatatggcgaagctgatttgggaatcggttagcgttaccgttgttgcagcggtggaggctatgaactggctgaaatctgcggcgaagctgttagctgcggaggtgaaggacaagaagacgggcgaaatcctgcgtaagcgctgcgcagtgcattgggttacgccggatggttttccggtatggcaggagtacaaaaagcctattcagacccgtctgaacctgatgtttctgggtcaatttcgtctgcagccgacgatcaacaccaataaggactccgagatcgacgcgcacaaacaggagtctggcatcgcacccaatttcgttcactcacaggacggttcccatctgcgtaagaccgtcgtgtgggcacacgagaagtatggcattgagtcgtttgcattgatccacgattcctttggtaccatcccggcggacgctgcgaacctgtttaaagcggttcgcgaaaccatggttgacacctatgaaagttgcgatgttctggcagacttttatgatcagttcgccgaccaactgcatgagtcccagctggataaaatgccggcgttaccggcgaagggcaacttaaatctccgcgacatcctggaatctgatttcgccttcgcgtaa

SEQ ID NO: 99 - DNA, 2652 bp, synthetic construct
  source 1..2652: mol_type = other DNA
atgaatacaattaacatagctaaaaatgatttcagcgatattgaactggctgcgatcccgtttaataccttggcggaccattatggtgagcgtctggcgcgtgagcaacttgctctggagcacgaatcctacgagatgggtgaagcgcgtttccggaagatgttcgagcgccagcttaaggctggcgaggtggcggataacgctgctgcgaagccgttgattacgaccctgctgccgaaaatgattgcgcgtattaacgattggttcgaggaagtgaaagcaaagcgtggtaaacgtccaaccgcattccagtttctgcaagagatcaagccggaggcggtggcatacattacgatcaaaaccactctcgcatgtctcaccagcgcggataatactacggtccaagcggtggccagcgcgattggccgcgcgattgaggacgaagcgcgttttggtcgcgatcgtgacctggaagcgaaacattttaagaagaacgttgaagaacaattgaataaacgcgtgggccacgtttacaagaaagcgttcatgcaagtcgttgaagctgatatgctgagcaaaggcctgttaggtggtgaagcatggagcagctggcataaggaggactcaattcacgtcggcgtgcggtgcattgaaatgctgatcgaatcgaccggtatggttagcctgcatcgccaaaacgccggcgtggtgggtcaagatagcgaaacgattgaactggcgccagagtacgcggaagctatcgctaccagagccggcgcattggcggggatcagcccgatgttccagccgtgtgttgtaccaccgaagccgtggaccggtatcaccggtggaggttactgggcgaatggtagacgtccgttggcgttggttcgtacccatagcaaaaaggctctgatgcgttatgaagacgtttacatgccggaagtgtacaaagccatcaacatcgcgcagaacactgcgtggaaaatcaacaaaaaggtgttagctgtggcgaacgtaattacaaaatggaagcactgcccggttgaggacatcccggctattgaacgtgaagagctgccaatgaaaccagaggacattgacatgaatccggaggcgctgaccgcatggaaacgtgcggcagcagcggtctatcgtaaggataaagccagaaagagccgtcgtatctccctggaattcatgcttgagcaggcgaacaaattcgctaaccacaaagccatctggtttccgtataatatggattggcgtggtcgtgtttacgcggtatcgatgttcaacccgcagggtaatgacatgaccaagggtttgttgaccttggccaaaggtaaaccgattggcaaagaaggttactattggttgaagatccacggtgcgaactgcgcaggggtggataaggtaccgttcccggaacgtattaaattcatcgaggaaaaccacgaaaacattatggcgtgcgcaaagagcccgctggaaaacacgtggtgggcagagcaggacagtccattctgcttcttggcgttctgtttcgaatatgcaggtgtccagcaccacggcctgagctataacagcagcctgccgctggcctttgatggttcttgtagcggtattcaacactttagcgccatgctgcgcgatgaggttggtggcagagcagtgaatctgctgccaagcgaaaccgtgcaagatatctatggcattgtggctaagaaggttaatgaaatcctgcaagcagacgcgattaacggcacggacaacgaggttgtcaccgtgaccgatgaaaacaccggtgagatctcggagaaagtgaaactgggcaccaaagccttggctggccaatggctggcatacggcgttactcgctccgtgaccaagcgttcggtgatgacccttgcttacggcagcaaagagtttggtttccgccaacaggttctggaggatactatccaaccggccatcgactctggtaaaggcctgatgttcacgcagccgaatcaggcagcgggctatatggcgaagctgatttgggaatcggttagcgttaccgttgttgcagcggtggaggctatgaactggctgaaatctgcggcgaagctgttagctgcggaggtgaaggacaagaagacgggcgaaatcctgcgtaagcgctgcgcagtgcattgggttacgccggatggttttccggtatggcaggagtacaaaaagcctattcagacccgtctgaacctgatgtttctgggtcaatttcgtctgcagccgacgatcaacaccaataaggactccgagatcgacgcgcacaaacaggagtctggcatcgcacccaatttcgttcactcacaggacggttcccatctgcgtaagaccgtcgtgtgggcacacgagaagtatggcattgagtcgtttgcattgatccacgattcctttggtaccatcccggcggacgctgcgaacctgtttaaagcggttcgcgaaaccatggttgacacctatgaaagttgcgatgttctggcagacttttatgatcagttcgccgaccaactgcatgagtcccagctggataaaatgccggcgttaccggcgaagggcaacttaaatctccgcgacatcctggaatctgatttcgccttcgcgtaa

SEQ ID NO: 100 - DNA, 2652 bp, synthetic construct
  source 1..2652: mol_type = other DNA
atgaatacaattaacatagctaaaaatgatttcagcgatattgaactggctgcgatcccgtttaataccttggcggaccattatggtgagcgtctggcgcgtgagcaacttgctctggagcacgaatcctacgagatgggtgaagcgcgtttccggaagatgttcgagcgccagcttaaggctggcgaggtggcggataacgctgctgcgaagccgttgattacgaccctgctgccgaaaatgattgcgcgtattaacgattggttcgaggaagtgaaagcaaagcgtggtaaacgtccaaccgcattccagtttctgcaagagatcaagccggaggcggtggcatacattacgatcaaaaccactctcgcatgtctcaccagcgcggataatactacggtccaagcggtggccagcgcgattggccgcgcgattgaggacgaagcgcgttttggtcgcgatcgtgacctggaagcgaaacattttaagaagaacgttgaagaacaattgaataaacgcgtgggccacgtttacaagaaagcgttcatgcaagtcgttgaagctgatatgctgagcaaaggcctgttaggtggtgaagcatggagcagctggcataaggaggactcaattcacgtcggcgtgcggtgcattgaaatgctgatcgaatcgaccggtatggttagcctgcatcgccaaaacgccggcgtggtgggtcaagatagcgaaacgattgaactggcgccagagtacgcggaagctatcgctaccagagccggcgcattggcggggatcagcccgatgttccagccgtgtgttgtaccaccgaagccgtggaccggtatcaccggtggaggttactgggcgaatggtagacgtccgttggcgttggttcgtacccatagcaaaaaggctctgatgcgttatgaagacgtttacatgccggaagtgtacaaagccatcaacatcgcgcagaacactgcgtggaaaatcaacaaaaaggtgttagctgtggcgaacgtaattacaaaatggaagcactgcccggttgaggacatcccggctattgaacgtgaagagctgccaatgaaaccagaggacattgacatgaatccggaggcgctgaccgcatggaaacgtgcggcagcagcggtctatcgtaaggataaagccagaaagagccgtcgtatctccctggaattcatgcttgagcaggcgaacaaattcgctaaccacaaagccatctggtttccgtataatatggattggcgtggtcgtgtttacgcggtatcgatgttcaacccgcagggtaatgacatgaccaagggtttgttgacctttgccaaaggtaaaccgattggcaaagaaggttactattggttgaagatccacggtgcgaactgcgcaggggtggataaggtaccgttcccggaacgtattaaattcatcgaggaaaaccacgaaaacattatggcgtgcgcaaagagcccgctggaaaacacgtggtgggcagagcaggacagtccattctgcttcttggcgttctgtttcgaatatgcaggtgtccagcaccacggcctgagctataactgcagcctgccgctggcctttgatggttcttgtagcggtattcaacactttagcgccatgctgcgcgatgaggttggtggcagagcagtgaatctgctgccaagcgaaaccgtgcaagatatctatggcattgtggctaagaaggttaatgaaatcctgcaagcagacgcgattaacggcacggacaacgaggttgtcaccgtgaccgatgaaaacaccggtgagatctcggagaaagtgaaactgggcaccaaagccttggctggccaatggctggcatacggcgttactcgctccgtgaccaagcgttcggtgatgacccttgcttacggcagcaaagagtttggtttccgccaacaggttctggaggatactatccaaccggccatcgactctggtaaaggcctgatgttcacgcagccgaatcaggcagcgggctatatggcgaagctgatttgggaatcggttagcgttaccgttgttgcagcggtggaggctatgaactggctgaaatctgcggcgaagctgttagctgcggaggtgaaggacaagaagacgggcgaaatcctgcgtaagcgctgcgcagtgcattgggttacgccggatggttttccggtatggcaggagtacaaaaagcctattcagacccgtctgaacctgatgtttctgggtcaatttcgtctgcagccgacgatcaacaccaataaggactccgagatcgacgcgcacaaacaggagtctggcatcgcacccaatttcgttcactcacaggacggttcccatctgcgtaagaccgtcgtgtgggcacacgagaagtatggcattgagtcgtttgcattgatccacgattcctttggtaccatcccggcggacgctgcgaacctgtttaaagcggttcgcgaaaccatggttgacacctatgaaagttgcgatgttctggcagacttttatgatcagttcgccgaccaactgcatgagtcccagctggataaaatgccggcgttaccggcgaagggcaacttaaatctccgcgacatcctggaatctgatttcgccttcgcgtaa

SEQ ID NO: 101 - DNA, 2652 bp, synthetic construct
  source 1..2652: mol_type = other DNA
atgaatacaattaacatagctaaaaatgatttcagcgatattgaactggctgcgatcccgtttaataccttggcggaccattatggtgagcgtctggcgcgtgagcaacttgctctggagcacgaatcctacgagatgggtgaagcgcgtttccggaagatgttcgagcgccagcttaaggctggcgaggtggcggataacgctgctgcgaagccgttgattacgaccctgctgccgaaaatgattgcgcgtattaacgattggttcgaggaagtgaaagcaaagcgtggtaaacgtccaaccgcattccagtttctgcaagagatcaagccggaggcggtggcatacattacgatcaaaaccactctcgcatgtctcaccagcgcggataatactacggtccaagcggtggccagcgcgattggccgcgcgattgaggacgaagcgcgttttggtcgcgatcgtgacctggaagcgaaacattttaagaagaacgttgaagaacaattgaataaacgcgtgggccacgtttacaagaaagcgttcatgcaagtcgttgaagctgatatgctgagcaaaggcctgttaggtggtgaagcatggagcagctggcataaggaggactcaattcacgtcggcgtgcggtgcattgaaatgctgatcgaatcgaccggtatggttagcctgcatcgccgaaacgccggcgtggtgggtcaagatagcgaaacgattgaactggcgccagagtacgcggaagctatcgctaccagagccggcgcattggcggggatcagcccgatgttccagccgtgtgttgtaccaccgaagccgtggaccggtatcaccggtggaggttactgggcgaatggtagacgtccgttggcgttggttcgtacccatagcaaaaaggctctgatgcgttatgaagacgtttacatgccggaagtgtacaaagccatcaacatcgcgcagaacactgcgtggaaaatcaacaaaaaggtgttagctgtggcgaacgtaattacaaaatggaagcactgcccggttgaggacatcccggctattgaacgtgaagagctgccaatgaaaccagaggacattgacatgaatccggaggcgctgaccgcatggaaacgtgcggcagcagcggtctatcgtaaggataaagccagaaagagccgtcgtatctccctggaattcatgcttgagcaggcgaacaaattcgctaaccacaaagccatctggtttccgtataatatggattggcgtggtcgtgtttacgcggtatcgatgttcaacccgcagggtaatgacatgaccaagggtttgttgaccttggccaaaggtaaaccgattggcaaagaaggttactattggttgaagatccacggtgcgaactgcgcaggggtggataaggtaccgttcccggaacgtattaaattcatcgaggaaaaccacgaaaacattatggcgtgcgcaaagagcccgctggaaaacacgtggtgggcagagcaggacagtccattccaattcttggcgttctgtttcgaatatgcaggtgtccagcaccacggcctgagctataactgcagcctgccgctggcctttgatggttcttgtagcggtattcaacactttagcgccatgctgcgcgatgaggttggtggcagagcagtgaatctgctgccaagcgaaaccgtgcaagatatctatggcattgtggctaagaaggttaatgaaatcctgcaagcagacgcgattaacggcacggacaacgaggttgtcaccgtgaccgatgaaaacaccggtgagatctcggagaaagtgaaactgggcaccaaagccttggctggccaatggctggcatacggcgttactcgctccgtgaccaagcgttcggtgatgacccttgcttacggcagcaaagagtttggtttccgccaacaggttctggaggatactatccaaccggccatcgactctggtaaaggcctgatgttcacgcagccgaatcaggcagcgggctatatggcgaagctgatttgggaatcggttagcgttaccgttgttgcagcggtggaggctatgaactggctgaaatctgcggcgaagctgttagctgcggaggtgaaggacaagaagacgggcgaaatcctgcgtaagcgctgcgcagtgcattgggttacgccggatggttttccggtatggcaggagtacaaaaagcctattcagacccgtctgaacctgatgtttctgggtcaatttcgtctgcagccgacgatcaacaccaataaggactccgagatcgacgcgcacaaacaggagtctggcatcgcacccaatttcgttcactcacaggacggttcccatctgcgtaagaccgtcgtgtgggcacacgagaagtatggcattgagtcgtttgcattgatccacgattcctttggtaccatcccggcggacgctgcgaacctgtttaaagcggttcgcgaaaccatggttgacacctatgaaagttgcgatgttctggcagacttttatgatcagttcgccgaccaactgcatgagtcccagctggataaaatgccggcgttaccggcgaagggcaacttaaatctccgcgacatcctggaatctgatttcgccttcgcgtaa

SEQ ID NO: 102 - DNA, 2652 bp, synthetic construct
  source 1..2652: mol_type = other DNA
atgaatacaattaacatagctaaaaatgatttcagcgatattgaactggctgcgatcccgtttaataccttggcggaccattatggtgagcgtctggcgcgtgagcaacttgctctggagcacgaatcctacgagatgggtgaagcgcgtttccggaagatgttcgagcgccagcttaaggctggcgaggtggcggataacgctgctgcgaagccgttgattacgaccctgctgccgaaaatgattgcgcgtattaacgattggttcgaggaagtgaaagcaaagcgtggtaaacgtccaaccgcattccagtttctgcaagagatcaagccggaggcggtggcatacattacgatcaaaaccactctcgcatgtctcaccagcgcggataatactacggtccaagcggtggccagcgcgattggccgcgcgattgaggacgaagcgcgttttggtcgcattcgtgacctggaagcgaaacattttaagaagaacgttgaagaacaattgaatgctggagtgggccacgtttacaagaaagcgttcatgcaagtcgttgaagctgatatgctgagcaaaggcctgttaggtggtgaagcatggagcagctggcataaggaggactcaattcacgtcggcgtgcggtgcattgaaatgctgatcgaatcgaccggtatggttagcctgcatcgccaaaacgccggcgtggtgggtcaagatagcgaaacgattgaactggcgccagagtacgcggaagctatcgctaccagagccggcgcattggcggggatcagcccgatgttccagccgtgtgttgtaccaccgaagccgtggaccggtatcaccggtggaggttactgggcgaatggtagacgtccgttggcgttggttcgtacccatagcaaaaaggctctgatgcgttatgaagacgtttacatgccggaagtgtacaaagccatcaacatcgcgcagaacactgcgtggaaaatcaacaaaaaggtgttagctgtggcgaacgtaattacaaaatggaagcactgcccggttgaggacatcccggctattgaacgtgaagagctgccaatgaaaccagaggacattgacatgaatccggaggcgctgaccgcatggaaacgtgcggcagcagcggtctatcgtgcggataaagccagaaagagccgtcgtatctccctggaattcatgcttgagcaggcgaacaaattcgctaaccacaaagccatctggtttccgtataatatggattggcgtggtcgtgtttacgcggtatcgatgttcaacccgcagggtaatgacatgaccaagggtttgttgaccttggccaaaggtaaaccgattggcaaagaaggttactattggttgaagatccacggtgcgaactgcgcaggggtggataaggtaccgttcccggaacgtattaaattcatcgaggaaaaccacgaaaacattatggcgtgcgcaaagagcccgctggaaaacacgtggtgggcagagcaggacagtccattctgcttcttggcgttctgtttcgaatatgcaggtgtccagcaccacggcctgagctataactgcagcctgccgctggcctttgatggttcttgtagcggtattcaacactttagcgccatgctgcgcgatgaggttggtggcagagcagtgaatctgctgccaagcgaaaccgtgcaagatatctatggcattgtggctaagaaggttaatgaaatcctgcaagcagacgcgattaacggcacggacaacgaggttgtcaccgtgaccgatgaaaacaccggtgagatctcggagaaagtgaaactgggcaccaaagccttggctggccaatggctggcatacggcgttactcgctccgtgaccaagcgttcggtgatgacccttgcttacggcagcaaagagtttggtttccgccaacaggttctggaggatactatccaaccggccatcgactctggtaaaggcctgatgttcacgcagccgaatcaggcagcgggctatatggcgaagctgatttgggaatcggttagcgttaccgttgttgcagcggtggaggctatgaactggctgaaatctgcggcgaagctgttagctgcggaggtgaaggacaagaagacgggcgaaatcctgcgtaagcgctgcgcagtgcattgggttacgccggatggttttccggtatggcaggagtacaaaaagcctattcagacccgtctgaacctgatgtttctgggtcaatttcgtctgcagccgacgatcaacaccaataaggactccgagatcgacgcgcacaaacaggagtctggcatcgcacccaatttcgttcactcacaggacggttcccatctgcgtaagaccgtcgtgtgggcacacgagaagtatggcattgagtcgtttgcattgatccacgattcctttggtaccatcccggcggacgctgcgaacctgtttaaagcggttcgcgaaaccatggttgacacctatgaaagttgcgatgttctggcagacttttatgatcagttcgccgaccaactgcatgagtcccagctggataaaatgccggcgttaccggcgaagggcaacttaaatctccgcgacatcctggaatctgatttcgccttcgcgtaa

SEQ ID NO: 103 - DNA, 2652 bp, synthetic construct
  source 1..2652: mol_type = other DNA
atgaatacaattaacatagctaaaaatgatttcagcgatattgaactggctgcgatcccgtttaataccttggcggaccattatggtgagcgtctggcgcgtgagcaacttgctctggagcacgaatcctacgagatgggtgaagcgcgtttccggaagatgttcgagcgccagcttaaggctggcgaggtggcggataacgctgctgcgaagccgttgattacgaccctgctgccgaaaatgattgcgcgtattaacgattggttcgaggaagtgaaagcaaagcgtggtaaacgtccaaccgcattccagtttctgcaagagatcaagccggaggcggtggcatacattacgatcaaaaccactctcgcatgtctcaccagcgcggataatactacggtccaagcggtggccagcgcgattggccgcgcgattgaggacgaagcgcgttttggtcgcattcgtgacctggaagcgaaacattttaagaagaacgttgaagaacaattgaatgctggagtgggccacgtttacaagaaagcgttcatgcaagtcgttgaagctgatatgctgagcaaaggcctgttaggtggtgaagcatggagcagctggcataaggaggactcaattcacgtcggcgtgcggtgcattgaaatgctgatcgaatcgaccggtatggttagcctgcatcgccaaaacgccggcgtggtgggtcaagatagcgaaacgattgaactggcgccagagtacgcggaagctatcgctaccagagccggcgcattggcggggatcagcccgatgttccagccgtgtgttgtaccaccgaagccgtggaccggtatcaccggtggaggttactgggcgaatggtagacgtccgttggcgttggttcgtacccatagcaaaaaggctctgatgcgttatgaagacgtttacatgccggaagtgtacaaagccatcaacatcgcgcagaacactgcgtggaaaatcaacaaaaaggtgttagctgtggcgaacgtaattacaaaatggaagcactgcccggttgaggacatcccggctattgaacgtgaagagctgccaatgaaaccagaggacattgacatgaatccggaggcgctgaccgcatggaaacgtgcggcagcagcggtctatcgtcaggataaagccagaaagagccgtcgtatctccctggaattcatgcttgagcaggcgaacaaattcgctaaccacaaagccatctggtttccgtataatatggattggcgtggtcgtgtttacgcggtatcgatgttcaacccgcagggtaatgacatgaccaagggtttgttgaccttggccaaaggtaaaccgattggcaaagaaggttactattggttgaagatccacggtgcgaactgcgcaggggtggataaggtaccgttcccggaacgtattaaattcatcgaggaaaaccacgaaaacattatggcgtgcgcaaagagcccgctggaaaacacgtggtgggcagagcaggacagtccattctgcttcttggcgttctgtttcgaatatgcaggtgtccagcaccacggcctgagctataactgcagcctgccgctggcctttgatggttcttgtagcggtattcaacactttagcgccatgctgcgcgatgaggttggtggcagagcagtgaatctgctgccaagcgaaaccgtgcaagatatctatggcattgtggctaagaaggttaatgaaatcctgcaagcagacgcgattaacggcacggacaacgaggttgtcaccgtgaccgatgaaaacaccggtgagatctcggagaaagtgaaactgggcaccaaagccttggctggccaatggctggcatacggcgttactcgctccgtgaccaagcgttcggtgatgacccttgcttacggcagcaaagagtttggtttccgccaacaggttctggaggatactatccaaccggccatcgactctggtaaaggcctgatgttcacgcagccgaatcaggcagcgggctatatggcgaagctgatttgggaatcggttagcgttaccgttgttgcagcggtggaggctatgaactggctgaaatctgcggcgaagctgttagctgcggaggtgaaggacaagaagacgggcgaaatcctgcgtaagcgctgcgcagtgcattgggttacgccggatggttttccggtatggcaggagtacaaaaagcctattcagacccgtctgaacctgatgtttctgggtcaatttcgtctgcagccgacgatcaacaccaataaggactccgagatcgacgcgcacaaacaggagtctggcatcgcacccaatttcgttcactcacaggacggttcccatctgcgtaagaccgtcgtgtgggcacacgagaagtatggcattgagtcgtttgcattgatccacgattcctttggtaccatcccggcggacgctgcgaacctgtttaaagcggttcgcgaaaccatggttgacacctatgaaagttgcgatgttctggcagacttttatgatcagttcgccgaccaactgcatgagtcccagctggataaaatgccggcgttaccggcgaagggcaacttaaatctccgcgacatcctggaatctgatttcgccttcgcgtaa

SEQ ID NO: 104 - DNA, 2652 bp, synthetic construct
  source 1..2652: mol_type = other DNA
atgaatacaattaacatagctaaaaatgatttcagcgatattgaactggctgcgatcccgtttaataccttggcggaccattatggtgagcgtctggcgcgtgagcaacttgctctggagcacgaatcctacgagatgggtgaagcgcgtttccggaagatgttcgagcgccagcttaaggctggcgaggtggcggataacgctgctgcgaagccgttgattacgaccctgctgccgaaaatgattgcgcgtattaacgattggttcgaggaagtgaaagcaaagcgtggtaaacgtccaaccgcattccagtttctgcaagagatcaagccggaggcggtggcatacattacgatcaaaaccactctcgcatgtctcaccagcgcggataatactacggtccaagcggtggccagcgcgattggccgcgcgattgaggacgaagcgcgttttggtcgcattcgtgacctggaagcgaaacattttaagaagaacgttgaagaacaattgaatgctggagtgggccacgtttacaagaaagcgttcatgcaagtcgttgaagctgatatgctgagcaaaggcctgttaggtggtgaagcatggagcagctggcataaggaggactcaattcacgtcggcgtgcggtgcattgaaatgctgatcgaatcgaccggtatggttagcctgcatcgccaaaacgccggcgtggtgggtcaagatagcgaaacgattgaactggcgccagagtacgcggaagctatcgctaccagagccggcgcattggcggggatcagcccgatgttccagccgtgtgttgtaccaccgaagccgtggaccggtatcaccggtggaggttactgggcgaatggtagacgtccgttggcgttggttcgtacccatagcaaaaaggctctgatgcgttatgaagacgtttacatgccggaagtgtacaaagccatcaacatcgcgcagaacactgcgtggaaaatcaacaaaaaggtgttagctgtggcgaacgtaattacaaaatggaagcactgcccggttgaggacatcccggctattgaacgtgaagagctgccaatgaaaccagaggacattgacatgaatccggaggcgctgaccgcatggaaacgtgcggcagcagcggtctatcgtaaggatgccgccagaaagagccgtcgtatctccctggaattcatgcttgagcaggcgaacaaattcgctaaccacaaagccatctggtttccgtataatatggattggcgtggtcgtgtttacgcggtatcgatgttcaacccgcagggtaatgacatgaccaagggtttgttgaccttggccaaaggtaaaccgattggcaaagaaggttactattggttgaagatccacggtgcgaactgcgcaggggtggataaggtaccgttcccggaacgtattaaattcatcgaggaaaaccacgaaaacattatggcgtgcgcaaagagcccgctggaaaacacgtggtgggcagagcaggacagtccattctgcttcttggcgttctgtttcgaatatgcaggtgtccagcaccacggcctgagctataactgcagcctgccgctggcctttgatggttcttgtagcggtattcaacactttagcgccatgctgcgcgatgaggttggtggcagagcagtgaatctgctgccaagcgaaaccgtgcaagatatctatggcattgtggctaagaaggttaatgaaatcctgcaagcagacgcgattaacggcacggacaacgaggttgtcaccgtgaccgatgaaaacaccggtgagatctcggagaaagtgaaactgggcaccaaagccttggctggccaatggctggcatacggcgttactcgctccgtgaccaagcgttcggtgatgacccttgcttacggcagcaaagagtttggtttccgccaacaggttctggaggatactatccaaccggccatcgactctggtaaaggcctgatgttcacgcagccgaatcaggcagcgggctatatggcgaagctgatttgggaatcggttagcgttaccgttgttgcagcggtggaggctatgaactggctgaaatctgcggcgaagctgttagctgcggaggtgaaggacaagaagacgggcgaaatcctgcgtaagcgctgcgcagtgcattgggttacgccggatggttttccggtatggcaggagtacaaaaagcctattcagacccgtctgaacctgatgtttctgggtcaatttcgtctgcagccgacgatcaacaccaataaggactccgagatcgacgcgcacaaacaggagtctggcatcgcacccaatttcgttcactcacaggacggttcccatctgcgtaagaccgtcgtgtgggcacacgagaagtatggcattgagtcgtttgcattgatccacgattcctttggtaccatcccggcggacgctgcgaacctgtttaaagcggttcgcgaaaccatggttgacacctatgaaagttgcgatgttctggcagacttttatgatcagttcgccgaccaactgcatgagtcccagctggataaaatgccggcgttaccggcgaagggcaacttaaatctccgcgacatcctggaatctgatttcgccttcgcgtaa

SEQ ID NO: 105 - DNA, 2652 bp, synthetic construct
  source 1..2652: mol_type = other DNA
atgaatacaattaacatagctaaaaatgatttcagcgatattgaactggctgcgatcccgtttaataccttggcggaccattatggtgagcgtctggcgcgtgagcaacttgctctggagcacgaatcctacgagatgggtgaagcgcgtttccggaagatgttcgagcgccagcttaaggctggcgaggtggcggataacgctgctgcgaagccgttgattacgaccctgctgccgaaaatgattgcgcgtattaacgattggttcgaggaagtgaaagcaaagcgtggtaaacgtccaaccgcattccagtttctgcaagagatcaagccggaggcggtggcatacattacgatcaaaaccactctcgcatgtctcaccagcgcggataatactacggtccaagcggtggccagcgcgattggccgcgcgattgaggacgaagcgcgttttggtcgcattcgtgacctggaagcgaaacattttaagaagaacgttgaagaacaagataataaacgcgtgggccacgtttacaagaaagcgttcatgcaagtcgttgaagctgatatgctgagcaaaggcctgttaggtggtgaagcatggagcagctggcataaggaggactcaattcacgtcggcgtgcggtgcattgaaatgctgatcgaatcgaccggtatggttagcctgcatcgccaaaacgccggcgtggtgggtcaagatagcgaaacgattgaactggcgccagagtacgcggaagctatcgctaccagagccggcgcattggcggggatcagcccgatgttccagccgtgtgttgtaccaccgaagccgtggaccggtatcaccggtggaggttactgggcgaatggtagacgtccgttggcgttggttcgtacccatagcaaaaaggctctgatgcgttatgaagacgtttacatgccggaagtgtacaaagccatcaacatcgcgcagaacactgcgtggaaaatcaacaaaaaggtgttagctgtggcgaacgtaattacaaaatggaagcactgcccggttgaggacatcccggctattgaacgtgaagagctgccaatgaaaccagaggacattgacatgaatccggaggcgctgaccgcatggaaacgtgcggcagcagcggtctatcgtaaggataaagccagaaagagccgtcgtatctccctggaattcatgcttgagcaggcgaacaaattcgctaaccacaaagccatctggtttccgtataatatggattggcgtggtcgtgtttacgcggtatcgatgttcaacccgcagggtaatgacatgaccaagggtttgttgaccttggccaaaggtaaaccgattggcaaagaaggttactattggttgaagatccacggtgcgaactgcgcaggggtggataaggtaccgttcccggaacgtattaaattcatcgaggaaaaccacgaaaacattatggcgtgcgcaaagagcccgctggaaaacacgtggtgggcagagcaggacagtccattctgcttcttggcgttctgtttcgaatatgcaggtgtccagcaccacggcctgagctataactgcagcctgccgctggcctttgatggttcttgtagcggtattcaacactttagcgccatgctgcgcgatgaggttggtggcagagcagtgaatctgctgccaagcgaaaccgtgcaagatatctatggcattgtggctaagaaggttaatgaaatcctgcaagcagacgcgattaacggcacggacaacgaggttgtcaccgtgaccgatgaaaacaccggtgagatctcggagaaagtgaaactgggcaccaaagccttggctggccaatggctggcatacggcgttactcgctccgtgaccaagcgttcggtgatgacccttgcttacggcagcaaagagtttggtttccgccaacaggttctggaggatactatccaaccggccatcgactctggtaaaggcctgatgttcacgcagccgaatcaggcagcgggctatatggcgaagctgatttgggaatcggttagcgttaccgttgttgcagcggtggaggctatgaactggctgaaatctgcggcgaagctgttagctgcggaggtgaaggacaagaagacgggcgaaatcctgcgtaagcgctgcgcagtgcattgggttacgccggatggttttccggtatggcaggagtacaaaaagcctattcagacccgtctgaacctgatgtttctgggtcaatttcgtctgcagccgacgatcaacaccaataaggactccgagatcgacgcgcacaaacaggagtctggcatcgcacccaatttcgttcactcacaggacggttcccatctgcgtaagaccgtcgtgtgggcacacgagaagtatggcattgagtcgtttgcattgatccacgattcctttggtaccatcccggcggacgctgcgaacctgtttaaagcggttcgcgaaaccatggttgacacctatgaaagttgcgatgttctggcagacttttatgatcagttcgccgaccaactgcatgagtcccagctggataaaatgccggcgttaccggcgaagggcaacttagatctccgcgacatcctggaatctgatttcgccttcgcgtaa

SEQ ID NO: 106 - DNA, 2646 bp, synthetic construct
  source 1..2646: mol_type = other DNA
atgaatacaattaacatagctaaaaatgatttcagcgatattgaactggctgcgatcccgtttaataccttggcggaccattatggtgagcgtctggcgcgtgagcaacttgctctggagcacgaatcctacgagatgggtgaagcgcgtttccggaagatgttcgagcgccaggctaaggctggcgaggtggcggataacgctgctgcgaagccgttgattacgaccctgctgccgaaaatgattgcgcgtattaacgattggttcgaggaagtgaaagcaaagcgtggtaaacgtccaaccgcattccagtttctgcaagagatcaagccggaggcggtggcatacattacgatcaaaaccactctcgcatgtctcaccagcgcggataatactacggtccaagcggtggccagcgcgattggccgcgcgattgaggacgaagcgcgttttggtcgcattcgtgacctggaagcgaaacattttaagaagaacgttgaagaacaattgaatgtgggccacgtttacaagaaagcgttcatgcaagtcgttgaagctgatatgctgagcaaaggcctgttaggtggtgaagcatggagcagctggcataaggaggactcaattcacgtcggcgtgcggtgcattgaaatgctgatcgaatcgaccggtatggttagcctgcatcgccaaaacgccggcgtggtgggtcaagatagcgaaacgattgaactggcgccagagtacgcggaagctatcgctaccagagccggcgcattggcggggatcagcccgatgttccagccgtgtgttgtaccaccgaagccgtggaccggtatcaccggtggaggttactgggcgaatggtagacgtccgttggcgttggttcgtacccatagcaaaaaggctctgatgcgttatgaagacgtttacatgccggaagtgtacaaagccatcaacatcgcgcagaacactgcgtggaaaatcaacaaaaaggtgttagctgtggcgaacgtaattacaaaatggaagcactgcccggttgaggacatcccggctattgaacgtgaagagctgccaatgaaaccagaggacattgacatgaatccggaggcgctgaccgcatggaaacgtgcggcagcagcggtctatcgtaaggataaagccagaaagagccgtcgtatctccctggaattcatgcttgagcaggcgaacaaattcgctaaccacaaagccatctggtttccgtataatatggattggcgtggtcgtgtttacgcggtatcgatgttcaacccgcagggtaatgacatgaccaagggtttgttgaccttggccaaaggtaaaccgattggcaaagaaggttactattggttgaagatccacggtgcgaactgcgcaggggtggataaggtaccgttcccggaacgtattaaattcatcgaggaaaaccacgaaaacattatggcgtgcgcaaagagcccgctggaaaacacgtggtgggcagagcaggacagtccattctgcttcttggcgttctgtttcgaatatgcaggtgtccagcaccacggcctgagctataactgcagcctgccgctggcctttgatggttcttgtagcggtattcaacactttagcgccatgctgcgcgatgaggttggtggcagagcagtgaatctgctgccaagcgaaaccgtgcaagatatctatggcattgtggctaagaaggttaatgaaatcctgcaagcagacgcgattaacggcacggacaacgaggttgtcaccgtgaccgatgaaaacaccggtgagatctcggagaaagtgaaactgggcaccaaagccttggctggccaatggctggcatacggcgttactcgctccgtgaccaagcgttcggtgatgacccttgcttacggcagcaaagagtttggtttccgccaacaggttctggaggatactatccaaccggccatcgactctggtaaaggcctgatgttcacgcagccgaatcaggcagcgggctatatggcgaagctgatttgggaatcggttagcgttaccgttgttgcagcggtggaggctatgaactggctgaaatctgcggcgaagctgttagctgcggaggtgaaggacaagaagacgggcgaaatcctgcgtaagcgctgcgcagtgcattgggttacgccggatggttttccggtatggcaggagtacaaaaagcctattcagacccgtctgaacctgatgtttctgggtcaatttcgtctgcagccgacgatcaacaccaataaggactccgagatcgacgcgcacaaacaggagtctggcatcgcacccaatttcgttcactcacaggacggttcccatctgcgtaagaccgtcgtgtgggcacacgagaagtatggcattgagtcgtttgcattgatccacgattcctttggtaccatcccggcggacgctgcgaacctgtttaaagcggttcgcgaaaccatggttgacacctatgaaagttgcgatgttctggcagacttttatgatcagttcgccgaccaactgcatgagtcccagctggataaaatgccggcgttaccggcgaagggcaacttaaatctccgcgacatcctggaatctgatttcgccttcgcgtaa

SEQ ID NO: 107 - DNA, 2652 bp, synthetic construct
  source 1..2652: mol_type = other DNA
atgaatacaattaacatagctaaaaatgatttcagcgatattgaactggctgcgatcccgtttaataccttggcggaccattatggtgagcgtctggcgcgtgagcaacttgctctggagcacgaatcctacgagatgggtgaagcgcgtttccggaagatgttcgagcgccaggctaaggctggcgaggtggcggataacgctgctgcgaagccgttgattacgaccctgctgccgaaaatgattgcgcgtattaacgattggttcgaggaagtgaaagcaaagcgtggtaaacgtccaaccgcattccagtttctgcaagagatcaagccggaggcggtggcatacattacgatcaaaaccactctcgcatgtctcaccagcgcggataatactacggtccaagcggtggccagcgcgattggccgcgcgattgaggacgaagcgcgttttggtcgcattcgtgacctggaagcgaaacattttaagaagaacgttgaagaacaattgaataaacgcgtgggccacgtttacaagaaagcgttcgaacaagtcgttgaagctgatatgctgagcaaaggcctgttaggtggtgaagcatggagcagctggcataaggaggactcaattcacgtcggcgtgcggtgcattgaaatgctgatcgaatcgaccggtatggttagcctgcatcgccaaaacgccggcgtggtgggtcaagatagcgaaacgattgaactggcgccagagtacgcggaagctatcgctaccagagccggcgcattggcggggatcagcccgatgttccagccgtgtgttgtaccaccgaagccgtggaccggtatcaccggtggaggttactgggcgaatggtagacgtccgttggcgttggttcgtacccatagcaaaaaggctctgatgcgttatgaagacgtttacatgccggaagtgtacaaagccatcaacatcgcgcagaacactgcgtggaaaatcaacaaaaaggtgttagctgtggcgaacgtaattacaaaatggaagcactgcccggttgaggacatcccggctattgaacgtgaagagctgccaatgaaaccagaggacattgacatgaatccggaggcgctgaccgcatggaaacgtgcggcagcagcggtctatcgtaaggataaagccagaaagagccgtcgtatctccctggaattcatgcttgagcaggcgaacaaattcgctaaccacaaagccatctggtttccgtataatatggattggcgtggtcgtgtttacgcggtatcgatgttcaacccgcagggtaatgacatgaccaagggtttgttgaccttggccaaaggtaaaccgattggcaaagaaggttactattggttgaagatccacggtgcgaactgcgcaggggtggataaggtaccgttcccggaacgtattaaattcatcgaggaaaaccacgaaaacattatggcgtgcgcaaagagcccgctggaaaacacgtggtgggcagagcaggacagtccattctgcttcttggcgttctgtttcgaatatgcaggtgtccagcaccacggcctgagctataactgcagcctgccgctggcctttgatggttcttgtagcggtattcaacactttagcgccatgctgcgcgatgaggttggtggcagagcagtgaatctgctgccaagcgaaaccgtgcaagatatctatggcattgtggctaagaaggttaatgaaatcctgcaagcagacgcgattaacggcacggacaacgaggttgtcaccgtgaccgatgaaaacaccggtgagatctcggagaaagtgaaactgggcaccaaagccttggctggccaatggctggcatacggcgttactcgctccgtgaccaagcgttcggtgatgacccttgcttacggcagcaaagagtttggtttccgccaacaggttctggaggatactatccaaccggccatcgactctggtaaaggcctgatgttcacgcagccgaatcaggcagcgggctatatggcgaagctgatttgggaatcggttagcgttaccgttgttgcagcggtggaggctatgaactggctgaaatctgcggcgaagctgttagctgcggaggtgaaggacaagaagacgggcgaaatcctgcgtaagcgctgcgcagtgcattgggttacgccggatggttttccggtatggcaggagtacaaaaagcctattcagacccgtctgaacctgatgtttctgggtcaatttcgtctgcagccgacgatcaacaccaataaggactccgagatcgacgcgcacaaacaggagtctggcatcgcacccaatttcgttcactcacaggacggttcccatctgcgtaagaccgtcgtgtgggcacacgagaagtatggcattgagtcgtttgcattgatccacgattcctttggtaccatcccggcggacgctgcgaacctgtttaaagcggttcgcgaaaccatggttgacacctatgaaagttgcgatgttctggcagacttttatgatcagttcgccgaccaactgcatgagtcccagctggataaaatgccggcgttaccggcgaagggcaacttaaatctccgcgacatcctggaatctgatttcgccttcgcgtaa

SEQ ID NO: 108 - DNA, 2652 bp, synthetic construct
  source 1..2652: mol_type = other DNA
atgaatacaattaacatagctaaaaatgatttcagcgatattgaactggctgcgatcccgtttaataccttggcggaccattatggtgagcgtctggcgcgtgagcaacttgctctggagcacgaatcctacgagatgggtgaagcgcgtttccggaagatgttcgagcgccagcttaaggctggcgaggtggcggataacgctgctgcgaagccgttgattacgaccctgctgccgaaaatgattgcgcgtattaacgattggttcgaggaagtgaaagcaaagcgtggtaaacgtccaaccgcattccagtttctgcaagagatcaagccggaggcggtggcatacattacgatcaaaaccactctcgcatgtctcaccagcgcggataatactacggtccaagcggtggccagcgcgattggccgcgcgattgaggacgaagcgcgttttggtcgcattcgtgacctggaagcgaaacattttaagaagaacgttgaagaacaattgaataaacgcgtgggccacgtttacaagaaagcgttcgaacaagtcgttgaagctgatatgctgagcaaaggcctgttaggtggtgaagcatggagcagctggcataaggaggactcagttcacgtcggcgtgcggtgcattgaaatgctgatcgaatcgaccggtatggttagcctgcatcgccaaaacgccggcgtggtgggtcaagatagcgaaacgattgaactggcgccagagtacgcggaagctatcgctaccagagccggcgcattggcggggatcagcccgatgttccagccgtgtgttgtaccaccgaagccgtggaccggtatcaccggtggaggttactgggcgaatggtagacgtccgttggcgttggttcgtacccatagcaaaaaggctctgatgcgttatgaagacgtttacatgccggaagtgtacaaagccatcaacatcgcgcagaacactgcgtggaaaatcaacaaaaaggtgttagctgtggcgaacgtaattacaaaatggaagcactgcccggttgaggacatcccggctattgaacgtgaagagctgccaatgaaaccagaggacattgacatgaatccggaggcgctgaccgcatggaaacgtgcggcagcagcggtctatcgtaaggataaagccagaaagagccgtcgtatctccctggaattcatgcttgagcaggcgaacaaattcgctaaccacaaagccatctggtttccgtataatatggattggcgtggtcgtgtttacgcggtatcgatgttcaacccgcagggtaatgacatgaccaagggtttgttgaccttggccaaaggtaaaccgattggcaaagaaggttactattggttgaagatccacggtgcgaactgcgcaggggtggataaggtaccgttcccggaacgtattaaattcatcgaggaaaaccacgaaaacattatggcgtgcgcaaagagcccgctggaaaacacgtggtgggcagagcaggacagtccattctgcttcttggcgttctgtttcgaatatgcaggtgtccagcaccacggcctgagctataactgcagcctgccgctggcctttgatggttcttgtagcggtattcaacactttagcgccatgctgcgcgatgaggttggtggcagagcagtgaatctgctgccaagcgaaaccgtgcaagatatctatggcattgtggctaagaaggttaatgaaatcctgcaagcagacgcgattaacggcacggacaacgaggttgtcaccgtgaccgatgaaaacaccggtgagatctcggagaaagtgaaactgggcaccaaagccttggctggccaatggctggcatacggcgttactcgctccgtgaccaagcgttcggtgatgacccttgcttacggcagcaaagagtttggtttccgccaacaggttctggaggatactatccaaccggccatcgactctggtaaaggcctgatgttcacgcagccgaatcaggcagcgggctatatggcgaagctgatttgggaatcggttagcgttaccgttgttgcagcggtggaggctatgaactggctgaaatctgcggcgaagctgttagctgcggaggtgaaggacaagaagacgggcgaaatcctgcgtaagcgctgcgcagtgcattgggttacgccggatggttttccggtatggcaggagtacaaaaagcctattcagacccgtctgaacctgatgtttctgggtcaatttcgtctgcagccgacgatcaacaccaataaggactccgagatcgacgcgcacaaacaggagtctggcatcgcacccaatttcgttcactcacaggacggttcccatctgcgtaagaccgtcgtgtgggcacacgagaagtatggcattgagtcgtttgcattgatccacgattcctttggtaccatcccggcggacgctgcgaacctgtttaaagcggttcgcgaaaccatggttgacacctatgaaagttgcgatgttctggcagacttttatgatcagttcgccgaccaactgcatgagtcccagctggataaaatgccggcgttaccggcgaagggcaacttaaatctccgcgacatcctggaatctgatttcgccttcgcgtaa

SEQ ID NO: 109 - DNA, 2652 bp, synthetic construct
  source 1..2652: mol_type = other DNA
atgaatacaattaacatagctaaaaatgatttcagcgatattgaactggctgcgatcccgtttaataccttggcggaccattatggtgagcgtctggcgcgtgagcaacttgctctggagcacgaatcctacgagatgggtgaagcgcgtttccggaagatgttcgagcgccagcttaaggctggcgaggtggcggataacgctgctgcgaagccgttgattacgaccctgctgccgaaaatgattgcgcgtattaacgattggttcgaggaagtgaaagcaaagcgtggtaaacgtccaaccgcattccagtttctgcaagagatcaagccggaggcggtggcatacattacgatcaaaaccactctcgcatgtctcaccagcgcggataatactacggtccaagcggtggccagcgcgattggccgcgcgattgaggacgaagcgcgttttggtcgcattcgtgacctggaagcgaaacattttaagaagaacgttgaagaacaattgaagaaacgcgtgggccacgtttacaagaaagcgttcgaacaagtcgttgaagctgatatgctgagcaaaggcctgttaggtggtgaagcatggagcagctggcataaggaggactcaattcacgtcggcgtgcggtgcattgaaatgctgatcgaatcgaccggtatggttagcctgcatcgccaaaacgccggcgtggtgggtcaagatagcgaaacgattgaactggcgccagagtacgcggaagctatcgctaccagagccggcgcattggcggggatcagcccgatgttccagccgtgtgttgtaccaccgaagccgtggaccggtatcaccggtggaggttactgggcgaatggtagacgtccgttggcgttggttcgtacccatagcaaaaaggctctgatgcgttatgaagacgtttacatgccggaagtgtacaaagccatcaacatcgcgcagaacactgcgtggaaaatcaacaaaaaggtgttagctgtggcgaacgtaattacaaaatggaagcactgcccggttgaggacatcccggctattgaacgtgaagagctgccaatgaaaccagaggacattgacatgaatccggaggcgctgaccgcatggaaacgtgcggcagcagcggtctatcgtaagaataaagccagaaagagccgtcgtatctccctggaattcatgcttgagcaggcgaacaaattcgctaaccacaaagccatctggtttccgtataatatggattggcgtggtcgtgtttacgcggtatcgatgttcaacccgcagggtaatgacatgaccaagggtttgttgaccttggccaaaggtaaaccgattggcaaagaaggttactattggttgaagatccacggtgcgaactgcgcaggggtggataaggtaccgttcccggaacgtattaaattcatcgaggaaaaccacgaaaacattatggcgtgcgcaaagagcccgctggaaaacacgtggtgggcagagcaggacagtccattctgcttcttggcgttctgtttcgaatatgcaggtgtccagcaccacggcctgagctataactgcagcctgccgctggcctttgatggttcttgtagcggtattcaacactttagcgccatgctgcgcgatgaggttggtggcagagcagtgaatctgctgccaagcgaaaccgtgcaagatatctatggcattgtggctaagaaggttaatgaaatcctgcaagcagacgcgattaacggcacggacaacgaggttgtcaccgtgaccgatgaaaacaccggtgagatctcggagaaagtgaaactgggcaccaaagccttggctggccaatggctggcatacggcgttactcgctccgtgaccaagcgttcggtgatgacccttgcttacggcagcaaagagtttggtttccgccaacaggttctggaggatactatccaaccggccatcgactctggtaaaggcctgatgttcacgcagccgaatcaggcagcgggctatatggcgaagctgatttgggaatcggttagcgttaccgttgttgcagcggtggaggctatgaactggctgaaatctgcggcgaagctgttagctgcggaggtgaaggacaagaagacgggcgaaatcctgcgtaagcgctgcgcagtgcattgggttacgccggatggttttccggtatggcaggagtacaaaaagcctattcagacccgtctgaacctgatgtttctgggtcaatttcgtctgcagccgacgatcaacaccaataaggactccgagatcgacgcgcacaaacaggagtctggcatcgcacccaatttcgttcactcacaggacggttcccatctgcgtaagaccgtcgtgtgggcacacgagaagtatggcattgagtcgtttgcattgatccacgattcctttggtaccatcccggcggacgctgcgaacctgtttaaagcggttcgcgaaaccatggttgacacctatgaaagttgcgatgttctggcagacttttatgatcagttcgccgaccaactgcatgagtcccagctggataaaatgccggcgttaccggcgaagggcaacttaaatctccgcgacatcctggaatctgatttcgccttcgcgtaa

SEQ ID NO: 110 - DNA, 2646 bp, synthetic construct
  source 1..2646: mol_type = other DNA
atgaatacaattaacatagctaaaaatgatttcagcgatattgaactggctgcgatcccgtttaataccttggcggaccattatggtgagcgtctggcggctgagcaacttgctctggagcacgaatcctacgagatgggtgaagcgcgtttccggaagatgttcgagcgccagcttaaggctggcgaggtggcggataacgctgctgcgaagccgttgattacgaccctgctgccgaaaatgattgcgcgtattaacgattggttcgaggaagtgaaagcaaagcgtggtaaacgtccaaccgcattccagtttctgcaagagatcaagccggaggcggtggcatacattacgatcaaaaccactctcgcatgtctcaccagcgcggataatactacggtccaagcggtggccagcgcgattggccgcgcgattgaggacgaagcgcgttttggtcgcattcgtgacctggaagcgaaacattttaagaagaacgttgaagaacaattgaatgtgggccacgtttacaagaaagcgttcatgcaagtcgttgaagctgatatgctgagcaaaggcctgttaggtggtgaagcatggagcagctggcataaggaggactcaattcacgtcggcgtgcggtgcattgaaatgctgatcgaatcgaccggtatggttagcctgcatcgccaaaacgccggcgtggtgggtcaagatagcgaaacgattgaactggcgccagagtacgcggaagctatcgctaccagagccggcgcattggcggggatcagcccgatgttccagccgtgtgttgtaccaccgaagccgtggaccggtatcaccggtggaggttactgggcgaatggtagacgtccgttggcgttggttcgtacccatagcaaaaaggctctgatgcgttatgaagacgtttacatgccggaagtgtacaaagccatcaacatcgcgcagaacactgcgtggaaaatcaacaaaaaggtgttagctgtggcgaacgtaattacaaaatggaagcactgcccggttgaggacatcccggctattgaacgtgaagagctgccaatgaaaccagaggacattgacatgaatccggaggcgctgaccgcatggaaacgtgcggcagcagcggtctatcgtaaggataaagccagaaagagccgtcgtatctccctggaattcatgcttgagcaggcgaacaaattcgctaaccacaaagccatctggtttccgtataatatggattggcgtggtcgtgtttacgcggtatcgatgttcaacccgcagggtaatgacatgaccaagggtttgttgaccttggccaaaggtaaaccgattggcaaagaaggttactattggttgaagatccacggtgcgaactgcgcaggggtggataaggtaccgttcccggaacgtattaaattcatcgaggaaaaccacgaaaacattatggcgtgcgcaaagagcccgctggaaaacacgtggtgggcagagcaggacagtccattctgcttcttggcgttctgtttcgaatatgcaggtgtccagcaccacggcctgagctataactgcagcctgccgctggcctttgatggttcttgtagcggtattcaacactttagcgccatgctgcgcgatgaggttggtggcagagcagtgaatctgctgccaagcgaaaccgtgcaagatatctatggcattgtggctaagaaggttaatgaaatcctgcaagcagacgcgattaacggcacggacaacgaggttgtcaccgtgaccgatgaaaacaccggtgagatctcggagaaagtgaaactgggcaccaaagccttggctggccaatggctggcatacggcgttactcgctccgtgaccaagcgttcggtgatgacccttgcttacggcagcaaagagtttggtttccgccaacaggttctggaggatactatccaaccggccatcgactctggtaaaggcctgatgttcacgcagccgaatcaggcagcgggctatatggcgaagctgatttgggaatcggttagcgttaccgttgttgcagcggtggaggctatgaactggctgaaatctgcggcgaagctgttagctgcggaggtgaaggacaagaagacgggcgaaatcctgcgtaagcgctgcgcagtgcattgggttacgccggatggttttccggtatggcaggagtacaaaaagcctattcagacccgtctgaacctgatgtttctgggtcaatttcgtctgcagccgacgatcaacaccaataaggactccgagatcgacgcgcacaaacaggagtctggcatcgcacccaatttcgttcactcacaggacggttcccatctgcgtaagaccgtcgtgtgggcacacgagaagtatggcattgagtcgtttgcattgatccacgattcctttggtaccatcccggcggacgctgcgaacctgtttaaagcggttcgcgaaaccatggttgacacctatgaaagttgcgatgttctggcagacttttatgatcagttcgccgaccaactgcatgagtcccagctggataaaatgccggcgttaccggcgaagggcaacttaaatctccgcgacatcctggaatctgatttcgccttcgcgtaa

SEQ ID NO: 111 - DNA, 2652 bp, synthetic construct
  source 1..2652: mol_type = other DNA
atgaatacaattaacatagctaaaaatgatttcagcgatattgaactggctgcgatcccgtttaataccttggcggaccattatggtgagcgtctggcggctgagcaacttgctctggagcacgaatcctacgagatgggtgaagcgcgtttccggaagatgttcgagcgccagcttaaggctggcgaggtggcggataacgctgctgcgaagccgttgattacgaccctgctgccgaaaatgattgcgcgtattaacgattggttcgaggaagtgaaagcaaagcgtggtaaacgtccaaccgcattccagtttctgcaagagatcaagccggaggcggtggcatacattacgatcaaaaccactctcgcatgtctcaccagcgcggataatactacggtccaagcggtggccagcgcgattggccgcgcgattgaggacgaagcgcgttttggtcgcattcgtgacctggaagcgaaacattttaagaagaacgttgaagaacaattgaataaacgcgtgggccacgtttacaagaaagcggaaatgcaagtcgttgaagctgatatgctgagcaaaggcctgttaggtggtgaagcatggagcagctggcataaggaggactcaattcacgtcggcgtgcggtgcattgaaatgctgatcgaatcgaccggtatggttagcctgcatcgccaaaacgccggcgtggtgggtcaagatagcgaaacgattgaactggcgccagagtacgcggaagctatcgctaccagagccggcgcattggcggggatcagcccgatgttccagccgtgtgttgtaccaccgaagccgtggaccggtatcaccggtggaggttactgggcgaatggtagacgtccgttggcgttggttcgtacccatagcaaaaaggctctgatgcgttatgaagacgtttacatgccggaagtgtacaaagccatcaacatcgcgcagaacactgcgtggaaaatcaacaaaaaggtgttagctgtggcgaacgtaattacaaaatggaagcactgcccggttgaggacatcccggctattgaacgtgaagagctgccaatgaaaccagaggacattgacatgaatccggaggcgctgaccgcatggaaacgtgcggcagcagcggtctatcgtaaggataaagccagaaagagccgtcgtatctccctggaattcatgcttgagcaggcgaacaaattcgctaaccacaaagccatctggtttccgtataatatggattggcgtggtcgtgtttacgcggtatcgatgttcaacccgcagggtaatgacatgaccaagggtttgttgaccttggccaaaggtaaaccgattggcaaagaaggttactattggttgaagatccacggtgcgaactgcgcaggggtggataaggtaccgttcccggaacgtattaaattcatcgaggaaaaccacgaaaacattatggcgtgcgcaaagagcccgctggaaaacacgtggtgggcagagcaggacagtccattctgcttcttggcgttctgtttcgaatatgcaggtgtccagcaccacggcctgagctataactgcagcctgccgctggcctttgatggttcttgtagcggtattcaacactttagcgccatgctgcgcgatgaggttggtggcagagcagtgaatctgctgccaagcgaaaccgtgcaagatatctatggcattgtggctaagaaggttaatgaaatcctgcaagcagacgcgattaacggcacggacaacgaggttgtcaccgtgaccgatgaaaacaccggtgagatctcggagaaagtgaaactgggcaccaaagccttggctggccaatggctggcatacggcgttactcgctccgtgaccaagcgttcggtgatgacccttgcttacggcagcaaagagtttggtttccgccaacaggttctggaggatactatccaaccggccatcgactctggtaaaggcctgatgttcacgcagccgaatcaggcagcgggctatatggcgaagctgatttgggaatcggttagcgttaccgttgttgcagcggtggaggctatgaactggctgaaatctgcggcgaagctgttagctgcggaggtgaaggacaagaagacgggcgaaatcctgcgtaagcgctgcgcagtgcattgggttacgccggatggttttccggtatggcaggagtacaaaaagcctattcagacccgtctgaacctgatgtttctgggtcaatttcgtctgcagccgacgatcaacaccaataaggactccgagatcgacgcgcacaaacaggagtctggcatcgcacccaatttcgttcactcacaggacggttcccatctgcgtaagaccgtcgtgtgggcacacgagaagtatggcattgagtcgtttgcattgatccacgattcctttggtaccatcccggcggacgctgcgaacctgtttaaagcggttcgcgaaaccatggttgacacctatgaaagttgcgatgttctggcagacttttatgatcagttcgccgaccaactgcatgagtcccagctggataaaatgccggcgttaccggcgaagggcaacttaaatctccgcgacatcctggaatctgatttcgccttcgcgtaa

SEQ ID NO: 112 - DNA, 2652 bp, synthetic construct
  source 1..2652: mol_type = other DNA
atgaatacaattaacatagctaaaaatgatttcagcgatattgaactggctgcgatcccgtttaataccttggcggaccattatggtgagcgtctggcggctgagcaacttgctctggagcacgaatcctacgagatgggtgaagcgcgtttccggaagatgttcgagcgccagcttaaggctggcgaggtggcggataacgctgctgcgaagccgttgattacgaccctgctgccgaaaatgattgcgcgtattaacgattggttcgaggaagtgaaagcaaagcgtggtaaacgtccaaccgcattccagtttctgcaagagatcaagccggaggcggtggcatacattacgatcaaaaccactctcgcatgtctcaccagcgcggataatactacggtccaagcggtggccagcgcgattggccgcgcgattgaggacgaagcgcgttttggtcgcattcgtgacctggaagcgaaacattttaagaagaacgttgaagaacaagaaaataaacgcgtgggccacgtttacaagaaagcgttcatgcaagtcgttgaagctgatatgctgagcaaaggcctgttaggtggtgaagcatggagcagctggcataaggaggactcaattcacgtcggcgtgcggtgcattgaaatgctgatcgaatcgaccggtatggttagcctgcatcgccaaaacgccggcgtggtgggtcaagatagcgaaacgattgaactggcgccagagtacgcggaagctatcgctaccagagccggcgcattggcggggatcagcccgatgttccagccgtgtgttgtaccaccgaagccgtggaccggtatcaccggtggaggttactgggcgaatggtagacgtccgttggcgttggttcgtacccatagcaaaaaggctctgatgcgttatgaagacgtttacatgccggaagtgtacaaagccatcaacatcgcgcagaacactgcgtggaaaatcaacaaaaaggtgttagctgtggcgaacgtaattacaaaatggaagcactgcccggttgaggacatcccggctattgaacgtgaagagctgccaatgaaaccagaggacattgacatgaatccggaggcgctgaccgcatggaaacgtgcggcagcagcggtctatcgtaaggataaagccagaaagagccgtcgtatctccctggaattcatgcttgagcaggcgaacaaattcgctaaccacaaagccatctggtttccgtataatatggattggcgtggtcgtgtttacgcggtatcgatgttcaacccgcagggtaatgacatgaccaagggtttgttgaccttggccaaaggtaaaccgattggcaaagaaggttactattggttgaagatccacggtgcgaactgcgcaggggtggataaggtaccgttcccggaacgtattaaattcatcgaggaaaaccacgaaaacattatggcgtgcgcaaagagcccgctggaaaacacgtggtgggcagagcaggacagtccattctgcttcttggcgttctgtttcgaatatgcaggtgtccagcaccacggcctgagctataactgcagcctgccgctggcctttgatggttcttgtagcggtattcaacactttagcgccatgctgcgcgatgaggttggtggcagagcagtgaatctgctgccaagcgaaaccgtgcaagatatctatggcattgtggctaagaaggttaatgaaatcctgcaagcagacgcgattaacggcacggacaacgaggttgtcaccgtgaccgatgaaaacaccggtgagatctcggagaaagtgaaactgggcaccaaagccttggctggccaatggctggcatacggcgttactcgctccgtgaccaagcgttcggtgatgacccttgcttacggcagcaaagagtttggtttccgccaacaggttctggaggatactatccaaccggccatcgactctggtaaaggcctgatgttcacgcagccgaatcaggcagcgggctatatggcgaagctgatttgggaatcggttagcgttaccgttgttgcagcggtggaggctatgaactggctgaaatctgcggcgaagctgttagctgcggaggtgaaggacaagaagacgggcgaaatcctgcgtaagcgctgcgcagtgcattgggttacgccggatggttttccggtatggcaggagtacaaaaagcctattcagacccgtctgaacctgatgtttctgggtcaatttcgtctgcagccgacgatcaacaccaataaggactccgagatcgacgcgcacaaacaggagtctggcatcgcacccaatttcgttcactcacaggacggttcccatctgcgtaagaccgtcgtgtgggcacacgagaagtatggcattgagtcgtttgcattgatccacgattcctttggtaccatcccggcggacgctgcgaacctgtttaaagcggttcgcgaaaccatggttgacacctatgaaagttgcgatgttctggcagacttttatgatcagttcgccgaccaactgcatgagtcccagctggataaaatgccggcgttaccggcgaagggcaacttaaatctccgcgacatcctggaatctgatttcgccttcgcgtaa

SEQ ID NO: 113 - DNA, 2652 bp, synthetic construct
  source 1..2652: mol_type = other DNA
atgaatacaattaacatagctaaaaatgatttcagcgatattgaactggctgcgatcccgtttaataccttggcggaccattatggtgagcgtctggcgcgtgagcaacttgctctggagcacgaatcctacgagatgggtgaagcgcgtttccggaagatgttcgagcgccagcttaaggctggcgaggtggcggataacgctgctgcgaagccgttgattacgaccctgctgccgaaaatgattgcgcgtattaacgattggttcgaggaagtgaaagcaaagcgtggtaaacgtccaaccgcattccagtttctgcaagagatcaagccggaggcggtggcatacattacgatcaaaaccactctcgcatgtctcaccagcgcggataatactacggtccaagcggtggccagcgcgattggccgcgcgattgaggacgaagcgcgttttggtcgcattcgtgacctggaagcgaaacattttaagaagaacgttgaagaacaattgaataaacgcgtgggccacgtttacaagaaagcgttcgaacaagtcgttgaagctgatatgctgagcaaaggcctgttaggtggtgaagcatggagcagctggcataaggaggactcagttcacgtcggcgtgcggtgcattgaaatgctgatcgaatcgaccggtatggttagcctgcatcgccaaaacgccggcgtggtgggtcaagatagcgaaacgattgaactggcgccagagtacgcggaagctatcgctaccagagccggcgcattggcggggatcagcccgatgttccagccgtgtgttgtaccaccgaagccgtggaccggtatcaccggtggaggttactgggcgaatggtagacgtccgttggcgttggttcgtacccatagcaaaaaggctctgatgcgttatgaagacgtttacatgccggaagtgtacaaagccatcaacatcgcgcagaacactgcgtggaaaatcaacaaaaaggtgttagctgtggcgaacgtaattacaaaatggaagcactgcccggttgaggacatcccggctattgaacgtgaagagctgccaatgaaaccagaggacattgacatgaatccggaggcgctgaccgcatggaaacgtgcggcagcagcggtctatcacaaggataaagccagaaagagccgtcgtatctccctggaattcatgcttgagcaggcgaacaaattcgctaaccacaaagccatctggtttccgtataatatggattggcgtggtcgtgtttacgcggtatcgatgttcaacccgcagggtaatgacatgaccaagggtttgttgaccttggccaaaggtaaaccgattggcaaagaaggttactattggttgaagatccacggtgcgaactgcgcaggggtggataaggtaccgttcccggaacgtattaaattcatcgaggaaaaccacgaaaacattatggcgtgcgcaaagagcccgctggaaaacacgtggtgggcagagcaggacagtccattctgcttcttggcgttctgtttcgaatatgcaggtgtccagcaccacggcctgagctataactgcagcctgccgctggcctttgatggttcttgtagcggtattcaacactttagcgccatgctgcgcgatgaggttggtggcagagcagtgaatctgctgccaagcgaaaccgtgcaagatatctatggcattgtggctaagaaggttaatgaaatcctgcaagcagacgcgattaacggcacggacaacgaggttgtcaccgtgaccgatgaaaacaccggtgagatctcggagaaagtgaaactgggcaccaaagccttggctggccaatggctggcatacggcgttactcgctccgtgaccaagcgttcggtgatgacccttgcttacggcagcaaagagtttggtttccgccaacaggttctggaggatactatccaaccggccatcgactctggtaaaggcctgatgttcacgcagccgaatcaggcagcgggctatatggcgaagctgatttgggaatcggttagcgttaccgttgttgcagcggtggaggctatgaactggctgaaatctgcggcgaagctgttagctgcggaggtgaaggacaagaagacgggcgaaatcctgcgtaagcgctgcgcagtgcattgggttacgccggatggttttccggtatggcaggagtacaaaaagcctattcagacccgtctgaacctgatgtttctgggtcaatttcgtctgcagccgacgatcaacaccaataaggactccgagatcgacgcgcacaaacaggagtctggcatcgcacccaatttcgttcactcacaggacggttcccatctgcgtaagaccgtcgtgtgggcacacgagaagtatggcattgagtcgtttgcattgatccacgattcctttggtaccatcccggcggacgctgcgaacctgtttaaagcggttcgcgaaaccatggttgacacctatgaaagttgcgatgttctggcagacttttatgatcagttcgccgaccaactgcatgagtcccagctggataaaatgccggcgttaccggcgaagggcaacttaaatctccgcgacatcctggaatctgatttcgccttcgcgtaa

SEQ ID NO: 114 - DNA, 2652 bp, synthetic construct
  source 1..2652: mol_type = other DNA
atgaatacaattaacatagctaaaaatgatttcagcgatattgaactggctgcgatcccgtttaataccttggcggaccattatggtgagcgtctggcgcgtgagcaacttgctctggagcacgaatcctacgagatgggtgaagcgcgtttccggaagatgttcgagcgccagcttaaggctggcgaggtggcggataacgctgctgcgaagccgttgattacgaccctgctgccgaaaatgattgcgcgtattaacgattggttcgaggaagtgaaagcaaagcgtggtaaacgtccaaccgcattccagtttctgcaagagatcaagccggaggcggtggcatacattacgatcaaaaccactctcgcatgtctcaccagcgcggataatactacggtccaagcggtggccagcgcgattggccgcgcgattgaggacgaagcgcgttttggtcgcattcgtgacctggaagcgaaacattttaagaagaacgttgaagaacaattgaataaacgcgtgggccacgtttacaagaaagcgttcgaacaagtcgttgaagctgatatgctgagcaaaggcctgttaggtggtgaagcatggagcagctggcataaggaggactcagttcacgtcggcgtgcggtgcattgaaatgctgatcgaatcgaccggtatggttagcctgcatcgccaaaacgccggcgtggtgggtcaagatagcgaaacgattgaactggcgccagagtacgcggaagctatcgctaccagagccggcgcattggcggggatcagcccgatgttccagccgtgtgttgtaccaccgaagccgtggaccggtatcaccggtggaggttactgggcgaatggtagacgtccgttggcgttggttcgtacccatagcaaaaaggctctgatgcgttatgaagacgtttacatgccggaagtgtacaaagccatcaacatcgcgcagaacactgcgtggaaaatcaacaaaaaggtgttagctgtggcgaacgtaattacaaaatggaagcactgcccggttgaggacatcccggctattgaacgtgaagagctgccaatgaaaccagaggacattgacatgaatccggaggcgctgaccgcatggaaacgtgcggcagcagcggtctataataaggataaagccagaaagagccgtcgtatctccctggaattcatgcttgagcaggcgaacaaattcgctaaccacaaagccatctggtttccgtataatatggattggcgtggtcgtgtttacgcggtatcgatgttcaacccgcagggtaatgacatgaccaagggtttgttgaccttggccaaaggtaaaccgattggcaaagaaggttactattggttgaagatccacggtgcgaactgcgcaggggtggataaggtaccgttcccggaacgtattaaattcatcgaggaaaaccacgaaaacattatggcgtgcgcaaagagcccgctggaaaacacgtggtgggcagagcaggacagtccattctgcttcttggcgttctgtttcgaatatgcaggtgtccagcaccacggcctgagctataactgcagcctgccgctggcctttgatggttcttgtagcggtattcaacactttagcgccatgctgcgcgatgaggttggtggcagagcagtgaatctgctgccaagcgaaaccgtgcaagatatctatggcattgtggctaagaaggttaatgaaatcctgcaagcagacgcgattaacggcacggacaacgaggttgtcaccgtgaccgatgaaaacaccggtgagatctcggagaaagtgaaactgggcaccaaagccttggctggccaatggctggcatacggcgttactcgctccgtgaccaagcgttcggtgatgacccttgcttacggcagcaaagagtttggtttccgccaacaggttctggaggatactatccaaccggccatcgactctggtaaaggcctgatgttcacgcagccgaatcaggcagcgggctatatggcgaagctgatttgggaatcggttagcgttaccgttgttgcagcggtggaggctatgaactggctgaaatctgcggcgaagctgttagctgcggaggtgaaggacaagaagacgggcgaaatcctgcgtaagcgctgcgcagtgcattgggttacgccggatggttttccggtatggcaggagtacaaaaagcctattcagacccgtctgaacctgatgtttctgggtcaatttcgtctgcagccgacgatcaacaccaataaggactccgagatcgacgcgcacaaacaggagtctggcatcgcacccaatttcgttcactcacaggacggttcccatctgcgtaagaccgtcgtgtgggcacacgagaagtatggcattgagtcgtttgcattgatccacgattcctttggtaccatcccggcggacgctgcgaacctgtttaaagcggttcgcgaaaccatggttgacacctatgaaagttgcgatgttctggcagacttttatgatcagttcgccgaccaactgcatgagtcccagctggataaaatgccggcgttaccggcgaagggcaacttaaatctccgcgacatcctggaatctgatttcgccttcgcgtaa

SEQ ID NO: 115 - DNA, 2652 bp, synthetic construct
  source 1..2652: mol_type = other DNA
atgaatacaattaacatagctaaaaatgatttcagcgatattgaactggctgcgatcccgtttaataccttggcggaccattatggtgagcgtctggcgcgtgagcaacttgctctggagcacgaatcctacgagatgggtgaagcgcgtttcgcgaagatgttcgagcgccagcttaaggctggcgaggtggcggataacgctgctgcgaagccgttgattacgaccctgctgccgaaaatgattgcgcgtattaacgattggttcgaggaagtgaaagcaaagcgtggtaaacgtccaaccgcattccagtttctgcaagagatcaagccggaggcggtggcatacattacgatcaaaaccactctcgcatgtctcaccagcgcggataatactacggtccaagcggtggccagcgcgattggccgcgcgattgaggacgaagcgcgttttggtcgcattcgtgacctggaagcgaaacattttaagaagaacgttgaagaacaattgaataaacgcgtgggccacgtttacgataaagcgttcatgcaagtcgttgaagctgatatgctgagcaaaggcctgttaggtggtgaagcatggagcagctggcataaggaggactcaattcacgtcggcgtgcggtgcattgaaatgctgatcgaatcgaccggtatggttagcctgcatcgccaaaacgccggcgtggtgggtcaagatagcgaaacgattgaactggcgccagagtacgcggaagctatcgctaccagagccggcgcattggcggggatcagcccgatgttccagccgtgtgttgtaccaccgaagccgtggaccggtatcaccggtggaggttactgggcgaatggtagacgtccgttggcgttggttcgtacccatagcaaaaaggctctgatgcgttatgaagacgtttacatgccggaagtgtacaaagccatcaacatcgcgcagaacactgcgtggaaaatcaacaaaaaggtgttagctgtggcgaacgtaattacaaaatggaagcactgcccggttgaggacatcccggctattgaacgtgaagagctgccaatgaaaccagaggacattgacatgaatccggaggcgctgaccgcatggaaacgtgcggcagcagcggtctatcgtaaggataaagccagaaagagccgtcgtatctccctggaattcatgcttgagcaggcgaacaaattcgctaaccacaaagccatctggtttccgtataatatggattggcgtggtcgtgtttacgcggtatcgatgttcaacccgcagggtaatgacatgaccaagggtttgttgaccttggccaaaggtaaaccgattggcaaagaaggttactattggttgaagatccacggtgcgaactgcgcaggggtggataaggtaccgttcccggaacgtattaaattcatcgaggaaaaccacgaaaacattatggcgtgcgcaaagagcccgctggaaaacacgtggtgggcagagcaggacagtccattctgcttcttggcgttctgtttcgaatatgcaggtgtccagcaccacggcctgagctataactgcagcctgccgctggcctttgatggttcttgtagcggtattcaacactttagcgccatgctgcgcgatgaggttggtggcagagcagtgaatctgctgccaagcgaaaccgtgcaagatatctatggcattgtggctaagaaggttaatgaaatcctgcaagcagacgcgattaacggcacggacaacgaggttgtcaccgtgaccgatgaaaacaccggtgagatctcggagaaagtgaaactgggcaccaaagccttggctggccaatggctggcatacggcgttactcgctccgtgaccaagcgttcggtgatgacccttgcttacggcagcaaagagtttggtttccgccaacaggttctggaggatactatccaaccggccatcgactctggtaaaggcctgatgttcacgcagccgaatcaggcagcgggctatatggcgaagctgatttgggaatcggttagcgttaccgttgttgcagcggtggaggctatgaactggctgaaatctgcggcgaagctgttagctgcggaggtgaaggacaagaagacgggcgaaatcctgcgtaagcgctgcgcagtgcattgggttacgccggatggttttccggtatggcaggagtacaaaaagcctattcagacccgtctgaacctgatgtttctgggtcaatttcgtctgcagccgacgatcaacaccaataaggactccgagatcgacgcgcacaaacaggagtctggcatcgcacccaatttcgttcactcacaggacggttcccatctgcgtaagaccgtcgtgtgggcacacgagaagtatggcattgagtcgtttgcattgatccacgattcctttggtaccatcccggcggacgctgcgaacctgtttaaagcggttcgcgaaaccatggttgacacctatgaaagttgcgatgttctggcagacttttatgatcagttcgccgaccaactgcatgagtcccagctggataaaatgccggcgttaccggcgaagggcaacttaaatctccgcgacatcctggaatctgatttcgccttcgcgtaa

SEQ ID NO: 116 - DNA, 2652 bp, synthetic construct
  source 1..2652: mol_type = other DNA
atgaatacaattaacatagctaaaaatgatttcagcgatattgaactggctgcgatcccgtttaataccttggcggaccattatggtgagcgtctggcgcgtgagcaacttgctctggagcacgaatcctacgagatgggtgaagcgcgtttcgcgaagatgttcgagcgccagcttaaggctggcgaggtggcggataacgctgctgcgaagccgttgattacgaccctgctgccgaaaatgattgcgcgtattaacgattggttcgaggaagtgaaagcaaagcgtggtaaacgtccaaccgcattccagtttctgcaagagatcaagccggaggcggtggcatacattacgatcaaaaccactctcgcatgtctcaccagcgcggataatactacggtccaagcggtggccagcgcgattggccgcgcgattgaggacgaagcgcgttttggtcgcattcgtgacctggaagcgaaacattttaagaagaacgttgaagaacaagaaaataaacgcgtgggccacgtttacaagaaagcgttcatgcaagtcgttgaagctgatatgctgagcaaaggcctgttaggtggtgaagcatggagcagctggcataaggaggactcaattcacgtcggcgtgcggtgcattgaaatgctgatcgaatcgaccggtatggttagcctgcatcgccaaaacgccggcgtggtgggtcaagatagcgaaacgattgaactggcgccagagtacgcggaagctatcgctaccagagccggcgcattggcggggatcagcccgatgttccagccgtgtgttgtaccaccgaagccgtggaccggtatcaccggtggaggttactgggcgaatggtagacgtccgttggcgttggttcgtacccatagcaaaaaggctctgatgcgttatgaagacgtttacatgccggaagtgtacaaagccatcaacatcgcgcagaacactgcgtggaaaatcaacaaaaaggtgttagctgtggcgaacgtaattacaaaatggaagcactgcccggttgaggacatcccggctattgaacgtgaagagctgccaatgaaaccagaggacattgacatgaatccggaggcgctgaccgcatggaaacgtgcggcagcagcggtctatcgtaaggataaagccagaaagagccgtcgtatctccctggaattcatgcttgagcaggcgaacaaattcgctaaccacaaagccatctggtttccgtataatatggattggcgtggtcgtgtttacgcggtatcgatgttcaacccgcagggtaatgacatgaccaagggtttgttgaccttggccaaaggtaaaccgattggcaaagaaggttactattggttgaagatccacggtgcgaactgcgcaggggtggataaggtaccgttcccggaacgtattaaattcatcgaggaaaaccacgaaaacattatggcgtgcgcaaagagcccgctggaaaacacgtggtgggcagagcaggacagtccattctgcttcttggcgttctgtttcgaatatgcaggtgtccagcaccacggcctgagctataactgcagcctgccgctggcctttgatggttcttgtagcggtattcaacactttagcgccatgctgcgcgatgaggttggtggcagagcagtgaatctgctgccaagcgaaaccgtgcaagatatctatggcattgtggctaagaaggttaatgaaatcctgcaagcagacgcgattaacggcacggacaacgaggttgtcaccgtgaccgatgaaaacaccggtgagatctcggagaaagtgaaactgggcaccaaagccttggctggccaatggctggcatacggcgttactcgctccgtgaccaagcgttcggtgatgacccttgcttacggcagcaaagagtttggtttccgccaacaggttctggaggatactatccaaccggccatcgactctggtaaaggcctgatgttcacgcagccgaatcaggcagcgggctatatggcgaagctgatttgggaatcggttagcgttaccgttgttgcagcggtggaggctatgaactggctgaaatctgcggcgaagctgttagctgcggaggtgaaggacaagaagacgggcgaaatcctgcgtaagcgctgcgcagtgcattgggttacgccggatggttttccggtatggcaggagtacaaaaagcctattcagacccgtctgaacctgatgtttctgggtcaatttcgtctgcagccgacgatcaacaccaataaggactccgagatcgacgcgcacaaacaggagtctggcatcgcacccaatttcgttcactcacaggacggttcccatctgcgtaagaccgtcgtgtgggcacacgagaagtatggcattgagtcgtttgcattgatccacgattcctttggtaccatcccggcggacgctgcgaacctgtttaaagcggttcgcgaaaccatggttgacacctatgaaagttgcgatgttctggcagacttttatgatcagttcgccgaccaactgcatgagtcccagctggataaaatgccggcgttaccggcgaagggcaacttaaatctccgcgacatcctggaatctgatttcgccttcgcgtaa

SEQ ID NO: 117 - DNA, 4388 bp, synthetic construct
  source 1..4388: mol_type = other DNA
taatacgactcactatagggagaaaataacaaatctcaacacaacatatacaaaacaaacgaatctcaagcaatcaagcattctacttctattgcagcaatttaaatcatttcttttaaagcaaaagcaattttctgaaaattttcaccatttacgaacgatagcagccaccatgttcgtgtttctggtgctgctgcctctggtgagctcccagtgcgtgaatctgaccacaaggacccagctgccccctgcctataccaactccttcacacggggcgtgtactatcccgacaaggtgttccggagcagcgtgctgcactccacacaggatctgtttctgcctttcttttctaacgtgacctggttccacgccatccacgtgagcggcaccaatggcacaaagaggttcgacaacccagtgctgcccttcaatgatggcgtgtacttcgcctccaccgagaagtctaatatcatccgcggctggatctttggcaccacactggacagcaagacacagtccctgctgatcgtgaacaatgccaccaacgtggtcatcaaggtgtgcgagttccagttttgtaacgatccattcctgggcgtgtactatcacaagaacaataagtcttggatggagagcgagtttcgcgtgtattcctctgccaacaattgcacatttgagtacgtgtcccagcccttcctgatggacctggagggcaagcagggcaatttcaagaacctgcgggagttcgtgtttaagaacatcgatggctacttcaaaatctactccaagcacaccccaatcaatctggtgagagacctgccacagggcttctctgccctggagccactggtggatctgcccatcggcatcaacatcacccggtttcagacactgctggccctgcacagaagctacctgacaccaggcgacagctcctctggatggaccgcaggagcagcagcctactatgtgggctatctgcagcccaggaccttcctgctgaagtacaacgagaatggcaccatcacagacgcagtggattgcgcactggaccccctgtctgagaccaagtgtacactgaagtcctttaccgtggagaagggcatctatcagacaagcaacttcagggtgcagcctaccgagtccatcgtgcgctttcccaatatcacaaacctgtgcccttttggcgaggtgttcaatgcaaccaggttcgcaagcgtgtacgcatggaataggaagcgcatctccaactgcgtggccgactattctgtgctgtacaatagcgcctccttctctacctttaagtgctacggcgtgagccccacaaagctgaatgacctgtgctttaccaacgtgtacgccgattccttcgtgatcaggggcgacgaggtgcgccagatcgcaccaggacagacaggcaagatcgcagactacaactataagctgcctgacgatttcaccggctgcgtgatcgcctggaacagcaacaatctggatagcaaagtgggcggcaactacaattatctgtaccggctgtttagaaagtctaacctgaagccattcgagagggacatctccacagaaatctaccaggccggctctaccccctgcaatggcgtggagggctttaactgttatttccctctgcagagctacggcttccagccaacaaatggcgtgggctatcagccctaccgcgtggtggtgctgtcttttgagctgctgcacgcccctgcaacagtgtgcggaccaaagaagtccaccaatctggtgaagaacaagtgcgtgaacttcaacttcaacggactgaccggcacaggcgtgctgaccgagtccaacaagaagttcctgccttttcagcagttcggcagggacatcgcagataccacagacgccgtgcgcgaccctcagaccctggagatcctggatatcacaccatgctccttcggcggcgtgtctgtgatcacaccaggcaccaatacaagcaaccaggtggccgtgctgtatcaggacgtgaactgtaccgaggtgcccgtggcaatccacgcagatcagctgacccctacatggcgggtgtactctaccggcagcaacgtgttccagacaagagccggatgcctgatcggagcagagcacgtgaacaatagctatgagtgcgacatccctatcggcgccggcatctgtgcctcctaccagacccagacaaactccccaaggagagcacggtctgtggcaagccagtccatcatcgcctataccatgagcctgggcgccgagaactccgtggcctactccaacaattctatcgccatccctaccaatttcacaatctccgtgaccacagagatcctgccagtgagcatgaccaagacatccgtggactgcacaatgtatatctgtggcgattccaccgagtgctctaatctgctgctgcagtacggctctttttgtacccagctgaacagagccctgacaggcatcgccgtggagcaggacaagaatacacaggaggtgttcgcccaggtgaagcaaatctacaagaccccacccatcaaggactttggcggcttcaactttagccagatcctgcccgatcctagcaagccatccaagcggtcttttatcgaggacctgctgttcaataaggtgaccctggccgatgccggcttcatcaagcagtatggcgattgcctgggcgacatcgccgccagagacctgatctgtgcccagaagtttaacggcctgaccgtgctgcctccactgctgacagatgagatgatcgcccagtacacatctgccctgctggcaggcaccatcacaagcggatggaccttcggcgcaggagccgccctgcagatcccctttgccatgcagatggcctatcggttcaatggcatcggcgtgacccagaatgtgctgtacgagaaccagaagctgatcgccaatcagtttaactccgccatcggcaagatccaggactctctgagctccacagcaagcgccctgggcaagctgcaggatgtggtgaatcagaacgcccaggccctgaacaccctggtgaagcagctgtctagcaatttcggcgccatctcctctgtgctgaacgatatcctgagccggctggacaaggtggaggcagaggtgcagatcgaccggctgatcacaggcagactgcagtccctgcagacctacgtgacacagcagctgatcagggcagcagagatcagggcatctgccaacctggcagcaaccaagatgagcgagtgcgtgctgggccagtccaagagagtggacttttgtggcaagggctatcacctgatgagcttcccacagtccgcccctcacggagtggtgtttctgcacgtgacctacgtgccagcccaggagaagaacttcaccacagcaccagcaatctgccacgatggcaaggcacactttcctagggagggcgtgttcgtgagcaatggcacccactggtttgtgacacagcgcaacttctacgagccacagatcatcaccacagacaatacattcgtgtccggcaactgtgacgtggtcatcggcatcgtgaacaataccgtgtatgatcctctgcagccagagctggactcttttaaggaggagctggataagtacttcaagaaccacaccagccccgacgtggatctgggcgacatctctggcatcaatgccagcgtggtgaacatccagaaggagatcgacaggctgaatgaggtggccaagaatctgaacgagtccctgatcgatctgcaggagctgggcaagtatgagcagtacatcaagtggccctggtatatctggctgggcttcatcgccggcctgatcgccatcgtgatggtgaccatcatgctgtgctgtatgacaagctgctgttcctgcctgaagggctgctgttcttgtggcagctgctgtaagtttgatgaggacgatagcgagcctgtgctgaagggcgtgaagctgcactacacctgagaattcaaccagcctcaagaacacccgaatggagtctctaagctacataataccaacttacactttacaaaatgttgtcccccaaaatgtagccattcgtatctgctcctaataaaaagaaagtttcttcacattctaaccagcctcaagaacacccgaatggagtctctaagctacataataccaacttacactttacaaaatgttgtcccccaaaatgtagccattcgtatctgctcctaataaaaagaaagtttcttcacattctaagcttaaaaaaaaaaaaaaaaaaaaaaaaaaaaaaaaaaaaaaaaaaaaaaaaaaaaaaaaaaaaaaaaaaaaaaaaaaaaaaaaaaaaaaaaaaaaaaaaaaaaaaaaaaaaaaaaaaaaaaaa